European Patent Application EP 4 342 298 A2, published March 27, 2024. Title: GRASS ENDOPHYTES. Applicant: RAGT 2N. The sequence listing filed with the application follows.

SEQUENCE LISTING (817 sequences)

SEQ ID NO: 1 - DNA, 102 bp, synthetic construct
  misc_feature 1..102: note = Epichloe festucae
  misc_feature 51: note = Variation - S is T strain AR37 or A strain RGT18
  source 1..102: mol_type = other DNA
ctttacctaaagcattaacttagggtttaaaggaatacctcctctaagaasaatttctaaatccttcgctcctataaggtattactaaaggtacttctaaag

SEQ ID NO: 2 - DNA, 102 bp, synthetic construct
  misc_feature 1..102: note = Epichloe festucae
  misc_feature 51: note = Variation - S is A strain AR37 or G strain RGT18
  source 1..102: mol_type = other DNA
gaccgactgcgcagatcccgtcaagttgtcatgccgatctgaaactctagscccctcccactcttcactgcacaactcgacagcccggtttgtgtcagtgaa

SEQ ID NO: 3 - DNA, 102 bp, synthetic construct
  misc_feature 1..102: note = Epichloe festucae
  misc_feature 51: note = Variation - S is G strain AR37 or A strain RGT18
  source 1..102: mol_type = other DNA
attccttaaactagttatcttaagatattatagaattacttactattaagsagaataaagttataaagataagaaagagagaaaaaagagttaagggagtaa

SEQ ID NO: 4 - DNA, 102 bp, synthetic construct
  misc_feature 1..102: note = Epichloe festucae
  misc_feature 51: note = Variation - S is A strain AR37 or G strain RGT18
  source 1..102: mol_type = other DNA
ctcctgggtctcctggtctagtcgcgagataagtcgcgagataagataagsctggacagcaacaagctgctgtgttgttgcatgttccaacagccattgagc

SEQ ID NO: 5 - DNA, 102 bp, synthetic construct
  misc_feature 1..102: note = Epichloe festucae
  misc_feature 51: note = Variation - S is C strain AR37 or A strain RGT18
  source 1..102: mol_type = other DNA
tagctcatcacaataattcatgagaacaattttttattattattattattsttcttcttcttcttcttcttcttgtccttctcctatttagccgccatttcc

SEQ ID NO: 6 - DNA, 102 bp, synthetic construct
  misc_feature 1..102: note = Epichloe festucae
  misc_feature 51: note = Variation - S is C strain AR37 or A strain RGT18
  source 1..102: mol_type = other DNA
cggccggccaggaacatgggaatggcagtggacgcggtttgcaggatgacscccaggttgaagacccagcatgagatgatgagagccagacgccggccaatg

SEQ ID NO: 7 - DNA, 102 bp, synthetic construct
  misc_feature 1..102: note = Epichloe festucae
  misc_feature 51: note = Variation - S is A strain AR37 or G strain RGT18
  source 1..102: mol_type = other DNA
atacagaatggtgtaattgtaagtcctatacaaagagagagagagagaaasggggggcaaaggagagaaaacatcatacgcaccagtcccaagatcagaaac

SEQ ID NO: 8 - DNA, 102 bp, synthetic construct
  misc_feature 1..102: note = Epichloe festucae
  misc_feature 51: note = Variation - S is G strain AR37 or A strain RGT18
  source 1..102: mol_type = other DNA
acgccatcatcggggcctcggccgccctcgccggcgtaacacgcatgacgstatccatcgtcgtcatcatgttcgagctcacgggcgcgctgacgtatgtgc

SEQ ID NO: 9 - DNA, 102 bp, synthetic construct
  misc_feature 1..102: note = Epichloe festucae
  misc_feature 51: note = Variation - S is A strain AR37 or T strain RGT18
  source 1..102: mol_type = other DNA
atttttttttcgatggatgcgggcggttttcgatggtattggcggtcggascgggtcagaggaggacgactcaccactgcgactctaccggcaacagagacg

SEQ ID NO: 10 - DNA, 102 bp, synthetic construct
  misc_feature 1..102: note = Epichloe festucae
  misc_feature 51: note = Variation - S is A strain AR37 or G strain RGT18
  source 1..102: mol_type = other DNA
tttccctgaatccattcgttccctggtccctggtctaggtgtgggagtgasttggtggagcaatttacggatccgtacccgagctctgatcgacgagcggac

SEQ ID NO: 11 - DNA, 102 bp, synthetic construct
  misc_feature 1..102: note = Epichloe festucae
  misc_feature 51: note = Variation - S is T strain AR37 or C strain RGT18
  source 1..102: mol_type = other DNA
tggtgttccaggtgacgaggttcgggctgacgccatgctctcgcatgattsgaaggatctgctcggccagcaggcggtcgcggccgttcatcaaaccccgca

SEQ ID NO: 12 - DNA, 102 bp, synthetic construct
  misc_feature 1..102: note = Epichloe festucae
  misc_feature 51: note = Variation - S is A strain AR37 or G strain RGT18
  source 1..102: mol_type = other DNA
atgggtgcgtctagcaggacaagccagacgtatatcctcaagggtgactasccgggaaaacccctccaatgtcagtaaaagacgactgcttttctcgaactg

SEQ ID NO: 13 - DNA, 102 bp, synthetic construct
  misc_feature 1..102: note = Epichloe festucae
  misc_feature 51: note = Variation - S is T strain AR37 or C strain RGT18
  source 1..102: mol_type = other DNA
tgttgttgtgtgttgtgtgcgggcgaggaggggcagttttccatacctatsgtgtgaccccgctgctccatgtagtcaaagaaggccttgcgcacccgcgca

SEQ ID NO: 14 - DNA, 102 bp, synthetic construct
  misc_feature 1..102: note = Epichloe festucae
  misc_feature 51: note = Variation - S is G strain AR37 or C strain RGT18
  source 1..102: mol_type = other DNA
ccgtctacggagactcccgtgagaagaaaagttaccaggctgttgcacacsccccgacactagaggcgtcatcttcttcttgtccccaccgcctggcaccac

SEQ ID NO: 15 - DNA, 102 bp, synthetic construct
  misc_feature 1..102: note = Epichloe festucae
  misc_feature 51: note = Variation - S is T strain AR37 or G strain RGT18
  source 1..102: mol_type = other DNA
acgagctctagaagtacttcttgcgcattgctgttgccgctgagtcgactsctattgatgaaggggaattcggatacctgatctatcgagggtaggcgcaca

SEQ ID NO: 16 - DNA, 102 bp, synthetic construct
  misc_feature 1..102: note = Epichloe festucae
  misc_feature 51: note = Variation - S is G strain AR37 or A strain RGT18
  source 1..102: mol_type = other DNA
agagctcaatgactgccacgccagagtacatggcccccaggcccaatatcsccaggcccgggcaagcgcaacaagactctgaggaatacatactgcaataag

SEQ ID NO: 17 - DNA, 102 bp, synthetic construct
  misc_feature 1..102: note = Epichloe festucae
  misc_feature 51: note = Variation - S is C strain AR37 or A strain RGT18
  source 1..102: mol_type = other DNA
tcccccactacatcacgtgtaaggaaaggggctgggcgctggcatgtattsgggcacactccaggccaccctgctcaggtccatctgcttactgttggttgg

SEQ ID NO: 18 - DNA, 102 bp, synthetic construct
  misc_feature 1..102: note = Epichloe festucae
  misc_feature 51: note = Variation - S is C strain AR37 or G strain RGT18
  source 1..102: mol_type = other DNA
cactgcactgcactgcacgtagcacccatctcgttcaaatctaggtccaasggaagcgtccctttttttcaaagagaagaaggaatgctgagacatcgggac

SEQ ID NO: 19 - DNA, 102 bp, synthetic construct
  misc_feature 1..102: note = Epichloe festucae
  misc_feature 51: note = Variation - S is C strain AR37 or T strain RGT18
  source 1..102: mol_type = other DNA
gcaagactgcaagactgcaagattgcactgcgacaacacccaggttggtascaccaaacacccccaaacacccccaaacaccccaggcagccacccggacgt

SEQ ID NO: 20 - DNA, 102 bp, synthetic construct
  misc_feature 1..102: note = Epichloe festucae
  misc_feature 51: note = Variation - S is T strain AR37 or C strain RGT18
  source 1..102: mol_type = other DNA
cgccgcaggagccgcaggagccacaggagccacagggactacgggagccastgatggaatccacggccaactccagcgtcacggcggccaatcacatctgca

SEQ ID NO: 21 - DNA, 102 bp, synthetic construct
  misc_feature 1..102: note = Epichloe festucae
  misc_feature 51: note = Variation - S is G strain AR37 or A strain RGT18
  source 1..102: mol_type = other DNA
gatacttgttacttatcacaaagaagagattaaaaatctagttaattctascgcatttcttaactatagccctagaggacaataacttaaccgcggtctcta

SEQ ID NO: 22 - DNA, 102 bp, synthetic construct
  misc_feature 1..102: note = Epichloe festucae
  misc_feature 51: note = Variation - S is T strain AR37 or C strain RGT18
  source 1..102: mol_type = other DNA
gcatattaactcatggctgctcataggtcgatttgattgaatgtatggttstctctcaccgtgagaacaatccacccctctcgtggaagagtcaatgttttt

SEQ ID NO: 23 - DNA, 102 bp, synthetic construct
  misc_feature 1..102: note = Epichloe festucae
  misc_feature 51: note = Variation - S is T strain AR37 or C strain RGT18
  source 1..102: mol_type = other DNA
ccttccttatgcctcctaataaactcatctttgataggaaaagtgtggagsggaaccaccagctatatgtatagacatgtatcagctgcctgcaaaagacct

SEQ ID NO: 24 - DNA, 102 bp, synthetic construct
  misc_feature 1..102: note = Epichloe festucae
  misc_feature 51: note = Variation - S is A strain AR37 or G strain RGT18
  source 1..102: mol_type = other DNA
ggaagatgccatgaagaacgaactcggaactattttaactggcctccaggscaggctccttgctcaggtaccggcgtacatgatcccgtccgcttacattcc

SEQ ID NO: 25 - DNA, 102 bp, synthetic construct
  misc_feature 1..102: note = Epichloe festucae
  misc_feature 51: note = Variation - S is T strain AR37 or C strain RGT18
  source 1..102: mol_type = other DNA
agcagcctcctctgcttggtctacggccacggccacggccaccccgacgcscacagattttgcaggctccgcctcgtccatggcgtcagttgctgggaagtc

SEQ ID NO: 26 - DNA, 102 bp, synthetic construct
  misc_feature 1..102: note = Epichloe festucae
  misc_feature 51: note = Variation - S is T strain AR37 or C strain RGT18
  source 1..102: mol_type = other DNA
aactttattttctaatatctttagtatattaacttataaattataactacsttatattaactttattacttagctattacttatagttattaataatttctc

SEQ ID NO: 27 - DNA, 102 bp, synthetic construct
  misc_feature 1..102: note = Epichloe festucae
  misc_feature 51: note = Variation - S is G strain AR37 or A strain RGT18
  source 1..102: mol_type = other DNA
tataaggggttaatgggaagaaaatcacctagggaaagggcctatgtgatsatctaggctttgcctagacctagcaatataggtgttaattgcataagttac

SEQ ID NO: 28 - DNA, 102 bp, synthetic construct
  misc_feature 1..102: note = Epichloe festucae
  misc_feature 51: note = Variation - S is C strain AR37 or T strain RGT18
  source 1..102: mol_type = other DNA
attctagaaataacgataaatcttcgcctttcctctatttatctttattasacctaaccttagtcgtggcaatttgccactagctataataacaatagcgct

SEQ ID NO: 29 - DNA, 102 bp, synthetic construct
  misc_feature 1..102: note = Epichloe festucae
  misc_feature 51: note = Variation - S is G strain AR37 or A strain RGT18
  source 1..102: mol_type = other DNA
cgtgcctaaataataataagcaattattaaagctatctataaggaacttasctataaaggagttaaagtggttttttaagtaataaagtaataatactagtg

SEQ ID NO: 30 - DNA, 102 bp, synthetic construct
  misc_feature 1..102: note = Epichloe festucae
  misc_feature 51: note = Variation - S is G strain AR37 or A strain RGT18
  source 1..102: mol_type = other DNA
cctagccgatctaaatcctattatactaggactaggtatataataaaggtstcctttagcttattaaaggcattattctctttaagtccttattagaaaggg

SEQ ID NO: 31 - DNA, 102 bp, synthetic construct
  misc_feature 1..102: note = Epichloe festucae
  misc_feature 51: note = Variation - S is C strain AR37 or T strain RGT18
  source 1..102: mol_type = other DNA
cttttatagttactcttactatactaatatcctattttattagtaagtacsttataaaaggaaactctaataataaatagtatactatacttaaattagtct

SEQ ID NO: 32 - DNA, 102 bp, synthetic construct
  misc_feature 1..102: note = Epichloe festucae
  misc_feature 51: note = Variation - S is G strain AR37 or A strain RGT18
  source 1..102: mol_type = other DNA
cctgagcactggcgctctactatggactacgccggacacgagtccagggasaccgagacccagagcggctcaaacgggactttgaggatcccaatggatggc

SEQ ID NO: 33 - DNA, 102 bp, synthetic construct
  misc_feature 1..102: note = Epichloe festucae
  misc_feature 51: note = Variation - S is G strain AR37 or A strain RGT18
  source 1..102: mol_type = other DNA
attaaacttctcttattattttagaagaaaacatagctaattttattaagsactttaaggtaaagataaaagcaataggtattcctaaggcaaattagcgta

SEQ ID NO: 34 - DNA, 102 bp, synthetic construct
  misc_feature 1..102: note = Epichloe festucae
  misc_feature 51: note = Variation - S is C strain AR37 or A strain RGT18
  source 1..102: mol_type = other DNA
attataatacttatttaaatagtaagtaaggtaaattcagtacttaactastaagtcagatatagtacttatactaatttagcctaaataaaagtctctttt

SEQ ID NO: 35 - DNA, 102 bp, synthetic construct
  misc_feature 1..102: note = Epichloe festucae
  misc_feature 51: note = Variation - S is C strain AR37 or T strain RGT18
  source 1..102: mol_type = other DNA
ttatagtttctagagtttttctagctaagtaatttactttattattactasagctttaatagtaagggttaagggtttgaatctaagtatagtctttataaa

SEQ ID NO: 36 - DNA, 102 bp, synthetic construct
  misc_feature 1..102: note = Epichloe festucae
  misc_feature 51: note = Variation - S is T strain AR37 or C strain RGT18
  source 1..102: mol_type = other DNA
gaagatataatagataatattacctagtaaggaaagaagtaataagtgccstataaaaggcttataataagtctaggtattttaaagcaaacctaacctagt

SEQ ID NO: 37 - DNA, 102 bp, synthetic construct
  misc_feature 1..102: note = Epichloe festucae
  misc_feature 51: note = Variation - S is T strain AR37 or C strain RGT18
  source 1..102: mol_type = other DNA
ctagaatagtattatatacctagttacttactactttactagccttatatscttataaaaaaactatataatttataataaaaaactattagctattatctt

SEQ ID NO: 38 - DNA, 102 bp, synthetic construct
  misc_feature 1..102: note = Epichloe festucae
  misc_feature 51: note = Variation - S is C strain AR37 or T strain RGT18
  source 1..102: mol_type = other DNA
tcttattaataagttctttaagatcctttaatagtattattaatatactcstaaaaagttactaatatattaaatagtttaaatagtattataagatattta

SEQ ID NO: 39 - DNA, 102 bp, synthetic construct
  misc_feature 1..102: note = Epichloe festucae
  misc_feature 51: note = Variation - S is T strain AR37 or C strain RGT18
  source 1..102: mol_type = other DNA
ttagcttaattactatattattagtaattaggttaagatagcttcctttcscttattattatgcccttatataataaggtataatttcttatatagtgattt

SEQ ID NO: 40 - DNA, 102 bp, synthetic construct
  misc_feature 1..102: note = Epichloe festucae
  misc_feature 51: note = Variation - S is A strain AR37 or G strain RGT18
  source 1..102: mol_type = other DNA
aggcacttaagcttactctttttagggttttaagtaataatattcttaagsgtaatattactttacttatagtaataattataagagaggttcttactagta

SEQ ID NO: 41 - DNA, 102 bp, synthetic construct
  misc_feature 1..102: note = Epichloe festucae
  misc_feature 51: note = Variation - S is A strain AR37 or G strain RGT18
  source 1..102: mol_type = other DNA
gtagttcctaggcattaaaatcattaggaatcgtaatactaaagagatatsgttattataggaattatatatttaaaagatagcttagaagtttatgcctaa

SEQ ID NO: 42 - DNA, 102 bp, synthetic construct
  misc_feature 1..102: note = Epichloe festucae
  misc_feature 51: note = Variation - S is A strain AR37 or G strain RGT18
  source 1..102: mol_type = other DNA
aagaatatatagctaaattagctataatataagtaatttactaaagagtasttaagccctcctaggagtaaaaattctctttaacctaagtatatatattag

SEQ ID NO: 43 - DNA, 102 bp, synthetic construct
  misc_feature 1..102: note = Epichloe festucae
  misc_feature 51: note = Variation - S is A strain AR37 or G strain RGT18
  source 1..102: mol_type = other DNA
tagttatagaatttatattttattagttattagtattataaggattaaaasaatgctagttatataaaagcttttattattacctattttatttaattagtt

SEQ ID NO: 44 - DNA, 102 bp, synthetic construct
  misc_feature 1..102: note = Epichloe festucae
  misc_feature 51: note = Variation - S is C strain AR37 or T strain RGT18
  source 1..102: mol_type = other DNA
agatttatattataagtagtatccctcctaatagcatttagctaactttasttctaatacctatttagcttattatatatttatagtaagctttagactctt

SEQ ID NO: 45 - DNA, 102 bp, synthetic construct
  misc_feature 1..102: note = Epichloe festucae
  misc_feature 51: note = Variation - S is C strain AR37 or T strain RGT18
  source 1..102: mol_type = other DNA
tcgctcggcggctggctggctgatcatggccctcttctttttttttttttsttttttttttttttttggttgtaacagttccattttgccgcgtcgcggacc

SEQ ID NO: 46 - DNA, 102 bp, synthetic construct
  misc_feature 1..102: note = Epichloe festucae
  misc_feature 51: note = Variation - S is T strain AR37 or A strain RGT18
  source 1..102: mol_type = other DNA
ttattataatttagttatttagttataaattcttaaagtttaagattattsagattattaagctaagtataggtatatagaagctaaatatagtatatttta

SEQ ID NO: 47 - DNA, 102 bp, synthetic construct
  misc_feature 1..102: note = Epichloe festucae
  misc_feature 51: note = Variation - S is C strain AR37 or A strain RGT18
  source 1..102: mol_type = other DNA
tttatttagtttattatagctaacttatatctattatagctaacttatagstagtttactatatctaagtcttatattagaactttacctttattactacct

SEQ ID NO: 48 - DNA, 102 bp, synthetic construct
  misc_feature 1..102: note = Epichloe festucae
  misc_feature 51: note = Variation - S is C strain AR37 or T strain RGT18
  source 1..102: mol_type = other DNA
aggtataaaatcctatataatagcactgttagtagtatatagaatctcttstagatataaaatcctatataatagcactcctatattaactttctttaagtt

SEQ ID NO: 49 - DNA, 102 bp, synthetic construct
  misc_feature 1..102: note = Epichloe festucae
  misc_feature 51: note = Variation - S is T strain AR37 or C strain RGT18
  source 1..102: mol_type = other DNA
ccttctaggtctcttacaaagtgcaaaatgcatataaccggacgcgctagstattttcattagctaagatccatacaaattcatggaattttatctaaatta

SEQ ID NO: 50 - DNA, 102 bp, synthetic construct
  misc_feature 1..102: note = Epichloe festucae
  misc_feature 51: note = Variation - S is G strain AR37 or A strain RGT18
  source 1..102: mol_type = other DNA
acggttagggactagtagaactaccacattgaatatttatttaacgtgacstaacggaaggttttagcagttattaactaatagaatttaatctagatgact

SEQ ID NO: 51 - DNA, 102 bp, synthetic construct
  misc_feature 1..102: note = Epichloe festucae
  misc_feature 51: note = Variation - S is G strain AR37 or A strain RGT18
  source 1..102: mol_type = other DNA
acattcgccgtgacggcaacgttttctactctttaccattactagatgatsggtccagcaaaaaaaactaagcatgctcatgctatactagatttggctaat

SEQ ID NO: 52 - DNA, 102 bp, synthetic construct
  misc_feature 1..102: note = Epichloe festucae
  misc_feature 51: note = Variation - S is T strain AR37 or C strain RGT18
  source 1..102: mol_type = other DNA
ttatttttcttagtttatgtggctattcccctataggttaactagtgctasaaaggtagtaaactatctataggcttagataaataggttattgcttactct

SEQ ID NO: 53 - DNA, 102 bp, synthetic construct
  misc_feature 1..102: note = Epichloe festucae
  misc_feature 51: note = Variation - S is C strain AR37 or T strain RGT18
  source 1..102: mol_type = other DNA
ctaaatgatgagaaagcagacacagatggcgtcaacttcgacacgatggasgatgacgatgatgaagatgatgacaatgacgacgaagcattgacaaatctt

SEQ ID NO: 54 - DNA, 102 bp, synthetic construct
  misc_feature 1..102: note = Epichloe festucae
  misc_feature 51: note = Variation - S is G strain AR37 or T strain RGT18
  source 1..102: mol_type = other DNA
ataagggttctattaactaattttctattaatcctaataataaccttagtsaataaaaagttatacttttttttacctaacaatacatttgtattgtttata

SEQ ID NO: 55 - DNA, 102 bp, synthetic construct
  misc_feature 1..102: note = Epichloe festucae
  misc_feature 51: note = Variation - S is T strain AR37 or C strain RGT18
  source 1..102: mol_type = other DNA
cttaaggtataggataatacctactaaattactaagggttagtaagactasatattcctaatagacctaagtataacattataggctaaagctaggtaatta

SEQ ID NO: 56 - DNA, 102 bp, synthetic construct
  misc_feature 1..102: note = Epichloe festucae
  misc_feature 51: note = Variation - S is A strain AR37 or G strain RGT18
  source 1..102: mol_type = other DNA
atacttattttcctatagtattaagtacttaaaatagtctaataaatctasgggttagcttttattttatattcttaagcctaatattctttactaatagta

SEQ ID NO: 57 - DNA, 102 bp, synthetic construct
  misc_feature 1..102: note = Epichloe festucae
  misc_feature 51: note = Variation - S is A strain AR37 or G strain RGT18
  source 1..102: mol_type = other DNA
aatctaaggtatatagctagaaaaccacactaagggcttaacctagaaatsaataaaagggagcttataaagttacttactcctatattcactctaggctat

SEQ ID NO: 58 - DNA, 102 bp, synthetic construct
  misc_feature 1..102: note = Epichloe festucae
  misc_feature 51: note = Variation - S is C strain AR37 or T strain RGT18
  source 1..102: mol_type = other DNA
aggcattaaagcttagagaagtatagtaaactacttatatattagagaagsgtagtaaattacttatatatctctttatatattatagttagtttactaata

SEQ ID NO: 59 - DNA, 102 bp, synthetic construct
  misc_feature 1..102: note = Epichloe festucae
  misc_feature 51: note = Variation - S is G strain AR37 or A strain RGT18
  source 1..102: mol_type = other DNA
taactaaaacgtatagctttttctatagtaatttacttatacttacttatstttatatttaagctatttatttattatttaattttaattaaactttaacac

SEQ ID NO: 60 - DNA, 102 bp, synthetic construct
  misc_feature 1..102: note = Epichloe festucae
  misc_feature 51: note = Variation - S is T strain AR37 or C strain RGT18
  source 1..102: mol_type = other DNA
gtataataaggtaataatacaaaatatactaatttgttaaggtatagaagsatttagtaagagctttataatatataagattttattaatagttaacttatt

SEQ ID NO: 61 - DNA, 102 bp, synthetic construct
  misc_feature 1..102: note = Epichloe festucae
  misc_feature 51: note = Variation - S is T strain AR37 or C strain RGT18
  source 1..102: mol_type = other DNA
agtataattagggatttaagctatagctactatagtaagatagtaatttasatagtcttaggctagtttatctctaggatgtctagagaaagttattttact

SEQ ID NO: 62 - DNA, 102 bp, synthetic construct
  misc_feature 1..102: note = Epichloe festucae
  misc_feature 51: note = Variation - S is T strain AR37 or C strain RGT18
  source 1..102: mol_type = other DNA
ttctataaaaaggattttcagtacgaatagaagacttcccttctataaaastggaagcgcacgagtaatatagaagcattcccttttataaaaaggaagttt

SEQ ID NO: 63 - DNA, 102 bp, synthetic construct
  misc_feature 1..102: note = Epichloe festucae
  misc_feature 51: note = Variation - S is T strain AR37 or C strain RGT18
  source 1..102: mol_type = other DNA
agctacccctataggaagctataaagctaattaccttaaggtagtaaaagsaaaggtaattaaggcctaggcttataatcctaatatccttatacttattaa

SEQ ID NO: 64 - DNA, 102 bp, synthetic construct
  misc_feature 1..102: note = Epichloe festucae
  misc_feature 51: note = Variation - S is T strain AR37 or C strain RGT18
  source 1..102: mol_type = other DNA
cctttaagcttagcagtcttagggaagctagtcttagggaagctataaacsctcttattaaattccttaataatcgaattattaaaggcagcttatatagag

SEQ ID NO: 65 - DNA, 102 bp, synthetic construct
  misc_feature 1..102: note = Epichloe festucae
  misc_feature 51: note = Variation - S is T strain AR37 or G strain RGT18
  source 1..102: mol_type = other DNA
agccggccccctatcttctattagatagactttataaagttcctttttaastctttagatataacgtaaatccggtctaattagaagacaatcatccacata

SEQ ID NO: 66 - DNA, 102 bp, synthetic construct
  misc_feature 1..102: note = Epichloe festucae
  misc_feature 51: note = Variation - S is A strain AR37 or G strain RGT18
  source 1..102: mol_type = other DNA
aattactaggagaagataaataggggcgcgctacctctatttagagttatsctactactactatagctatagtattattattactaggtaatagttatagta

SEQ ID NO: 67 - DNA, 102 bp, synthetic construct
  misc_feature 1..102: note = Epichloe festucae
  misc_feature 51: note = Variation - S is A strain AR37 or G strain RGT18
  source 1..102: mol_type = other DNA
ttttagttagattaatacccttagataattctagccttaaggttattattsattattgtagttataatgtattccttagtagtaaaatatacgcttatatct

SEQ ID NO: 68 - DNA, 102 bp, synthetic construct
  misc_feature 1..102: note = Epichloe festucae
  misc_feature 51: note = Variation - S is T strain AR37 or C strain RGT18
  source 1..102: mol_type = other DNA
tggctagagttagtgtttaattaactacgcactaaattactaagggttagsaagactatatattcctaatagacctaggtataatattataggctaaagcta

SEQ ID NO: 69 - DNA, 102 bp, synthetic construct
  misc_feature 1..102: note = Epichloe festucae
  misc_feature 51: note = Variation - S is A strain AR37 or G strain RGT18
  source 1..102: mol_type = other DNA
aatagtataaggggttttctaatatactaagactaggtagttattccctasaagcttatcttataataagagcttttatagctatactataataatttacta

SEQ ID NO: 70 - DNA, 102 bp, synthetic construct
  misc_feature 1..102: note = Epichloe festucae
  misc_feature 51: note = Variation - S is A strain AR37 or C strain RGT18
  source 1..102: mol_type = other DNA
tggatggatgcatgggtgcgcggccttttttttttttttttttttttttcsccgggctaggcacgatattggcgttggctgtttgtattcatgctttttgga

SEQ ID NO: 71 - DNA, 102 bp, synthetic construct
  misc_feature 1..102: note = Epichloe festucae
  misc_feature 51: note = Variation - S is A strain AR37 or G strain RGT18
  source 1..102: mol_type = other DNA
ggatcctggtcatttccatgtctggggttcttcaactacctacctctatgsacctggctattagcccatggacctggacattaacccatgaccgttttggtg

SEQ ID NO: 72 - DNA, 102 bp, synthetic construct
  misc_feature 1..102: note = Epichloe festucae
  misc_feature 51: note = Variation - S is T strain AR37 or C strain RGT18
  source 1..102: mol_type = other DNA
tggtagttattaactaatagaatttaatttagataacttttacaatatctsatatactaatagaattgattttagtgacgttatacgggcaatgcagctgtt

SEQ ID NO: 73 - DNA, 102 bp, synthetic construct
  misc_feature 1..102: note = Epichloe festucae
  misc_feature 51: note = Variation - S is A strain AR37 or T strain RGT18
  source 1..102: mol_type = other DNA
taggtaagggtaaagtaaaggtaactaaaggtataataataatttataaasaacttatttagtgttataaaagagaaaagtatataatataatagggagtta

SEQ ID NO: 74 - DNA, 102 bp, synthetic construct
  misc_feature 1..102: note = Epichloe festucae
  misc_feature 51: note = Variation - S is G strain AR37 or A strain RGT18
  source 1..102: mol_type = other DNA
atttcttaactagtcgctgaagagtatttcgcgtctgactaatcagaagasacatctctataggatggccttattttaataaagggaaagcgggaagcttcg

SEQ ID NO: 75 - DNA, 102 bp, synthetic construct
  misc_feature 1..102: note = Epichloe festucae
  misc_feature 51: note = Variation - S is G strain AR37 or A strain RGT18
  source 1..102: mol_type = other DNA
atattataatttagtattagttattttccttaatataaatataactaggtsctagtaacctaggactaatattataagtatagccttaattatatatctaga

SEQ ID NO: 76 - DNA, 102 bp, synthetic construct
  misc_feature 1..102: note = Epichloe festucae
  misc_feature 51: note = Variation - S is C strain AR37 or T strain RGT18
  source 1..102: mol_type = other DNA
gtaaaataaaaacctatccctataagtaacctatataatagtaataaggcsttatttactatataaaagtttttaatagaatataaactataggtaaataag

SEQ ID NO: 77 - DNA, 102 bp, synthetic construct
  misc_feature 1..102: note = Epichloe festucae
  misc_feature 51: note = Vairation - S is G strain AR37 or C strain RGT18
  source 1..102: mol_type = other DNA
tctataataactataaggtattatagcctctttagagatattactagtaastttattataaagtctatagaaatctaagactagaactagttagggataagt

SEQ ID NO: 78 - DNA, 102 bp, synthetic construct
  misc_feature 1..102: note = Epichloe festucae
  misc_feature 51: note = Variation - S is C strain AR37 or A strain RGT18
  source 1..102: mol_type = other DNA
atattaaataggctcttactactagtgtcttaaactattatttaccttaasgtaaggagttatattctccttattagtagtattatattacctatatatagt

SEQ ID NO: 79 - DNA, 102 bp, synthetic construct
  misc_feature 1..102: note = Epichloe festucae
  misc_feature 51: note = Variation - S is C strain AR37 or T strain RGT18
  source 1..102: mol_type = other DNA
tacttttagaagaaactatataactaggaaaggaaactaaagatagtaaasattattaaacttacttttaaagcttatttttaaatacctttaatattaata

SEQ ID NO: 80 - DNA, 102 bp, synthetic construct
  misc_feature 1..102: note = Epichloe festucae
  misc_feature 51: note = Variation - S is T strain AR37 or C strain RGT18
  source 1..102: mol_type = other DNA
taatataactaaagaaaaaagggtattataatactagaccttaaattaaasctataattaccccttaatctagacttataattacctcttaaatattagcta

SEQ ID NO: 81 - DNA, 102 bp, synthetic construct
  misc_feature 1..102: note = Epichloe festucae
  misc_feature 51: note = Variation - S is T strain AR37 or C strain RGT18
  source 1..102: mol_type = other DNA
aatcttactttacttatattatttactcctttccttatccttctataattstaataatttctatattaactctttctctatactaatataaagtaagtttgc

SEQ ID NO: 82 - DNA, 102 bp, synthetic construct
  misc_feature 1..102: note = Epichloe festucae
  misc_feature 51: note = Variation - S is C strain AR37 or T strain RGT18
  source 1..102: mol_type = other DNA
gtttattactattattagataaatagaaaagcccttagctagtttaagttsttctttaaagataactataactttaactataagattattattaatattata

SEQ ID NO: 83 - DNA, 102 bp, synthetic construct
  misc_feature 1..102: note = Epichloe festucae
  misc_feature 51: note = Variation - S is C strain AR37 or T strain RGT18
  source 1..102: mol_type = other DNA
attaacctaaagtttagctagttaaagtaatgatttttataagaatttagsgtagctactagagaagtccctagaagaagatatagtaatgtattttatagg

SEQ ID NO: 84 - DNA, 102 bp, synthetic construct
  misc_feature 1..102: note = Epichloe festucae
  misc_feature 51: note = Variation - S is A strain AR37 or G strain RGT18
  source 1..102: mol_type = other DNA
ctagtattctctaattatatcctaaatattataagctttctatttcttagsgttaaggaattaagctacttaaaataaggttactattgaaatgtagggagc

SEQ ID NO: 85 - DNA, 102 bp, synthetic construct
  misc_feature 1..102: note = Epichloe festucae
  misc_feature 51: note = Variation - S is A strain AR37 or G strain RGT18
  source 1..102: mol_type = other DNA
acctattagggactaaattccttgctataatctataggggagaccctaaasgtatagctagcaaaagcttaataggttattgtgacagtgattttatagggg

SEQ ID NO: 86 - DNA, 102 bp, synthetic construct
  misc_feature 1..102: note = Epichloe festucae
  misc_feature 51: note = Variation - S is T strain AR37 or C strain RGT18
  source 1..102: mol_type = other DNA
agtaatattattactttataagcactttaattattatcttttttttccttsaataatattactaatagtattcttaaagcttagactactattatataggct

SEQ ID NO: 87 - DNA, 102 bp, synthetic construct
  misc_feature 1..102: note = Epichloe festucae
  misc_feature 51: note = Variation - S is A strain AR37 or G strain RGT18
  source 1..102: mol_type = other DNA
ttatatatgctattataggagttatagaaaataagtttattacccttaaasataataaggtaaaagtatataaaactattaaagatatccctaagaaactat

SEQ ID NO: 88 - DNA, 102 bp, synthetic construct
  misc_feature 1..102: note = Epichloe festucae
  misc_feature 51: note = Variation - S is G strain AR37 or A strain RGT18
  source 1..102: mol_type = other DNA
tataagtaggtgtttttattacttaataaggaaggcctaactgtttatagsgctattaagggcttctttaaagggcttaaaaattaactaggttaatatcct

SEQ ID NO: 89 - DNA, 102 bp, synthetic construct
  misc_feature 1..102: note = Epichloe festucae
  misc_feature 51: note = Variation - S is T strain AR37 or C strain RGT18
  source 1..102: mol_type = other DNA
ttttccgcaaaatttatttatatataaaatctaaaaaattaacttactacsatacaaactagcaacctatatgcactaaattttagtctaaaaaatattcct

SEQ ID NO: 90 - DNA, 102 bp, synthetic construct
  misc_feature 1..102: note = Epichloe festucae
  misc_feature 51: note = Variation - S is T strain AR37 or A strain RGT18
  source 1..102: mol_type = other DNA
ataataaggtataataaatactacttaatcctaatttaagtaaaggtatasataatataactaaagaaaaaagggtattataataatactataaggttatat

SEQ ID NO: 91 - DNA, 102 bp, synthetic construct
  misc_feature 1..102: note = Epichloe festucae
  misc_feature 51: note = Variation - S is A strain AR37 or C strain RGT18
  source 1..102: mol_type = other DNA
ttttactagtaaaagacttaaattagacttataatataattctagttattsttaactattttataatatatagtatttatattcctattttaatataactaa

SEQ ID NO: 92 - DNA, 102 bp, synthetic construct
  misc_feature 1..102: note = Epichloe festucae
  misc_feature 51: note = Variation - S is C strain AR37 or T strain RGT18
  source 1..102: mol_type = other DNA
aagttatctatagtatctaaagccctaaattatgaggctaaagtcatctasagtatccaaagccctgaattatagggctaaagacctagaaaagggtactaa

SEQ ID NO: 93 - DNA, 102 bp, synthetic construct
  misc_feature 1..102: note = Epichloe festucae
  misc_feature 51: note = Variation - S is T strain AR37 or G strain RGT18
  source 1..102: mol_type = other DNA
atataaaaagcctaagtatatattctttacgctaggtagctaattatgtasctattcctagtactccgactgcttagttaagagggaaaacccttaactagg

SEQ ID NO: 94 - DNA, 102 bp, synthetic construct
  misc_feature 1..102: note = Epichloe festucae
  misc_feature 51: note = Variation - S is A strain AR37 or C strain RGT18
  source 1..102: mol_type = other DNA
tattattatataagttacctataagaataggtttatattttaccttaggtstagttaagactaggttaaaggtaagagataaagtaaggttaattactaata

SEQ ID NO: 95 - DNA, 102 bp, synthetic construct
  misc_feature 1..102: note = Epichloe festucae
  misc_feature 51: note = Variation - S is C strain AR37 or T strain RGT18
  source 1..102: mol_type = other DNA
tctattagttaataactactatatccttccgttacgttacgttagttattstaacgtggtggttctactagtccctaactgtagagctgcacctgtacagct

SEQ ID NO: 96 - DNA, 102 bp, synthetic construct
  misc_feature 1..102: note = Epichloe festucae
  misc_feature 51: note = Variation - S is T strain AR37 or C strain RGT18
  source 1..102: mol_type = other DNA
gcactaaagagtattatatctaataagggattagtctttataagctaattstagttaaacttatattacttattatatataaagtaaaggctttttatagtg

SEQ ID NO: 97 - DNA, 102 bp, synthetic construct
  misc_feature 1..102: note = Epichloe festucae
  misc_feature 51: note = Variation - S is A strain AR37 or G strain RGT18
  source 1..102: mol_type = other DNA
ccttaaagaataaaaatcactatataaatattataattagaggtttagtgsaagaaactagggataggaattggtatttacgtagttagtaatataagtaaa

SEQ ID NO: 98 - DNA, 102 bp, synthetic construct
  misc_feature 1..102: note = Epichloe festucae
  misc_feature 51: note = Variation - S is C strain AR37 or G strain RGT18
  source 1..102: mol_type = other DNA
aataagaaactaatataatcctagtaattaatatagctaaactagtaaagstattttataaagagattaagctataatttaaagccctaaaaggcattatat

SEQ ID NO: 99 - DNA, 102 bp, synthetic construct
  misc_feature 1..102: note = Epichloe festucae
  misc_feature 51: note = Variation - S is C strain AR37 or A strain RGT18
  source 1..102: mol_type = other DNA
gaacatgatgagggttaagaagcttatgtaaatgggggattgggattgggsttgggatcatcatgtcttaaagcgaagacataccatgtaaaaatatactga

SEQ ID NO: 100 - DNA, 102 bp, synthetic construct
  misc_feature 1..102: note = Epichloe festucae
  misc_feature 51: note = Variation - S is T strain AR37 or A strain RGT18
  source 1..102: mol_type = other DNA
agtaatagaaaataagaaggtaataaatagaaaattaattttagaaaggtsaaatatattatttaatataataattctagaggacttattaagggatatata

SEQ ID NO: 101 - DNA, 102 bp, synthetic construct
  misc_feature 1..102: note = Epichloe festucae
  misc_feature 51: note = Variation - S is A strain AR37 or C strain RGT18
  source 1..102: mol_type = other DNA
ttatttagctttataaatagcaagactaactatagctttagctaataaatsaagactatatataaataccttattagattaataagcttataaaaaattcaa

SEQ ID NO: 102 - DNA, 102 bp, synthetic construct
  misc_feature 1..102: note = Epichloe festucae
  misc_feature 51: note = Variation - S is C strain AR37 or T strain RGT18
  source 1..102: mol_type = other DNA
cttatattactctttttaagaattattaatagattttattactagactttsactagtaaaagacttaaattaaacctataatataattctagttattattaa

SEQ ID NO: 103 - DNA, 102 bp, synthetic construct
  misc_feature 1..102: note = Epichloe festucae
  misc_feature 51: note = Variation - S is T strain AR37 or C strain RGT18
  source 1..102: mol_type = other DNA
gcctagggcgttctaagccactaggatttgcttaacctaatattccttaasaagtttattattaccttctatagggacctattctagtcctagataggagtc

SEQ ID NO: 104 - DNA, 102 bp, synthetic construct
  misc_feature 1..102: note = Epichloe festucae
  misc_feature 51: note = Variation - S is T strain AR37 or C strain RGT18
  source 1..102: mol_type = other DNA
agtgtgtactatataggtaattaaggaggtattctcctatactctctttcsctttctttttatttttactatagtgtactatataggtaattaaggaggtgt

SEQ ID NO: 105 - DNA, 102 bp, synthetic construct
  misc_feature 1..102: note = Epichloe festucae
  misc_feature 51: note = Variation - S is T strain AR37 or G strain RGT18
  source 1..102: mol_type = other DNA
tagtgtaagatatatatctttagattattaatattaatcttttaaccttascctttatctagaggtttaatcttatataatactaataataactttctctta

SEQ ID NO: 106 - DNA, 102 bp, synthetic construct
  misc_feature 1..102: note = Epichloe festucae
  misc_feature 51: note = Variation - S is A strain AR37 or T strain RGT18
  source 1..102: mol_type = other DNA
ggttccgaccgaacatctctcgggtgtgtactacgtgcatggcctgggggsccaaagaccacacgagattgccatgtggcctggcatatatgaagtggtgct

SEQ ID NO: 107 - DNA, 102 bp, synthetic construct
  misc_feature 1..102: note = Epichloe festucae
  misc_feature 51: note = Variation - S is T strain AR37 or C strain RGT18
  source 1..102: mol_type = other DNA
cccgcgtacagggtagcctgcttacctaattactagtgccgcggttatggstacgcttgcagctacaatgcaattgactaatccacaattaattggaattag

SEQ ID NO: 108 - DNA, 102 bp, synthetic construct
  misc_feature 1..102: note = Epichloe festucae
  misc_feature 51: note = Variation - S is A strain AR37 or G strain RGT18
  source 1..102: mol_type = other DNA
aaccctttgcactagtgtaatattccttagtgtaactaatactaattagtsgttaaatataactataaataagctaggtattataagaaaagacatttctat

SEQ ID NO: 109 - DNA, 102 bp, synthetic construct
  misc_feature 1..102: note = Epichloe festucae
  misc_feature 51: note = Variation - S is A strain AR37 or G strain RGT18
  source 1..102: mol_type = other DNA
attctctagcgttttctatttaatcctagctagttatattaaactataagsgtatctcttccttagacttcttttaagattataatatagttagtatcttaa

SEQ ID NO: 110 - DNA, 102 bp, synthetic construct
  misc_feature 1..102: note = Epichloe festucae
  misc_feature 51: note = Variation - S is T strain AR37 or C strain RGT18
  source 1..102: mol_type = other DNA
tttagctgcttttaggtgctctatatagggcctagctagtgctatagggcstagctagtgctataaatagccactaaagtgtaaaggctatgtctagcctta

SEQ ID NO: 111 - DNA, 102 bp, synthetic construct
  misc_feature 1..102: note = Epichloe festucae
  misc_feature 51: note = Variation - S is G strain AR37 or A strain RGT18
  source 1..102: mol_type = other DNA
ttagagcaaaagatctagtatatacttattatagttaattatttttcttastttatatagctatttccctataggttaactagtactataaaggtagtaaac

SEQ ID NO: 112 - DNA, 102 bp, synthetic construct
  misc_feature 1..102: note = Epichloe festucae
  misc_feature 51: note = Variation - S is T strain AR37 or C strain RGT18
  source 1..102: mol_type = other DNA
gtttataaatactaaatataattatagtatagtaaattaaaagctacttastatagtaaagttatttaaatactagtaatactatattaaagatatagtaac

SEQ ID NO: 113 - DNA, 102 bp, synthetic construct
  misc_feature 1..102: note = Epichloe festucae
  misc_feature 51: note = Variation - S is A strain AR37 or G strain RGT18
  source 1..102: mol_type = other DNA
ataatggccgccaatcggcacactggagagctcaggccagcgggctaaatsgaatatgtgggctaggcagggggggtggtggcagggggggtggtggcagca

SEQ ID NO: 114 - DNA, 102 bp, synthetic construct
  misc_feature 1..102: note = Epichloe festucae
  misc_feature 51: note = Variation - S is T strain AR37 or C strain RGT18
  source 1..102: mol_type = other DNA
ctaagtatctcctctaaaggtaatataacttagcttatataaccttatagsgttattataatgcccttttttctttagttatattatctatatctttaccta

SEQ ID NO: 115 - DNA, 102 bp, synthetic construct
  misc_feature 1..102: note = Epichloe festucae
  misc_feature 51: note = Variation - S is A strain AR37 or G strain RGT18
  source 1..102: mol_type = other DNA
ctagagctagctagcctttagctagaaataatattccttatcttactaggsttactatttttacttactattctcttactagtacttttattatacccttac

SEQ ID NO: 116 - DNA, 102 bp, synthetic construct
  misc_feature 1..102: note = Epichloe festucae
  misc_feature 51: note = Variation - S is C strain AR37 or T strain RGT18
  source 1..102: mol_type = other DNA
tttataaaatacacttataataacctaaggtattagttaaagagaaagagsactaaaactaaggctagtaactaaattaaggaattagtatattaatagaac

SEQ ID NO: 117 - DNA, 102 bp, synthetic construct
  misc_feature 1..102: note = Epichloe festucae
  misc_feature 51: note = Variation - S is A strain AR37 or C strain RGT18
  source 1..102: mol_type = other DNA
atactagtttaattagtatagacttaggaatataatcttactataaagtascttatagataataaaataagaatataagtatctttataataagataactag

SEQ ID NO: 118 - DNA, 102 bp, synthetic construct
  misc_feature 1..102: note = Epichloe festucae
  misc_feature 51: note = Variation - S is G strain AR37 or A strain RGT18
  source 1..102: mol_type = other DNA
taaagatattataaagaaaataagatattatagagaaaatagaaaataagsataagaatagtaataaatctaataaggaaaagaataagcttaacctaaaga

SEQ ID NO: 119 - DNA, 102 bp, synthetic construct
  misc_feature 1..102: note = Epichloe festucae
  misc_feature 51: note = Variation - S is C strain AR37 or T strain RGT18
  source 1..102: mol_type = other DNA
taaggtttaatattaggatgaactttaaacttataattaaagttaaggagsgtaaagataaagttatatttattaagggacttttagtagctttatctaatt

SEQ ID NO: 120 - DNA, 102 bp, synthetic construct
  misc_feature 1..102: note = Epichloe festucae
  misc_feature 51: note = Variation - S is C strain AR37 or T strain RGT18
  source 1..102: mol_type = other DNA
aatagtaaagttagggataaaagataatattataactataatagcctagastaccttataaataagtgtagtaagcgtataaagatattaaaatagtagtaa

SEQ ID NO: 121 - DNA, 102 bp, synthetic construct
  misc_feature 1..102: note = Epichloe festucae
  misc_feature 51: note = Variation - S is A strain AR37 or G strain RGT18
  source 1..102: mol_type = other DNA
tatattacatccttctaatgttccctctttctaatatatatattatatctsagttttgcttatcttatatttagagcttatttcttctttatctagtaatat

SEQ ID NO: 122 - DNA, 102 bp, synthetic construct
  misc_feature 1..102: note = Epichloe festucae
  misc_feature 51: note = Variation - S is T strain AR37 or C strain RGT18
  source 1..102: mol_type = other DNA
tatagcttaaagaaaaaccttcttattatattatttactatttttattaastattttgtatttctataaattattattattacttatttaaaaaaaacacta

SEQ ID NO: 123 - DNA, 102 bp, synthetic construct
  misc_feature 1..102: note = Epichloe festucae
  misc_feature 51: note = Variation - S is A strain AR37 or G strain RGT18
  source 1..102: mol_type = other DNA
tatagtgtaaaaaaggcagtgaattactattgcctaggctatatagcctasgttagctagctaaagctaaagaactatatatacctcctagatagctatagc

SEQ ID NO: 124 - DNA, 102 bp, synthetic construct
  misc_feature 1..102: note = Epichloe festucae
  misc_feature 51: note = Variation - S is T strain AR37 or C strain RGT18
  source 1..102: mol_type = other DNA
taacatagccttataattattatctattattttgcagtccttatatagtcsttaagtgtaatattagactaattaaactaagaaactatagttttagacgct

SEQ ID NO: 125 - DNA, 102 bp, synthetic construct
  misc_feature 1..102: note = Epichloe festucae
  misc_feature 51: note = Variation - S is C strain AR37 or T strain RGT18
  source 1..102: mol_type = other DNA
taaagcttctcttactagctacctaagagtaatataggggggagaattacstaatttactagagtaatattagtaagggtaacactataggtataaatatgc

SEQ ID NO: 126 - DNA, 102 bp, synthetic construct
  misc_feature 1..102: note = Epichloe festucae
  misc_feature 51: note = Variation - S is A strain AR37 or G strain RGT18
  source 1..102: mol_type = other DNA
ttactttagagaagactttataaaagactttataggtataagctaaataasggtaaaaaactaagataaataaggataaataataataataattagggacta

SEQ ID NO: 127 - DNA, 102 bp, synthetic construct
  misc_feature 1..102: note = Epichloe festucae
  misc_feature 51: note = Variation - S is C strain AR37 or A strain RGT18
  source 1..102: mol_type = other DNA
aaagtgttggttgtagcagcctcacatcttaggcatcactatcgcgatgtsttccctcttcgaggccttgttgcgagacctcggcacttagggcaaagactc

SEQ ID NO: 128 - DNA, 102 bp, synthetic construct
  misc_feature 1..102: note = Epichloe festucae
  misc_feature 51: note = Variation - S is A strain AR37 or G strain RGT18
  source 1..102: mol_type = other DNA
ttaagcatttaaacctatgccttaaataagtcttatctagaagtaattacstcctaattaattagtctctaggttaggaattttacttctagtagtaaaatt

SEQ ID NO: 129 - DNA, 102 bp, synthetic construct
  misc_feature 1..102: note = Epichloe festucae
  misc_feature 51: note = Variation - S is G strain AR37 or C strain RGT18
  source 1..102: mol_type = other DNA
atccttctatcctaatagttactaaattacttataataaacctcttaaatsccttatttagtaatacctttgtaaatatatttgcaaggttattatccctat

SEQ ID NO: 130 - DNA, 102 bp, synthetic construct
  misc_feature 1..102: note = Epichloe festucae
  misc_feature 51: note = Variation - S is A strain AR37 or G strain RGT18
  source 1..102: mol_type = other DNA
cacgatcccgccgccgcccacaagtatgccaccctgctaagccaattgtcsgagaagctgtccaaagatttgtgcatcatcatgcgcgcctacctcgaaaag

SEQ ID NO: 131 - DNA, 102 bp, synthetic construct
  misc_feature 1..102: note = Epichloe festucae
  misc_feature 51: note = Variation - S is A strain AR37 or G strain RGT18
  source 1..102: mol_type = other DNA
gataaggagggctaatatatagaggcctatctccttactaaatattattasgaaaattataaaagcagtgattataaaataacttatagcctttactaaggt

SEQ ID NO: 132 - DNA, 102 bp, synthetic construct
  misc_feature 1..102: note = Epichloe festucae
  misc_feature 51: note = Variation - S is T strain AR37 or C strain RGT18
  source 1..102: mol_type = other DNA
aagcttaagctaaggtaaaagctaagttacttaaagaaatccttatatatstaagaattactatctttttaatagcttaaataatactataagaaagtaaat

SEQ ID NO: 133 - DNA, 102 bp, synthetic construct
  misc_feature 1..102: note = Epichloe festucae
  misc_feature 51: note = Variation - S is C strain AR37 or T strain RGT18
  source 1..102: mol_type = other DNA
ggaaaggggattagcatactaaaccccttaactagctaatagggttatatstagaggacttataattaggactcttagggaacttactaaatctagaggaat

SEQ ID NO: 134 - DNA, 102 bp, synthetic construct
  misc_feature 1..102: note = Epichloe festucae
  misc_feature 51: note = Variation - S is C strain AR37 or A strain RGT18
  source 1..102: mol_type = other DNA
tcgtcctggcgctgctgcttactgtcttcttattcgcacttgatatggtascggattccatccacgaaagcgtcaggaagataaaccatgctgatgcttatt

SEQ ID NO: 135 - DNA, 102 bp, synthetic construct
  misc_feature 1..102: note = Epichloe festucae
  misc_feature 51: note = Variation - S is G strain AR37 or A strain RGT18
  source 1..102: mol_type = other DNA
attaataacttaatctttataagtattaaatttaatatctttaaataagcsctatagacttatagtctcctttactacctattataaagtaagtaatttagc

SEQ ID NO: 136 - DNA, 102 bp, synthetic construct
  misc_feature 1..102: note = Epichloe festucae
  misc_feature 51: note = Variation - S is T strain AR37 or C strain RGT18
  source 1..102: mol_type = other DNA
taccaatagaattgattttagtgacgttgtacaggcaatgcggtaccgacsgtattggtggatccagaccgctaaagaggtcttataggctactttttattt

SEQ ID NO: 137 - DNA, 102 bp, synthetic construct
  misc_feature 1..102: note = Epichloe festucae
  misc_feature 51: note = Variation - S is G strain AR37 or A strain RGT18
  source 1..102: mol_type = other DNA
cctagggctaggtttacgtgacactagtaagccgctagctataagatagtsacttatatgtataatatatttagacttagtaagctttagttaatatactaa

SEQ ID NO: 138 - DNA, 102 bp, synthetic construct
  misc_feature 1..102: note = Epichloe festucae
  misc_feature 51: note = Variation - S is A strain AR37 or G strain RGT18
  source 1..102: mol_type = other DNA
tctagggatagtcctagctgctaacttctaggctttaggttatttttctasggggattagaatcttatagtgagatcctatggctctaatactgctaatatt

SEQ ID NO: 139 - DNA, 102 bp, synthetic construct
  misc_feature 1..102: note = Epichloe festucae
  misc_feature 51: note = Variation - S is T strain AR37 or C strain RGT18
  source 1..102: mol_type = other DNA
gacccctaataagggggtaggctattagctctagccttattaaaaaggtcsgtgaagttagctaactccttaggtaatattaacgtgtctaggctattaggc

SEQ ID NO: 140 - DNA, 102 bp, synthetic construct
  misc_feature 1..102: note = Epichloe festucae
  misc_feature 51: note = Variation - S is T strain AR37 or C strain RGT18
  source 1..102: mol_type = other DNA
tttaactattatactattatagaaagctactactactatttttacctagcsctttactcttcttattgctctatattctattagattaatagtaatctaata

SEQ ID NO: 141 - DNA, 102 bp, synthetic construct
  misc_feature 1..102: note = Epichloe festucae
  misc_feature 51: note = Variation - S is C strain AR37 or T strain RGT18
  source 1..102: mol_type = other DNA
attattactttatatgtaactacctatatatactaccttagttatattatscttaaaggtatagtagtttaatttaaataatatatttaagtttactaagaa

SEQ ID NO: 142 - DNA, 102 bp, synthetic construct
  misc_feature 1..102: note = Epichloe festucae
  misc_feature 51: note = Variation - S is T strain AR37 or A strain RGT18
  source 1..102: mol_type = other DNA
tctcgtcgtgtgaaattcaagatgctcccgacttccgtgttctggggactsgccatcttttataagtccatcgatgaataatttattaatcaatcaatcggc

SEQ ID NO: 143 - DNA, 102 bp, synthetic construct
  misc_feature 1..102: note = Epichloe festucae
  misc_feature 51: note = Variation - S is G strain AR37 or A strain RGT18
  source 1..102: mol_type = other DNA
taactttatatctagatattcgatcttagctaaaccctctaaaacctattscctagctatataaggcagggttataagtagtggttatagcgccttaattat

SEQ ID NO: 144 - DNA, 102 bp, synthetic construct
  misc_feature 1..102: note = Epichloe festucae
  misc_feature 51: note = Variation - S is G strain AR37 or A strain RGT18
  source 1..102: mol_type = other DNA
taagtaatctaaggtatatagctagaaaaccacactataagcttaacctasaaataaataaaagggagcttataaagttacttactcttatatttactttag

SEQ ID NO: 145 - DNA, 102 bp, synthetic construct
  misc_feature 1..102: note = Epichloe festucae
  misc_feature 51: note = Variation - S is C strain AR37 or T strain RGT18
  source 1..102: mol_type = other DNA
atctctaatactttatagctaataactaataaatatagcttaagttacttstaatagcttaatttacttataataatatagtaaataagactataagctact

SEQ ID NO: 146 - DNA, 102 bp, synthetic construct
  misc_feature 1..102: note = Epichloe festucae
  misc_feature 51: note = Variation - S is A strain AR37 or T strain RGT18
  source 1..102: mol_type = other DNA
gagttagctaacttcgcggacctttttaataaggctagagctaatagcctscccccttattagggatcccttaattaccacatacacttgcgtaagaattag

SEQ ID NO: 147 - DNA, 102 bp, synthetic construct
  misc_feature 1..102: note = Epichloe festucae
  misc_feature 51: note = Variation - S is T strain AR37 or C strain RGT18
  source 1..102: mol_type = other DNA
aacgggcgcagtgactttggtgaggggcgggctcccaacgttggccgcagsgatccaatcaaaaccagctgcggttgggcaacgccttccctttggcgcaag

SEQ ID NO: 148 - DNA, 102 bp, synthetic construct
  misc_feature 1..102: note = Epichloe festucae
  misc_feature 51: note = Variation - S is T strain AR37 or C strain RGT18
  source 1..102: mol_type = other DNA
aatactcttatagaaaaagcctagccttattagctactattatactttaastaatagtctaggaattactactaaaaaataaaagaaaaaagccctaaaggt

SEQ ID NO: 149 - DNA, 102 bp, synthetic construct
  misc_feature 1..102: note = Epichloe festucae
  misc_feature 51: note = Variation - S is G strain AR37 or A strain RGT18
  source 1..102: mol_type = other DNA
tataaagggattattaatttaataataaacctctctaaggtttataagaasgttacttaataggtaaatattttataagagttaaatatagaatatatatac

SEQ ID NO: 150 - DNA, 102 bp, synthetic construct
  misc_feature 1..102: note = Epichloe festucae
  misc_feature 51: note = Variation - S is A strain AR37 or G strain RGT18
  source 1..102: mol_type = other DNA
aataaaggcattctttagcttattaaagatattattctctttaggttcttsttaaaaagaggtatttctcttagttaattatattagtaatgctactagctc

SEQ ID NO: 151 - DNA, 102 bp, synthetic construct
  misc_feature 1..102: note = Epichloe festucae
  misc_feature 51: note = Variation - S is A strain AR37 or G strain RGT18
  source 1..102: mol_type = other DNA
tcgctaacttctagtaaaactttaacttagctactaaggctatgtaactasagagcttaatattaactaaaactttattaatattaattaaataactagaga

SEQ ID NO: 152 - DNA, 102 bp, synthetic construct
  misc_feature 1..102: note = Epichloe festucae
  misc_feature 51: note = Variation - S is T strain AR37 or C strain RGT18
  source 1..102: mol_type = other DNA
ttaaattattatgctaacttaaatataattataagctaccctaactatacstaatattatttagtactagggaagtaatactaataaggtctatactttatt

SEQ ID NO: 153 - DNA, 102 bp, synthetic construct
  misc_feature 1..102: note = Epichloe festucae
  misc_feature 51: note = Variation - S is A strain AR37 or G strain RGT18
  source 1..102: mol_type = other DNA
taattactttaaaagctaagaataaagatatatatatattaattactatasactatataataaggtttatattaagataatcctatataaaggtaactagag

SEQ ID NO: 154 - DNA, 102 bp, synthetic construct
  misc_feature 1..102: note = Epichloe festucae
  misc_feature 51: note = Variation - S is A strain AR37 or G strain RGT18
  source 1..102: mol_type = other DNA
cctaatccttaggagtagcctttagcttataaagctttaaataaattatasgattcctattactttaaggtatctttaatattataactagagtatctaggg

SEQ ID NO: 155 - DNA, 102 bp, synthetic construct
  misc_feature 1..102: note = Epichloe festucae
  misc_feature 51: note = Variation - S is A strain AR37 or G strain RGT18
  source 1..102: mol_type = other DNA
tattaagttctatagttattagattaatcatttaattatttagttatttasttatttagttatttagttatttagttatttagttatttagttatttagtta

SEQ ID NO: 156 - DNA, 102 bp, synthetic construct
  misc_feature 1..102: note = Epichloe festucae
  misc_feature 51: note = Variation - S is A strain AR37 or G strain RGT18
  source 1..102: mol_type = other DNA
taatattatatatatatattctttacactagatagctaattatgtagctastcctagtactccatccgcttagtcaagagggaaaaccctatataataatat

SEQ ID NO: 157 - DNA, 102 bp, synthetic construct
  misc_feature 1..102: note = Epichloe festucae
  misc_feature 51: note = Variation - S is G strain AR37 or A strain RGT18
  source 1..102: mol_type = other DNA
gctagaatattataatataatggatactatagctagaatattataatatasttatttatatagtaaaacagtaattagttattaaagtagtaaagggcttat

SEQ ID NO: 158 - DNA, 102 bp, synthetic construct
  misc_feature 1..102: note = Epichloe festucae
  misc_feature 51: note = Variation - S is T strain AR37 or C strain RGT18
  source 1..102: mol_type = other DNA
tactttaagataaaaaaccttattttaactttactactttattatgtaatstaattactaagtaagttaaatttagcttactatataaataacttagctata

SEQ ID NO: 159 - DNA, 102 bp, synthetic construct
  misc_feature 1..102: note = Epichloe festucae
  misc_feature 51: note = Variation - S is A strain AR37 or G strain RGT18
  source 1..102: mol_type = other DNA
actaattcttatagttctaatactataatagtctttaggtttatttatagsacttatattctagtttattaatatactagatataagtaataataagatttt

SEQ ID NO: 160 - DNA, 102 bp, synthetic construct
  misc_feature 1..102: note = Epichloe festucae
  misc_feature 51: note = Variation - S is A strain AR37 or G strain RGT18
  source 1..102: mol_type = other DNA
atatatataaaagggtctagtagctttaatctatcctattaaatctagctstttactattaacttttttcctttattattactattctataggcagattaag

SEQ ID NO: 161 - DNA, 102 bp, synthetic construct
  misc_feature 1..102: note = Epichloe festucae
  misc_feature 51: note = Variation - S is G strain AR37 or A strain RGT18
  source 1..102: mol_type = other DNA
ctataatataaattatctacttattattatactagataattaatagagaasggacctatatgctaatattataaagtaatttacctagagatatacgctctt

SEQ ID NO: 162 - DNA, 102 bp, synthetic construct
  misc_feature 1..102: note = Epichloe festucae
  misc_feature 51: note = Variation - S is C strain AR37 or A strain RGT18
  source 1..102: mol_type = other DNA
aagtagcctaattccttaaccttaagaagtaaaaagcttataatatttagsatataattaaagagtgctagattaatatatatctaggccctctagactaga

SEQ ID NO: 163 - DNA, 102 bp, synthetic construct
  misc_feature 1..102: note = Epichloe festucae
  misc_feature 51: note = Variation - S is G strain AR37 or T strain RGT18
  source 1..102: mol_type = other DNA
gctatagctatataggggtaaagctaccctaggaatatatctttagaaaasgaacttattaaggctaatctttcctatatatagttatattattataaaaga

SEQ ID NO: 164 - DNA, 102 bp, synthetic construct
  misc_feature 1..102: note = Epichloe festucae
  misc_feature 51: note = Variation - S is A strain AR37 or G strain RGT18
  source 1..102: mol_type = other DNA
taggaaggggcctagaggtttcctattaagacacttataagagaataggtsgtaaattactctataaggcacttataagagagtaagtagtaaattgttcta

SEQ ID NO: 165 - DNA, 102 bp, synthetic construct
  misc_feature 1..102: note = Epichloe festucae
  misc_feature 51: note = Variation - S is T strain AR37 or A strain RGT18
  source 1..102: mol_type = other DNA
ggaaacttaagggtaaatataagagggaaagcatagaagtaaactctaggsgtagctttagtataaggggtaggctagtttatcttactaaccccttccact

SEQ ID NO: 166 - DNA, 102 bp, synthetic construct
  misc_feature 1..102: note = Epichloe festucae
  misc_feature 51: note = Variation - S is T strain AR37 or C strain RGT18
  source 1..102: mol_type = other DNA
gagttttaggtctttaccccctatataaaataataaatatattaagggaastattagctagctaggcttataggctaataccctagggagtaattagtctat

SEQ ID NO: 167 - DNA, 102 bp, synthetic construct
  misc_feature 1..102: note = Epichloe festucae
  misc_feature 51: note = Variation - S is T strain AR37 or C strain RGT18
  source 1..102: mol_type = other DNA
tcgttattaataatattagggataaacttctaagctatcttttaaatatasgattcctataataactatatctctttagtattatgattcctaatgatttta

SEQ ID NO: 168 - DNA, 102 bp, synthetic construct
  misc_feature 1..102: note = Epichloe festucae
  misc_feature 51: note = Variation - S is C strain AR37 or T strain RGT18
  source 1..102: mol_type = other DNA
atacaaaacaccatagatataagggtaattttgcctactagatagtagccsttaattaatctagaatagtataaatagaacgttttgctaatctattttgct

SEQ ID NO: 169 - DNA, 102 bp, synthetic construct
  misc_feature 1..102: note = Epichloe festucae
  misc_feature 51: note = Variation - S is A strain AR37 or T strain RGT18
  source 1..102: mol_type = other DNA
agtatcattagctataaagaatagttagtacttaatacctaatagtatatsgttagtaacttacctagtggaattttagttatattgtaatttattactagt

SEQ ID NO: 170 - DNA, 102 bp, synthetic construct
  misc_feature 1..102: note = Epichloe festucae
  misc_feature 51: note = Variation - S is G strain AR37 or C strain RGT18
  source 1..102: mol_type = other DNA
gggtacttactttaagtgtaaagttactagatattatactataaactatastataactagaaataatttattataataataggaatccttatagttaaaatt

SEQ ID NO: 171 - DNA, 102 bp, synthetic construct
  misc_feature 1..102: note = Epichloe festucae
  misc_feature 51: note = Variation - S is T strain AR37 or C strain RGT18
  source 1..102: mol_type = other DNA
taactatagtatttacctctttacctttaacttctataagtaataaattasatatagttagcttcttaattattactatctccttaagtttatatagtctta

SEQ ID NO: 172 - DNA, 102 bp, synthetic construct
  misc_feature 1..102: note = Epichloe festucae
  misc_feature 51: note = Variation - S is G strain AR37 or A strain RGT18
  source 1..102: mol_type = other DNA
acgtgtatgcaaacacttccaaaaacgatgcgcagaatggagctcctgatstttgaggaacatctcgtggtctactagggcactgggacaattattggctgt

SEQ ID NO: 173 - DNA, 102 bp, synthetic construct
  misc_feature 1..102: note = Epichloe festucae
  misc_feature 51: note = Variation - S is G strain AR37 or A strain RGT18
  source 1..102: mol_type = other DNA
ttgtaaaggaaactagctattttaataaaagttttaagacttaataaattscttagaaaaatcattttttaaaaggctttaagtctattattagtgttaata

SEQ ID NO: 174 - DNA, 102 bp, synthetic construct
  misc_feature 1..102: note = Epichloe festucae
  misc_feature 51: note = Variation - S is G strain AR37 or T strain RGT18
  source 1..102: mol_type = other DNA
atagctatagggtaacctgcgtacagggtagcctgcttacctaattactastggcgtggttatggctgcgcttgcagccataacgcaattgactaatccaca

SEQ ID NO: 175 - DNA, 102 bp, synthetic construct
  misc_feature 1..102: note = Epichloe festucae
  misc_feature 51: note = Variation - S is C strain AR37 or T strain RGT18
  source 1..102: mol_type = other DNA
cctaaggtaatattttccctttttttaatttaatagtataagtataacctsttagtttaaaaagcttacttactaactctttagaaaaaatatttataaact

SEQ ID NO: 176 - DNA, 102 bp, synthetic construct
  misc_feature 1..102: note = Epichloe festucae
  misc_feature 51: note = Variation - S is A strain AR37 or T strain RGT18
  source 1..102: mol_type = other DNA
gggggatcgaagtcatgccgtcggttcccggtcagtaacttgggggccacscgcgcaaatgcaatgtagtgtccactttgaagcgagtcgcctctatgacaa

SEQ ID NO: 177 - DNA, 102 bp, synthetic construct
  misc_feature 1..102: note = Epichloe festucae
  misc_feature 51: note = Variation - S is A strain AR37 or G strain RGT18
  source 1..102: mol_type = other DNA
ttaaattcaatacctataaagattaggttattaattataataattaataastaatttagcttatacttaataagagtaaataattaaatacttaactatatt

SEQ ID NO: 178 - DNA, 102 bp, synthetic construct
  misc_feature 1..102: note = Epichloe festucae
  misc_feature 51: note = Variation - S is A strain AR37 or G strain RGT18
  source 1..102: mol_type = other DNA
aactagattaaactaggaaaaaacccctattatacacttattctaagttasaataaatatcttctgaagattcattagaagaatctttagagatattctagt

SEQ ID NO: 179 - DNA, 102 bp, synthetic construct
  misc_feature 1..102: note = Epichloe festucae
  misc_feature 51: note = Variation - S is A strain AR37 or G strain RGT18
  source 1..102: mol_type = other DNA
accttaatactaaggctcctatactaattttatataggagttttttattasgtattcctaaggccttaatactagattacatataaaatattaagttaatag

SEQ ID NO: 180 - DNA, 102 bp, synthetic construct
  misc_feature 1..102: note = Epichloe festucae
  misc_feature 51: note = Variation - S is A strain AR37 or G strain RGT18
  source 1..102: mol_type = other DNA
ctgctattagtgcggctgccccgtattttaaatccactccctctgctgtgscttaccactacatataactttatggagttaaatgtgaatattagaagcatt

SEQ ID NO: 181 - DNA, 102 bp, synthetic construct
  misc_feature 1..102: note = Epichloe festucae
  misc_feature 51: note = Variation - S is G strain AR37 or A strain RGT18
  source 1..102: mol_type = other DNA
agtttttttcttttaaataattatttcctttactaaaatgccttaatactsaactaatgcccttacttctatagctttagtagctactcctatagttactct

SEQ ID NO: 182 - DNA, 102 bp, synthetic construct
  misc_feature 1..102: note = Epichloe festucae
  misc_feature 51: note = Variation - S is T strain AR37 or C strain RGT18
  source 1..102: mol_type = other DNA
atatttacttataaagtgtttaattatatatattaaccttattattaaaasaaataaaatctagtatagcttttaggttatagtatagatttatataaggtt

SEQ ID NO: 183 - DNA, 102 bp, synthetic construct
  misc_feature 1..102: note = Epichloe festucae
  misc_feature 51: note = Variation - S is G strain AR37 or A strain RGT18
  source 1..102: mol_type = other DNA
aattaggttataatacttaagaattaggctttttaatatgccttacttaastaaaagctataccttaaagagccttttaataaggatattttaatttattat

SEQ ID NO: 184 - DNA, 102 bp, synthetic construct
  misc_feature 1..102: note = Epichloe festucae
  misc_feature 51: note = Variation - S is A strain AR37 or G strain RGT18
  source 1..102: mol_type = other DNA
ctactctggtgccaatctgctgaaccaggtccttgagagcctgttgagcastctcctgaggaccagtggcatcaaaccgaaggcggccattggatgccgtag

SEQ ID NO: 185 - DNA, 102 bp, synthetic construct
  misc_feature 1..102: note = Epichloe festucae
  misc_feature 51: note = Variation - S is A strain AR37 or G strain RGT18
  source 1..102: mol_type = other DNA
ctatattctctaaatattatataaatactagtatacacttatagattattsttatagactttgcatttgctataattccttaacctttcttatccttaatac

SEQ ID NO: 186 - DNA, 102 bp, synthetic construct
  misc_feature 1..102: note = Epichloe festucae
  misc_feature 51: note = Variation - S is C strain AR37 or T strain RGT18
  source 1..102: mol_type = other DNA
aatatcttagtttacttaggggaattaaggaaaaactatatagctaaggtstagctaatattaggctatctaagagctataggtttatacttagatcttaat

SEQ ID NO: 187 - DNA, 102 bp, synthetic construct
  misc_feature 1..102: note = Epichloe festucae
  misc_feature 51: note = Variation - S is G strain AR37 or C strain RGT18
  source 1..102: mol_type = other DNA
ataaaaagtaactaattaatcctaactaaggagtataatattatctaaaastttcctaattaatctaaactataatctataataattaattaaggaaacccc

SEQ ID NO: 188 - DNA, 102 bp, synthetic construct
  misc_feature 1..102: note = Epichloe festucae
  misc_feature 51: note = Variation - S is A strain AR37 or G strain RGT18
  source 1..102: mol_type = other DNA
tatggccaaagtgtaagtctactaaagggatacacgtaatgtaattagctscattataggtaaccctatactatttatagtggctttacactactaccttac

SEQ ID NO: 189 - DNA, 102 bp, synthetic construct
  misc_feature 1..102: note = Epichloe festucae
  misc_feature 51: note = Variation - S is C strain AR37 or T strain RGT18
  source 1..102: mol_type = other DNA
agctatatttaataatagctaggattaaaaaggaggtcttttatcttttcstgtttttcccttttatctatttttatctaaaagttattgtttaccctatag

SEQ ID NO: 190 - DNA, 102 bp, synthetic construct
  misc_feature 1..102: note = Epichloe festucae
  misc_feature 51: note = Variation - S is A strain AR37 or C strain RGT18
  source 1..102: mol_type = other DNA
tataattagtttaaataaataaggtacctaatactatagttttaaatagtstaactaaagggcttatattatagttactataagtttatagctattaggcat

SEQ ID NO: 191 - DNA, 102 bp, synthetic construct
  misc_feature 1..102: note = Epichloe festucae
  misc_feature 51: note = Variation - S is G strain AR37 or A strain RGT18
  source 1..102: mol_type = other DNA
tatagatttatataatatctataaagcttatatttaacttctagtgtaatstttttatgttttacttaatatgtctaagagtccggaggaagccacagtttg

SEQ ID NO: 192 - DNA, 102 bp, synthetic construct
  misc_feature 1..102: note = Epichloe festucae
  misc_feature 51: note = Variation - S is G strain AR37 or A strain RGT18
  source 1..102: mol_type = other DNA
cttatttatttaaaatctttaaaattactaatctaagactagtaatctttsctagatttactactaatagtagtagggttagctttttcctttccttttccc

SEQ ID NO: 193 - DNA, 102 bp, synthetic construct
  misc_feature 1..102: note = Epichloe festucae
  misc_feature 51: note = Variation - S is A strain AR37 or T strain RGT18
  source 1..102: mol_type = other DNA
atcttataaaagagtaattacttaactaaatattataatactagtaagatsttcttagagaaagacttttaataaggtaatatttatagtaataagtaacct

SEQ ID NO: 194 - DNA, 102 bp, synthetic construct
  misc_feature 1..102: note = Epichloe festucae
  misc_feature 51: note = Variation - S is T strain AR37 or C strain RGT18
  source 1..102: mol_type = other DNA
acattgcacatgcctagcatatgcttagcatatggctagcattagcctagsatatgctaactatatgtaaaattttcttaaagatcttaaatatacataaag

SEQ ID NO: 195 - DNA, 102 bp, synthetic construct
  misc_feature 1..102: note = Epichloe festucae
  misc_feature 51: note = Variation - S is T strain AR37 or C strain RGT18
  source 1..102: mol_type = other DNA
atttaactagtagcctctccctaatattgcgtttatttcgaaatagcgctscttatctagattaaataaacctatataatttgtctaataagtttattatta

SEQ ID NO: 196 - DNA, 102 bp, synthetic construct
  misc_feature 1..102: note = Epichloe festucae
  misc_feature 51: note = Variation - S is C strain AR37 or A strain RGT18
  source 1..102: mol_type = other DNA
tatagctagcttcttactaggttatcttaggttaatattctttattaatastaaaatatagttactaactttaaaccttattagagttctcttctagttata

SEQ ID NO: 197 - DNA, 102 bp, synthetic construct
  misc_feature 1..102: note = Epichloe festucae
  misc_feature 51: note = Variation - S is C strain AR37 or T strain RGT18
  source 1..102: mol_type = other DNA
taaagctttggttaaagcattagttataatctctctaattataacattagstataatccctttaattaacgccttagttgtaatctctttaattaatgcttt

SEQ ID NO: 198 - DNA, 102 bp, synthetic construct
  misc_feature 1..102: note = Epichloe festucae
  misc_feature 51: note = Variation - S is T strain AR37 or C strain RGT18
  source 1..102: mol_type = other DNA
tatataaagaaatatataaatagtttactacccttatttaagtgcttaccscttattactatagtaagaactagtattattattaaattactaagttaagta

SEQ ID NO: 199 - DNA, 102 bp, synthetic construct
  misc_feature 1..102: note = Epichloe festucae
  misc_feature 51: note = Variation - S is G strain AR37 or A strain RGT18
  source 1..102: mol_type = other DNA
aagtacttatacttatttacttaactctatttatacgtaaatttattctasgaaggttagacttagtaattactattaaaagggctttcttttataagatcc

SEQ ID NO: 200 - DNA, 102 bp, synthetic construct
  misc_feature 1..102: note = Epichloe festucae
  misc_feature 51: note = Variation - S is C strain AR37 or T strain RGT18
  source 1..102: mol_type = other DNA
gcgtatatattagaataaagagtaattaagctctcttagaagtaaagattstctttagcctaagcgtatatattagaatttatattaattaaaatataagct

SEQ ID NO: 201 - DNA, 102 bp, synthetic construct
  misc_feature 1..102: note = Epichloe festucae
  misc_feature 51: note = Variation - S is G strain AR37 or A strain RGT18
  source 1..102: mol_type = other DNA
agacggtcagattaattggtctaacaacggaagctttcgttaacggcagasgccttattagaagaccttctgtacgtcagattcccctttaaaagtcggaag

SEQ ID NO: 202 - DNA, 102 bp, synthetic construct
  misc_feature 1..102: note = Epichloe festucae
  misc_feature 51: note = Variation - S is T strain AR37 or C strain RGT18
  source 1..102: mol_type = other DNA
aaggtattagtaatattaaactccctattagcaaaggctatttagaactasctaatacttaataggcactaaaggctaaagttaatataattttactaggcc

SEQ ID NO: 203 - DNA, 102 bp, synthetic construct
  misc_feature 1..102: note = Epichloe festucae
  misc_feature 51: note = Variation - S is C strain AR37 or T strain RGT18
  source 1..102: mol_type = other DNA
gatattaaacgcaatgcaggaagctgcattattaattaaagagaggataasaagagtgatgcctaatatctaaggctataatataaggctgtgaatatcctt

SEQ ID NO: 204 - DNA, 102 bp, synthetic construct
  misc_feature 1..102: note = Epichloe festucae
  misc_feature 51: note = Variation - S is A strain AR37 or G strain RGT18
  source 1..102: mol_type = other DNA
tccgtaactataagctaacctaatagttaattctattatattaaagctagsatctaaatataaaggtatcctacttatatttacttataaagtgtttaatta

SEQ ID NO: 205 - DNA, 102 bp, synthetic construct
  misc_feature 1..102: note = Epichloe festucae
  misc_feature 51: note = Variation - S is C strain AR37 or T strain RGT18
  source 1..102: mol_type = other DNA
actagatttagactttagataaaaagaattaactttctttagatatcttascttatacctaatagtagctcttatagtaaacttagtataaccttataatag

SEQ ID NO: 206 - DNA, 102 bp, synthetic construct
  misc_feature 1..102: note = Epichloe festucae
  misc_feature 51: note = Variation - S is T strain AR37 or C strain RGT18
  source 1..102: mol_type = other DNA
ataatttaatatgctttagagcctttattattattagaaacgccttatatstataagcttatagatatataattaagggcttttaaacttctaatatctata

SEQ ID NO: 207 - DNA, 102 bp, synthetic construct
  misc_feature 1..102: note = Epichloe festucae
  misc_feature 51: note = Variation - S is A strain AR37 or T strain RGT18
  source 1..102: mol_type = other DNA
tttattattctagtttttagctattttagaaaatttacctaggtaattaasaaataatttatatacttatttatagctatataatatatttattattacttt

SEQ ID NO: 208 - DNA, 102 bp, synthetic construct
  misc_feature 1..102: note = Epichloe festucae
  misc_feature 51: note = Variation - S is T strain AR37 or C strain RGT18
  source 1..102: mol_type = other DNA
agttagtaatatctaaatagcagcctatacatagctttaatatagtaaaasaaatgttattacctattatatagctagaagaaaaaaaaatagataacctat

SEQ ID NO: 209 - DNA, 102 bp, synthetic construct
  misc_feature 1..102: note = Epichloe festucae
  misc_feature 51: note = Variation - S is G strain AR37 or A strain RGT18
  source 1..102: mol_type = other DNA
agatacttatcctatcctagagatactactatctcctatcctatcttagasatattactatcttattagttactaaaatactctccttaactaagtgtagtt

SEQ ID NO: 210 - DNA, 102 bp, synthetic construct
  misc_feature 1..102: note = Epichloe festucae
  misc_feature 51: note = Variation - S is A strain AR37 or G strain RGT18
  source 1..102: mol_type = other DNA
agaaaatagggcttttatttaatgcaggaatattttttagactaaaagttsgtgtatataggttactagtttgtatagtggtaagttaattttttagatttt

SEQ ID NO: 211 - DNA, 102 bp, synthetic construct
  misc_feature 1..102: note = Epichloe festucae
  misc_feature 51: note = Variation - S is T strain AR37 or C strain RGT18
  source 1..102: mol_type = other DNA
agagatatataagccctttactactctaataactaattactattttactasataaataaccatattataatattctagctatagtatccctagtattatatc

SEQ ID NO: 212 - DNA, 102 bp, synthetic construct
  misc_feature 1..102: note = Epichloe festucae
  misc_feature 51: note = Variation - S is A strain AR37 or G strain RGT18
  source 1..102: mol_type = other DNA
gatttaatatattataaatagctttagttattactatagtaataaagtaasagagccttaaggaagtatataaactaattttaaaattcttagtatatagag

SEQ ID NO: 213 - DNA, 102 bp, synthetic construct
  misc_feature 1..102: note = Epichloe festucae
  misc_feature 51: note = Variation - S is T strain AR37 or C strain RGT18
  source 1..102: mol_type = other DNA
attataagatatattctctagtttatacttactaagttattttaagaaaastactagaatatatattactaaggctattttagagaatctattaggatcttt

SEQ ID NO: 214 - DNA, 102 bp, synthetic construct
  misc_feature 1..102: note = Epichloe festucae
  misc_feature 51: note = Variation - S is T strain AR37 or A strain RGT18
  source 1..102: mol_type = other DNA
taaaaagaaaaaaatagataacttatattaatttttataattagtttaaasaaataaagtacctaatactatagttttaaatagtctaactaaagggcttat

SEQ ID NO: 215 - DNA, 102 bp, synthetic construct
  misc_feature 1..102: note = Epichloe festucae
  misc_feature 51: note = Variation - S is T strain AR37 or A strain RGT18
  source 1..102: mol_type = other DNA
taattttatagtaattatatacagttatagttatagtagttaactataatstaatactagttttcttttacctagctatagctatagaaaggtaatgctacc

SEQ ID NO: 216 - DNA, 102 bp, synthetic construct
  misc_feature 1..102: note = Epichloe festucae
  misc_feature 51: note = Variation - S is C strain AR37 or T strain RGT18
  source 1..102: mol_type = other DNA
taaactaaggttttatatttactagtggtttttaaataactttttattatsttcttataactaagtagctacttagctttattattttcttataactaagta

SEQ ID NO: 217 - DNA, 102 bp, synthetic construct
  misc_feature 1..102: note = Epichloe festucae
  misc_feature 51: note = Variation - S is G strain AR37 or A strain RGT18
  source 1..102: mol_type = other DNA
tatctatattataggtaatagcctagattatacctattatattagcgtgcstatgtttaatataatgctaccttataacactcttactaattatactaagct

SEQ ID NO: 218 - DNA, 102 bp, synthetic construct
  misc_feature 1..102: note = Epichloe festucae
  misc_feature 51: note = Variation - S is G strain AR37 or T strain RGT18
  source 1..102: mol_type = other DNA
atttttagcccttttctagttaaaggacctttttattactagcttgcatcscaagcctaacagctgcactgcagctgttaacggtcacgcaggtaactgtca

SEQ ID NO: 219 - DNA, 102 bp, synthetic construct
  misc_feature 1..102: note = Epichloe festucae
  misc_feature 51: note = Variation - S is C strain AR37 or T strain RGT18
  source 1..102: mol_type = other DNA
tagaaagagagaattactaaacttaatataggtaaaatactaattaaattsaataaataaattaatactttaaaataaagcatagtttaaaaggataagtat

SEQ ID NO: 220 - DNA, 102 bp, synthetic construct
  misc_feature 1..102: note = Epichloe festucae
  misc_feature 51: note = Variation - S is A strain AR37 or G strain RGT18
  source 1..102: mol_type = other DNA
tccctttataattcttattagtcttttctaaaggtatattaataactagcsctagtccctttataatttctattagtcttttctaaagataactattctcta

SEQ ID NO: 221 - DNA, 102 bp, synthetic construct
  misc_feature 1..102: note = Epichloe festucae
  misc_feature 51: note = Variation - S is T strain AR37 or A strain RGT18
  source 1..102: mol_type = other DNA
caagcctctttaacctcttatttttctatgaaaaggccttaaaataatacsattatagaggaattttcatctaaaaaggctattactctagttattaagttt

SEQ ID NO: 222 - DNA, 102 bp, synthetic construct
  misc_feature 1..102: note = Epichloe festucae
  misc_feature 51: note = Variation - S is A strain AR37 or G strain RGT18
  source 1..102: mol_type = other DNA
ctttaaacgctatagatagctctaaagggaattagaatatagttatctatsattctagagctaatgtttatatttttaataatatttattagtttaaatagt

SEQ ID NO: 223 - DNA, 102 bp, synthetic construct
  misc_feature 1..102: note = Epichloe festucae
  misc_feature 51: note = Variation - S is T strain AR37 or A strain RGT18
  source 1..102: mol_type = other DNA
atttatctaataaaaggttctttacctttataactattttattataattasaagtaattactttaattttttagtcttttttacttaaaagaaaagtaaaaa

SEQ ID NO: 224 - DNA, 102 bp, synthetic construct
  misc_feature 1..102: note = Epichloe festucae
  misc_feature 51: note = Variation - S is T strain AR37 or C strain RGT18
  source 1..102: mol_type = other DNA
ataagaccagattcagtatcttaccttatacctaatagtagctcttatagsaaacttagtataaccttataatagtaaatccattagcctctctaatagatt

SEQ ID NO: 225 - DNA, 102 bp, synthetic construct
  misc_feature 1..102: note = Epichloe festucae
  misc_feature 51: note = Variation - S is G strain AR37 or A strain RGT18
  source 1..102: mol_type = other DNA
ttagataaatcctatatctatatgcctttcctagataatattatagtaaasggactaataataatatataataagaaggaaattatgctaggagtatataaa

SEQ ID NO: 226 - DNA, 102 bp, synthetic construct
  misc_feature 1..102: note = Epichloe festucae
  misc_feature 51: note = Variation - S is C strain AR37 or T strain RGT18
  source 1..102: mol_type = other DNA
atataaaggaaactataatatatagtattacctatacctcttagtttactstctttatattactattagtctataggtaatataatatagaaagtaactaat

SEQ ID NO: 227 - DNA, 102 bp, synthetic construct
  misc_feature 1..102: note = Epichloe festucae
  misc_feature 51: note = Variation - S is T strain AR37 or C strain RGT18
  source 1..102: mol_type = other DNA
tataagtacttaaaatagtctagtaaatctaggggttagcttttattttasatccttaagcctaatgttctttgctaataatagtactaggttacctctttt

SEQ ID NO: 228 - DNA, 102 bp, synthetic construct
  misc_feature 1..102: note = Epichloe festucae
  misc_feature 51: note = Variation - S is A strain AR37 or T strain RGT18
  source 1..102: mol_type = other DNA
gtgtatataggaggatttattatttatagaagagagtttacttaggtatasaaggcttagttcttaaaccataaaaataacacttaaatttagtttctaata

SEQ ID NO: 229 - DNA, 102 bp, synthetic construct
  misc_feature 1..102: note = Epichloe festucae
  misc_feature 51: note = Variation - S is T strain AR37 or G strain RGT18
  source 1..102: mol_type = other DNA
cttagataaagcctagatttagtaggaattttattaggtataaaaactatsattaaggagcttcctatagcctatataatactcttattattttctagagat

SEQ ID NO: 230 - DNA, 102 bp, synthetic construct
  misc_feature 1..102: note = Epichloe festucae
  misc_feature 51: note = Variation - S is T strain AR37 or G strain RGT18
  source 1..102: mol_type = other DNA
tatatttaatttttatattctagggatagcttataaaactaaaattactasatattttatagtaatagtaaatataatactaaatctaagactaaaattatt

SEQ ID NO: 231 - DNA, 102 bp, synthetic construct
  misc_feature 1..102: note = Epichloe festucae
  misc_feature 51: note = Variation - S is T strain AR37 or C strain RGT18
  source 1..102: mol_type = other DNA
aataaacaggctagctagctataagatagctatatgcttataaagcagggsatttattaaagactatgtatattattagtgtaaggttagagattaaaacct

SEQ ID NO: 232 - DNA, 102 bp, synthetic construct
  misc_feature 1..102: note = Epichloe festucae
  misc_feature 51: note = Variation - S is T strain AR37 or C strain RGT18
  source 1..102: mol_type = other DNA
ggagataaagaactatataagaatccctaatattatagaaataacttaccstagagttataagccttataggaactaaaggaataagaactagaaaaagagc

SEQ ID NO: 233 - DNA, 102 bp, synthetic construct
  misc_feature 1..102: note = Epichloe festucae
  misc_feature 51: note = Variation - S is T strain AR37 or C strain RGT18
  source 1..102: mol_type = other DNA
atagctattcctaaataattagcttctattactatagggagatctaggtcstattatactagtactaggtatgtaataaaggtatcttttagcctattaaag

SEQ ID NO: 234 - DNA, 102 bp, synthetic construct
  misc_feature 1..102: note = Epichloe festucae
  misc_feature 51: note = Variation - S is A strain AR37 or G strain RGT18
  source 1..102: mol_type = other DNA
gaatagctttaattattaaagctataattactaaggactataggacttaastaataggtttaagaactataaggcttagatatactagctaaaagactaata

SEQ ID NO: 235 - DNA, 102 bp, synthetic construct
  misc_feature 1..102: note = Epichloe festucae
  misc_feature 51: note = Variation - S is G strain AR37 or A strain RGT18
  source 1..102: mol_type = other DNA
tattaaagtttttttctttcttaaagaagttattattactaaggcctagtstattatttatttatattcctataattctaaagagattcttattatttaagg

SEQ ID NO: 236 - DNA, 102 bp, synthetic construct
  misc_feature 1..102: note = Epichloe festucae
  misc_feature 51: note = Variation - S is T strain AR37 or C strain RGT18
  source 1..102: mol_type = other DNA
gttaatccttatgctatattattacctaaaggtagtgtctctaaatctagsatatattcctagtaacctagttaatccttatgctatattattatagtaata

SEQ ID NO: 237 - DNA, 102 bp, synthetic construct
  misc_feature 1..102: note = Epichloe festucae
  misc_feature 51: note = Variation - S is T strain AR37 or C strain RGT18
  source 1..102: mol_type = other DNA
gctagaaaaccacactaagggcttaacctagaaataaacaaaagggagctsataaagttacttactcttatatttactctaggctattagatttagtttttt

SEQ ID NO: 238 - DNA, 102 bp, synthetic construct
  misc_feature 1..102: note = Epichloe festucae
  misc_feature 51: note = Variation - S is A strain AR37 or G strain RGT18
  source 1..102: mol_type = other DNA
aggaaacctattactagttataaaagcattatactctaatatctaatgtasacctaataggatagaaaactataataatctagtctaactatatctataagg

SEQ ID NO: 239 - DNA, 102 bp, synthetic construct
  misc_feature 1..102: note = Epichloe festucae
  misc_feature 51: note = Variation - S is A strain AR37 or C strain RGT18
  source 1..102: mol_type = other DNA
tatatatatatatataactatcttattaataagagaatattaaaatttaastaataaagaagttcctagtaatatagctattttattagaattataaataat

SEQ ID NO: 240 - DNA, 102 bp, synthetic construct
  misc_feature 1..102: note = Epichloe festucae
  misc_feature 51: note = Variation - S is A strain AR37 or G strain RGT18
  source 1..102: mol_type = other DNA
agtaactttaaagatattagaattagcctataataatagcctaatttaaasgggtttattactttaagtataaagttattaataaaattagttacttagact

SEQ ID NO: 241 - DNA, 102 bp, synthetic construct
  misc_feature 1..102: note = Epichloe festucae
  misc_feature 51: note = Variation - S is T strain AR37 or C strain RGT18
  source 1..102: mol_type = other DNA
atttttagagactatagagccctagaaggtattataatagactaaggtttsatatttactagtggtttctagataactttttgttattttcttgcaataaag

SEQ ID NO: 242 - DNA, 102 bp, synthetic construct
  misc_feature 1..102: note = Epichloe festucae
  misc_feature 51: note = Variation - S is A strain AR37 or G strain RGT18
  source 1..102: mol_type = other DNA
attttataaggaatattaagtcttattatatagtagttaaggctaataggsagttaaaggctattacttataaaaaacgctataaataataaagagttaaac

SEQ ID NO: 243 - DNA, 102 bp, synthetic construct
  misc_feature 1..102: note = Epichloe festucae
  misc_feature 51: note = Variation - S is G strain AR37 or T strain RGT18
  source 1..102: mol_type = other DNA
agatcctcggcgcatctctagagtctagcctttttttttttttttttttgstcttgtctctctgtctttggttctcaaatccttagattctgtcatctcctg

SEQ ID NO: 244 - DNA, 102 bp, synthetic construct
  misc_feature 1..102: note = Epichloe festucae
  misc_feature 51: note = Variation - S is A strain AR37 or G strain RGT18
  source 1..102: mol_type = other DNA
ctagcttccttactaaactattgaataattacacatagaattaattctatstataattcctctaagcattagattatttagtaaatctaatattagttataa

SEQ ID NO: 245 - DNA, 102 bp, synthetic construct
  misc_feature 1..102: note = Epichloe festucae
  misc_feature 51: note = Variation - S is C strain AR37 or T strain RGT18
  source 1..102: mol_type = other DNA
aataaaaaggagggagttcttattttctaagagagttttaggtctttaccscttatataaaataataaatatattaaaggaactattagctagctaggctta

SEQ ID NO: 246 - DNA, 102 bp, synthetic construct
  misc_feature 1..102: note = Epichloe festucae
  misc_feature 51: note = Variation - S is T strain AR37 or C strain RGT18
  source 1..102: mol_type = other DNA
accttttatattatttactaaaacctattagttatatttacttagctaacscttttattttactaggtatttattacctccttaacctccttaactttatat

SEQ ID NO: 247 - DNA, 102 bp, synthetic construct
  misc_feature 1..102: note = Epichloe festucae
  misc_feature 51: note = Variation - S is T strain AR37 or C strain RGT18
  source 1..102: mol_type = other DNA
aagccctatcttctagctttaatttactatatataagacttttatataacstctagttaaagagaaaatcgctattaaagatagctatagggtaacctgctt

SEQ ID NO: 248 - DNA, 102 bp, synthetic construct
  misc_feature 1..102: note = Epichloe festucae
  misc_feature 51: note = Variation - S is T strain AR37 or G strain RGT18
  source 1..102: mol_type = other DNA
aaaaattagttttaattaattatattatagcttatttacttagttataggstttttttattaaaaataagcttaagagataagttctattagttctattagt

SEQ ID NO: 249 - DNA, 102 bp, synthetic construct
  misc_feature 1..102: note = Epichloe festucae
  misc_feature 51: note = Variation - S is T strain AR37 or C strain RGT18
  source 1..102: mol_type = other DNA
ataaagagattaataagctaaaggaataaggaatatagtggtaaataaagsattctatagtataattaaagctattactattaaaataagtgttttcttata

SEQ ID NO: 250 - DNA, 102 bp, synthetic construct
  misc_feature 1..102: note = Epichloe festucae
  misc_feature 51: note = Variation - S is C strain AR37 or T strain RGT18
  source 1..102: mol_type = other DNA
aaaataaagtacttagtaaattagtctataattactagaattatattagtsttttatttacttacttaagtaattactataatattagtaagaatttaaggc

SEQ ID NO: 251 - DNA, 102 bp, synthetic construct
  misc_feature 1..102: note = Epichloe festucae
  misc_feature 51: note = Variation - S is A strain AR37 or G strain RGT18
  source 1..102: mol_type = other DNA
tatatatttattaagatattcttaaagcttataagctccttctagtcctasattatattaactctatatatatttattaagatactattaactaataaaata

SEQ ID NO: 252 - DNA, 102 bp, synthetic construct
  misc_feature 1..102: note = Epichloe festucae
  misc_feature 51: note = Variation - S is C strain AR37 or T strain RGT18
  source 1..102: mol_type = other DNA
accactttaactcctttatagctaagttccttatagatagctttaataatsgcttattattatctaggcacgttaataactagcgctagtccctttatgatt

SEQ ID NO: 253 - DNA, 102 bp, synthetic construct
  misc_feature 1..102: note = Epichloe festucae
  misc_feature 51: note = Variation - S is C strain AR37 or T strain RGT18
  source 1..102: mol_type = other DNA
tttacctaaaagtaagaaattatatttttcttattagtaatactatattasttatatatagtatactaagcttctatttactaacttataactttactatac

SEQ ID NO: 254 - DNA, 102 bp, synthetic construct
  misc_feature 1..102: note = Epichloe festucae
  misc_feature 51: note = Variation - S is C strain AR37 or T strain RGT18
  source 1..102: mol_type = other DNA
agaaaactatataataaggcaaagaagttttacctagagatagaaaactasataataaggcaaagaagttttacctagagaatagttatctttagaaaagac

SEQ ID NO: 255 - DNA, 102 bp, synthetic construct
  misc_feature 1..102: note = Epichloe festucae
  misc_feature 51: note = Variation - S is C strain AR37 or T strain RGT18
  source 1..102: mol_type = other DNA
taatataggtagaactagactattttaattctaggtttgccctagctttasaatataggtataaagtttaatattaggaactctaaacttataattagagtt

SEQ ID NO: 256 - DNA, 102 bp, synthetic construct
  misc_feature 1..102: note = Epichloe festucae
  misc_feature 51: note = Variation - S is C strain AR37 or T strain RGT18
  source 1..102: mol_type = other DNA
ctaggttatatatagcaaactttaatatcctattatattttaaagtattasactttattataatatgtaattctttattatagtaataataataatttaact

SEQ ID NO: 257 - DNA, 102 bp, synthetic construct
  misc_feature 1..102: note = Epichloe festucae
  misc_feature 51: note = Variation - S is G strain AR37 or A strain RGT18
  source 1..102: mol_type = other DNA
gagtaagaatatatctaatatatacttataatatataatatacttaactasaactacccttaggtatagtataactatataagtagctatttattttcttaa

SEQ ID NO: 258 - DNA, 102 bp, synthetic construct
  misc_feature 1..102: note = Epichloe festucae
  misc_feature 51: note = Variation - S is C strain AR37 or T strain RGT18
  source 1..102: mol_type = other DNA
tattttaataagattaccttatagactataggtaaaattatagctaatatstaaggggtaattataagtctaaattaaggggtaattataggtctaatttaa

SEQ ID NO: 259 - DNA, 102 bp, synthetic construct
  misc_feature 1..102: note = Epichloe festucae
  misc_feature 51: note = Variation - S is C strain AR37 or G strain RGT18
  source 1..102: mol_type = other DNA
ttaaaaagggattttattactaaagaaattattaataattataagtaatasctaagtaataaagttaatataaggtaattataatttataagttaatatact

SEQ ID NO: 260 - DNA, 102 bp, synthetic construct
  misc_feature 1..102: note = Epichloe festucae
  misc_feature 51: note = Variation - S is T strain AR37 or C strain RGT18
  source 1..102: mol_type = other DNA
cataaatcccttagtaataagttaggccttgtattttaaaggattattttstttatccttaggccttgtattttaaaggattattttctttatcctttttaa

SEQ ID NO: 261 - DNA, 102 bp, synthetic construct
  misc_feature 1..102: note = Epichloe festucae
  misc_feature 51: note = Variation - S is T strain AR37 or C strain RGT18
  source 1..102: mol_type = other DNA
ggtggccgtcaatggctacgtcgcagctgtcaacagctacgaccgttattsaactgcgttgtggctgcaagcgtagccacaactataacgccactagtaatt

SEQ ID NO: 262 - DNA, 102 bp, synthetic construct
  misc_feature 1..102: note = Epichloe festucae
  misc_feature 51: note = Variation - S is A strain AR37 or G strain RGT18
  source 1..102: mol_type = other DNA
ataaggataataaaggcattactaattatatttctaagggcctaaaggagstatataaattagataaaaaaggtaaaataagatttttcctagggatctaga

SEQ ID NO: 263 - DNA, 102 bp, synthetic construct
  misc_feature 1..102: note = Epichloe festucae
  misc_feature 51: note = Variation - S is C strain AR37 or T strain RGT18
  source 1..102: mol_type = other DNA
agtttatatctttaaaaaggttaagagagattaatttattatagcttatastaaaaggttaagaataaagtaatagctaagactattatagttactactaga

SEQ ID NO: 264 - DNA, 102 bp, synthetic construct
  misc_feature 1..102: note = Epichloe festucae
  misc_feature 51: note = Variation - S is C strain AR37 or T strain RGT18
  source 1..102: mol_type = other DNA
ctataacccttaactaggtttaaggtttattaagatagtaataactttaastaggtaatactaattaaactagggtaggattagttaagctagtaaaactat

SEQ ID NO: 265 - DNA, 102 bp, synthetic construct
  misc_feature 1..102: note = Epichloe festucae
  misc_feature 51: note = Variation - S is C strain AR37 or T strain RGT18
  source 1..102: mol_type = other DNA
cacttttatttatcttactaggtctactatttagttagtagcttatttctstctttactattattcttttatttatttttatagtaattctattctagctat

SEQ ID NO: 266 - DNA, 102 bp, synthetic construct
  misc_feature 1..102: note = Epichloe festucae
  misc_feature 51: note = Variation - S is T strain AR37 or C strain RGT18
  source 1..102: mol_type = other DNA
tatctaactatattataagcttaagtaagtaaataaaagactaatataatsctagtaattatagactaatttactaagtactttattttcttacttataact

SEQ ID NO: 267 - DNA, 102 bp, synthetic construct
  misc_feature 1..102: note = Epichloe festucae
  misc_feature 51: note = Variation - S is G strain AR37 or T strain RGT18
  source 1..102: mol_type = other DNA
ccatctatcttatctcttgaccccgccatcgtcaaggatcgtcaagccccscttgtctccatcagctttctcaaagtgcggctaccttctaccttgatcgtc

SEQ ID NO: 268 - DNA, 102 bp, synthetic construct
  misc_feature 1..102: note = Epichloe festucae
  misc_feature 51: note = Variation - S is T strain AR37 or C strain RGT18
  source 1..102: mol_type = other DNA
gctaagattaatgccttataagcttataatatgtttagatttataatattsaatctagcaaagcatagaggccactggatctttaattcttatatggtctaa

SEQ ID NO: 269 - DNA, 102 bp, synthetic construct
  misc_feature 1..102: note = Epichloe festucae
  misc_feature 51: note = Variation - S is A strain AR37 or G strain RGT18
  source 1..102: mol_type = other DNA
aattataaggctataatagcacttatagtagcttactataagcttataagsgtattaataagggcattaaattacatagctaggctagctagggtattatat

SEQ ID NO: 270 - DNA, 102 bp, synthetic construct
  misc_feature 1..102: note = Epichloe festucae
  misc_feature 51: note = Variation - S is G strain AR37 or A strain RGT18
  source 1..102: mol_type = other DNA
tagctataaggtatattatatttaagctatattttataaagatttatttasggctcttaattatagtatttacctctttacctttaacttctataagtaata

SEQ ID NO: 271 - DNA, 102 bp, synthetic construct
  misc_feature 1..102: note = Epichloe festucae
  misc_feature 51: note = Variation - S is A strain AR37 or G strain RGT18
  source 1..102: mol_type = other DNA
tcttcgggcatctgtgcgaggaaagtttccacatgatccgaattgggagasacacaacttgcaactgccagcaaaatgatggtgcatgtacggagttacttt

SEQ ID NO: 272 - DNA, 102 bp, synthetic construct
  misc_feature 1..102: note = Epichloe festucae
  misc_feature 51: note = Variation - S is A strain AR37 or G strain RGT18
  source 1..102: mol_type = other DNA
aagaggatttagaagcgtttaaaaatagcgaatttttgcattattttacgsaagatatctcttctattaaagagagacaagattataaggaatttaagtcct

SEQ ID NO: 273 - DNA, 102 bp, synthetic construct
  misc_feature 1..102: note = Epichloe festucae
  misc_feature 51: note = Variation - S is C strain AR37 or T strain RGT18
  source 1..102: mol_type = other DNA
ttattagttattagtatttataaggttaaaagaaagccttatataaaagcstttattattacctattttattaaattagttatagaatttataatattatat

SEQ ID NO: 274 - DNA, 102 bp, synthetic construct
  misc_feature 1..102: note = Epichloe festucae
  misc_feature 51: note = Variation - S is C strain AR37 or T strain RGT18
  source 1..102: mol_type = other DNA
tctagctattaagattttattattagatagttatattatctttttagaggsaaataagtaatagttatataagataagttttaggttagatattattaagtc

SEQ ID NO: 275 - DNA, 102 bp, synthetic construct
  misc_feature 1..102: note = Epichloe festucae
  misc_feature 51: note = Variation - S is T strain AR37 or C strain RGT18
  source 1..102: mol_type = other DNA
gaggcctagctatctagctagattaaaaagatcttctttctctcatatacscactaaccatattagtgaatccaggccgctagagaggtcttaagagccact

SEQ ID NO: 276 - DNA, 102 bp, synthetic construct
  misc_feature 1..102: note = Epichloe festucae
  misc_feature 51: note = Variation - S is A strain AR37 or G strain RGT18
  source 1..102: mol_type = other DNA
agttacctagaaagctagtaattaaataaatatagggagatagataataasatcctaatttcttttagtatttcttatataaagaatagggatatataggat

SEQ ID NO: 277 - DNA, 102 bp, synthetic construct
  misc_feature 1..102: note = Epichloe festucae
  misc_feature 51: note = Variation - S is G strain AR37 or A strain RGT18
  source 1..102: mol_type = other DNA
gctaatatctttagattatccctctaatactatccctttaatgccttactsccttctaatctagtggatttattaagaaaacctttagatttagctttataa

SEQ ID NO: 278 - DNA, 102 bp, synthetic construct
  misc_feature 1..102: note = Epichloe festucae
  misc_feature 51: note = Variation - S is A strain AR37 or T strain RGT18
  source 1..102: mol_type = other DNA
ctttaacttagtctatacctaggattattcctttacttatattagtaatasagtagctaacttagtaaacctttataaatcctatactatcttttattttta

SEQ ID NO: 279 - DNA, 102 bp, synthetic construct
  misc_feature 1..102: note = Epichloe festucae
  misc_feature 51: note = Variation - S is C strain AR37 or T strain RGT18
  source 1..102: mol_type = other DNA
ttaagtttaataattacctattacccttatagttccccttaatttctaggstacctcctaatatttaatttaactctagataatcttctatatattagctat

SEQ ID NO: 280 - DNA, 102 bp, synthetic construct
  misc_feature 1..102: note = Epichloe festucae
  misc_feature 51: note = Variation - S is T strain AR37 or A strain RGT18
  source 1..102: mol_type = other DNA
agaaagccactactactgtttttacctagccctttgcttttcttattgctstatattctattagattaatagtaatctaatatgtaggctttcctacctatc

SEQ ID NO: 281 - DNA, 102 bp, synthetic construct
  misc_feature 1..102: note = Epichloe festucae
  misc_feature 51: note = Variation - S is C strain AR37 or T strain RGT18
  source 1..102: mol_type = other DNA
aattactacactataaactacactacactataaactacactaactataagsgaaaaaaaactataatataatataatataaatttttttccttaaactacac

SEQ ID NO: 282 - DNA, 102 bp, synthetic construct
  misc_feature 1..102: note = Epichloe festucae
  misc_feature 51: note = Variation - S is G strain AR37 or A strain RGT18
  source 1..102: mol_type = other DNA
agagattaatatagccttataggaacaaatttaggagagactaggagcttscttagaataggataaaccctagtagaatttaattaatcctatttaaatctt

SEQ ID NO: 283 - DNA, 102 bp, synthetic construct
  misc_feature 1..102: note = Epichloe festucae
  misc_feature 51: note = Variation - S is A strain AR37 or G strain RGT18
  source 1..102: mol_type = other DNA
cgcaggggttctagcaaactccggacaggtcggatctgtacaccttgggastggtggaaatgggaattgggtcatcgaggccttgtcgtaaaaggcactgtc

SEQ ID NO: 284 - DNA, 102 bp, synthetic construct
  misc_feature 1..102: note = Epichloe festucae
  misc_feature 51: note = Variation - S is A strain AR37 or G strain RGT18
  source 1..102: mol_type = other DNA
taccactacatttagcactcctagtatatatgtcacttttaagttaaattstaatagataatttgtaaccttagctaattttagattagccttatctaaatc

SEQ ID NO: 285 - DNA, 102 bp, synthetic construct
  misc_feature 1..102: note = Epichloe festucae
  misc_feature 51: note = Variation - S is A strain AR37 or G strain RGT18
  source 1..102: mol_type = other DNA
ataactaccctacccttacctatttataacttacctagtataagtgtaatstctagtataaatatcttacttatacttacactatcttactttcccctttat

SEQ ID NO: 286 - DNA, 102 bp, synthetic construct
  misc_feature 1..102: note = Epichloe festucae
  misc_feature 51: note = Variation - S is C strain AR37 or A strain RGT18
  source 1..102: mol_type = other DNA
accttagggttagtgcggaaaagtatgcaaaggttagattaaattataatsgggtcacaaactatagtatatatagctacataagtaaactattttaaccct

SEQ ID NO: 287 - DNA, 102 bp, synthetic construct
  misc_feature 1..102: note = Epichloe festucae
  misc_feature 51: note = Variation - S is A strain AR37 or C strain RGT18
  source 1..102: mol_type = other DNA
ttatattaactttattacttagctattacttatagttattaataatttctstagtaataaaatccctttttaatacctaagaattctttaaagtattatagc

SEQ ID NO: 288 - DNA, 102 bp, synthetic construct
  misc_feature 1..102: note = Epichloe festucae
  misc_feature 51: note = Variation - S is A strain AR37 or C strain RGT18
  source 1..102: mol_type = other DNA
tataataaaatattactaaatactataagtattttattattagtgctattstagttttaatttacctaggaaattataaccttagagaggtattactataag

SEQ ID NO: 289 - DNA, 102 bp, synthetic construct
  misc_feature 1..102: note = Epichloe festucae
  misc_feature 51: note = Variation - S is A strain AR37 or G strain RGT18
  source 1..102: mol_type = other DNA
atttaataactttaataactttaataaccttaataaccttaattactattsttactattattactattattactattattactataattactatttactttt

SEQ ID NO: 290 - DNA, 102 bp, synthetic construct
  misc_feature 1..102: note = Epichloe festucae
  misc_feature 51: note = Variation - S is T strain AR37 or C strain RGT18
  source 1..102: mol_type = other DNA
gcctttaaagcatccttatagaagtctaagctatacccttaagctatgccstccccttactcttaatctatctaagttaataagttaataggaagcatgcct

SEQ ID NO: 291 - DNA, 102 bp, synthetic construct
  misc_feature 1..102: note = Epichloe festucae
  misc_feature 51: note = Variation - S is T strain AR37 or A strain RGT18
  source 1..102: mol_type = other DNA
ttttaaagattaaactaaagatatatttagaaaagctactaataagcttasaagagagctataaaactctctataagataataatatttatattagctaagg

SEQ ID NO: 292 - DNA, 102 bp, synthetic construct
  misc_feature 1..102: note = Epichloe festucae
  misc_feature 51: note = Variation - S is C strain AR37 or T strain RGT18
  source 1..102: mol_type = other DNA
gctaaattagctagaagttttagctataaaccttctaaagattaagtaatsttattataaaagtctttatatagcctaaaataaagattaaggtatctaacc

SEQ ID NO: 293 - DNA, 102 bp, synthetic construct
  misc_feature 1..102: note = Epichloe festucae
  misc_feature 51: note = Variation - S is T strain AR37 or A strain RGT18
  source 1..102: mol_type = other DNA
ttagcgctagttattaacatgcctaaataataataagtaattattaaagcsatctataaggaacttagctataaaggagttaaagtggttttttaagtaata

SEQ ID NO: 294 - DNA, 102 bp, synthetic construct
  misc_feature 1..102: note = Epichloe festucae
  misc_feature 51: note = Variation - S is T strain AR37 or A strain RGT18
  source 1..102: mol_type = other DNA
gaatttaacctttaataaattaggtcttttatgattagacctttgacctasccttcgttagctaggtccgtcgttatagattaattaatctaactatctaat

SEQ ID NO: 295 - DNA, 102 bp, synthetic construct
  misc_feature 1..102: note = Epichloe festucae
  misc_feature 51: note = Variation - S is A strain AR37 or G strain RGT18
  source 1..102: mol_type = other DNA
ccatactaggttgctagttatctagtactagataactagttagttgcctasttaggtgaaaaacctactacgatttgtttgttttagctacatacatggttt

SEQ ID NO: 296 - DNA, 102 bp, synthetic construct
  misc_feature 1..102: note = Epichloe festucae
  misc_feature 51: note = Variation - S is A strain AR37 or G strain RGT18
  source 1..102: mol_type = other DNA
attaaggtatatttctataagaattagtattttctaagtatttagcttatsttaatcttaaagaagcttaagtattttataagtataatattaaactaactc

SEQ ID NO: 297 - DNA, 102 bp, synthetic construct
  misc_feature 1..102: note = Epichloe festucae
  misc_feature 51: note = Variation - S is G strain AR37 or T strain RGT18
  source 1..102: mol_type = other DNA
tccctgtgccaggaacgccggtgcctggattgaacttatggcactcgtgasatgcaattcattgtgctaatcgtgaatccttcatagaccacacaatctcca

SEQ ID NO: 298 - DNA, 102 bp, synthetic construct
  misc_feature 1..102: note = Epichloe festucae
  misc_feature 51: note = Variation - S is A strain AR37 or T strain RGT18
  source 1..102: mol_type = other DNA
ctttatccttttataattatattttattataatataaaatatatatccttsaagttaacttctaatctattaaatactattatagtacctttaagggtaaat

SEQ ID NO: 299 - DNA, 102 bp, synthetic construct
  misc_feature 1..102: note = Epichloe festucae
  misc_feature 51: note = Variation - S is T strain AR37 or A strain RGT18
  source 1..102: mol_type = other DNA
taagctaaaagtaaagttttagcactaaaagagaagtatactataattaastagcttttaagtaacttatagacttagtataaaaaatattataactagaag

SEQ ID NO: 300 - DNA, 102 bp, synthetic construct
  misc_feature 1..102: note = Epichloe festucae
  misc_feature 51: note = Variation - S is A strain AR37 or C strain RGT18
  source 1..102: mol_type = other DNA
gaggcattattcctatgcctaaggataagaaaataaggattaatcttgttsataggtagtaatattaaataaggctaattagaccttatagattaggtagct

SEQ ID NO: 301 - DNA, 102 bp, synthetic construct
  misc_feature 1..102: note = Epichloe festucae
  misc_feature 51: note = Variation - S is G strain AR37 or C strain RGT18
  source 1..102: mol_type = other DNA
tactttagaatagtaattataatataaaaacttcataaaaagtgcttttasctagataaaagtaaagatataaaatcttattattacttatatctagtatat

SEQ ID NO: 302 - DNA, 102 bp, synthetic construct
  misc_feature 1..102: note = Epichloe festucae
  misc_feature 51: note = Variation - S is T strain AR37 or A strain RGT18
  source 1..102: mol_type = other DNA
aacactaagaaccctttactaataatatcttataacttaataaacgccttsagtagtaaattaagcattaataatagggattatagtatatccccttaactc

SEQ ID NO: 303 - DNA, 102 bp, synthetic construct
  misc_feature 1..102: note = Epichloe festucae
  misc_feature 51: note = Variation - S is G strain AR37 or A strain RGT18
  source 1..102: mol_type = other DNA
aagaacatagttactagcctattactagttagttacgttaaaatagggatstaaatactatattttgtaaaatagttaataataactaaaatcacgttatag

SEQ ID NO: 304 - DNA, 102 bp, synthetic construct
  misc_feature 1..102: note = Epichloe festucae
  misc_feature 51: note = Variation - S is A strain AR37 or T strain RGT18
  source 1..102: mol_type = other DNA
actagctaagtagtagctctcttactggctagtataacttccctatctagsctattatagctaacttatagctagtttactatatctaagtcttatgcctaa

SEQ ID NO: 305 - DNA, 102 bp, synthetic construct
  misc_feature 1..102: note = Epichloe festucae
  misc_feature 51: note = Variation - S is G strain AR37 or A strain RGT18
  source 1..102: mol_type = other DNA
atctagttctaataataatagatataagattagcctatgttactatagtasataataaaaggtaagatctatataattacttataaagtaaagattagtcta

SEQ ID NO: 306 - DNA, 102 bp, synthetic construct
  misc_feature 1..102: note = Epichloe festucae
  misc_feature 51: note = Variation - S is A strain AR37 or T strain RGT18
  source 1..102: mol_type = other DNA
aagacttctattcttaaggatcttaatatctttctcttactagtattactsataactataaaagcctctttttataataatagtttactatactactagact

SEQ ID NO: 307 - DNA, 102 bp, synthetic construct
  misc_feature 1..102: note = Epichloe festucae
  misc_feature 51: note = Variation - S is C strain AR37 or T strain RGT18
  source 1..102: mol_type = other DNA
gtatttataaatttaaataaaaaggtaagaagttatatagttattactttstctttccttactttacttactaaatctagttttcttaaaagtaagttagta

SEQ ID NO: 308 - DNA, 102 bp, synthetic construct
  misc_feature 1..102: note = Epichloe festucae
  misc_feature 51: note = Variation - S is G strain AR37 or A strain RGT18
  source 1..102: mol_type = other DNA
atcttaatgctattaagatataggttaataaaatccttaatatcccctttsatatcttaatctaattaatttaaagccttaaggcctttcctagataaggca

SEQ ID NO: 309 - DNA, 102 bp, synthetic construct
  misc_feature 1..102: note = Epichloe festucae
  misc_feature 51: note = Variation - S is A strain AR37 or G strain RGT18
  source 1..102: mol_type = other DNA
ttacatatttctttacatatagcgtttaggctactaatactatagtaatasggggtaagtacctagataagggtagtaaactatttatatatttctttacat

SEQ ID NO: 310 - DNA, 102 bp, synthetic construct
  misc_feature 1..102: note = Epichloe festucae
  misc_feature 51: note = Variation - S is T strain AR37 or C strain RGT18
  source 1..102: mol_type = other DNA
atttaacgtatgtaagataaactaatataatactagtcactaaaataatasaattaattaaaagtaattacgggtttaaggctaatttagctattattaaac

SEQ ID NO: 311 - DNA, 102 bp, synthetic construct
  misc_feature 1..102: note = Epichloe festucae
  misc_feature 51: note = Variation - S is A strain AR37 or G strain RGT18
  source 1..102: mol_type = other DNA
ccttaattaattattatagattatagtttagattagttaggaaaattttasataatattatactctttagttaggattaattagttactttttatattatat

SEQ ID NO: 312 - DNA, 102 bp, synthetic construct
  misc_feature 1..102: note = Epichloe festucae
  misc_feature 51: note = Variation - S is G strain AR37 or T strain RGT18
  source 1..102: mol_type = other DNA
gactagattaaagaatatttacctataattatatattaggagtataaatastagagatatatagtaataataaaatatctctcctttacttataataagtag

SEQ ID NO: 313 - DNA, 102 bp, synthetic construct
  misc_feature 1..102: note = Epichloe festucae
  misc_feature 51: note = Variation - S is C strain AR37 or G strain RGT18
  source 1..102: mol_type = other DNA
aagaagaagaagaagaagaagaagaagaagaagaacaacaacaacaacaasaacaacaacaacaacgagacggactgacaacgggcaaccgagccagggggg

SEQ ID NO: 314 - DNA, 102 bp, synthetic construct
  misc_feature 1..102: note = Epichloe festucae
  misc_feature 51: note = Variation - S is A strain AR37 or G strain RGT18
  source 1..102: mol_type = other DNA
ttacttaattttatcacagatatactagaagtattagctataaatataatstggtaaatagaaggatacataacatataatttattatgcctagtaaattac

SEQ ID NO: 315 - DNA, 102 bp, synthetic construct
  misc_feature 1..102: note = Epichloe festucae
  misc_feature 51: note = Variation - S is A strain AR37 or T strain RGT18
  source 1..102: mol_type = other DNA
gcgccacttttgtatgccaatcccaaaggtctgcccgtcaaagcggcgacsgcttcttcggatttgccagggcgactgcacttcgataaaaaccggaattac

SEQ ID NO: 316 - DNA, 102 bp, synthetic construct
  misc_feature 1..102: note = Epichloe festucae
  misc_feature 51: note = Variation - S is A strain AR37 or G strain RGT18
  source 1..102: mol_type = other DNA
acaggtcgcgcgagcgcgggatacacattgccgcgggataccttgtcggcscggccgggctgttgtggctcgccctcgcgcccagcggcgtgggcaaatgga

SEQ ID NO: 317 - DNA, 102 bp, synthetic construct
  misc_feature 1..102: note = Epichloe festucae
  misc_feature 51: note = Variation - S is C strain AR37 or T strain RGT18
  source 1..102: mol_type = other DNA
tatttatatatttattactactagattctttaattagcctttaccttttcstttttaatttttattttctagaatacttagcttaatctttattacttttaa

SEQ ID NO: 318 - DNA, 102 bp, synthetic construct
  misc_feature 1..102: note = Epichloe festucae
  misc_feature 51: note = Variation - S is C strain AR37 or T strain RGT18
  source 1..102: mol_type = other DNA
ttaactagtaaatattaagataaataaaagataccttttaataagtacctstcctttattattataacctaagttagctagtatatattaagataaatactt

SEQ ID NO: 319 - DNA, 102 bp, synthetic construct
  misc_feature 1..102: note = Epichloe festucae
  misc_feature 51: note = Variation - S is A strain AR37 or G strain RGT18
  source 1..102: mol_type = other DNA
tatactaggaaattataacctttctaatggagcccttaatctatataagasacctagctctcataggactagttataagagctctagcaatagtaagtttaa

SEQ ID NO: 320 - DNA, 102 bp, synthetic construct
  misc_feature 1..102: note = Epichloe festucae
  misc_feature 51: note = Variation - S is T strain AR37 or A strain RGT18
  source 1..102: mol_type = other DNA
atagtattactaagtaatactataaatctaaagatatagattaatattttsaactatctttactttatagcttaaaatatcctaatagtaagctttcttaat

SEQ ID NO: 321 - DNA, 102 bp, synthetic construct
  misc_feature 1..102: note = Epichloe festucae
  misc_feature 51: note = Variation - S is T strain AR37 or A strain RGT18
  source 1..102: mol_type = other DNA
aaaaggaaagaaaaagataaataagctagtatttactaaaggactagctasgagaattattaaattaaaaactagacttaagaatatattaagtaaactatt

SEQ ID NO: 322 - DNA, 102 bp, synthetic construct
  misc_feature 1..102: note = Epichloe festucae
  misc_feature 51: note = Variation - S is T strain AR37 or A strain RGT18
  source 1..102: mol_type = other DNA
atataaacttagcttaattactactaaaatctataaaattaaattaataasatctaggaaatcctagatattatataagtattataaataattaaggtaata

SEQ ID NO: 323 - DNA, 102 bp, synthetic construct
  misc_feature 1..102: note = Epichloe festucae
  misc_feature 51: note = Variation - S is A strain AR37 or C strain RGT18
  source 1..102: mol_type = other DNA
cttctaacctttaggggccttttccttgtctttagcacccttttctaggtsttaagccctataattcagggctttagatactatagataacttatccctctg

SEQ ID NO: 324 - DNA, 102 bp, synthetic construct
  misc_feature 1..102: note = Epichloe festucae
  misc_feature 51: note = Variation - S is C strain AR37 or T strain RGT18
  source 1..102: mol_type = other DNA
ttaggttatagctatatagtaacttatttagggtagtaactaaactagctstaggttatagctatatagtagcttatttagggtaactcctattataaaaaa

SEQ ID NO: 325 - DNA, 102 bp, synthetic construct
  misc_feature 1..102: note = Epichloe festucae
  misc_feature 51: note = Variation - S is G strain AR37 or A strain RGT18
  source 1..102: mol_type = other DNA
taagggtatatataatataagtattatatatattactaggggatattatasagaggagtttattagtaataagtaagtaagggtatatataagggcttaggc

SEQ ID NO: 326 - DNA, 102 bp, synthetic construct
  misc_feature 1..102: note = Epichloe festucae
  misc_feature 51: note = Variation - S is T strain AR37 or C strain RGT18
  source 1..102: mol_type = other DNA
tcttaggctttaataactatattactagctttatagtctcctaagaagacstttacttacttctctcttataatagatttatttataataagagttaataaa

SEQ ID NO: 327 - DNA, 102 bp, synthetic construct
  misc_feature 1..102: note = Epichloe festucae
  misc_feature 51: note = Variation - S is T strain AR37 or C strain RGT18
  source 1..102: mol_type = other DNA
tacttagtaactaataaggttaagccttttttatagtatatttatatttcsttattagtactttaatctaatattactacctttcttactagacttacttta

SEQ ID NO: 328 - DNA, 102 bp, synthetic construct
  misc_feature 1..102: note = Epichloe festucae
  misc_feature 51: note = Variation - S is G strain AR37 or A strain RGT18
  source 1..102: mol_type = other DNA
ttattagctagaaatcaaagaaagctagtataatagctctattaatattasaagctaaagctaacgctatttacaagaccttctaggagctatagtggcttt

SEQ ID NO: 329 - DNA, 102 bp, synthetic construct
  misc_feature 1..102: note = Epichloe festucae
  misc_feature 51: note = Variation - S is A strain AR37 or G strain RGT18
  source 1..102: mol_type = other DNA
cttgtcatgaagcaaatgtctaaatgtttgaaccattcgatctcggtcagsgtatatatcttttgaatgtcaagtgttgatggtcgtagtcggaatagaatg

SEQ ID NO: 330 - DNA, 102 bp, synthetic construct
  misc_feature 1..102: note = Epichloe festucae
  misc_feature 51: note = Variation - S is G strain AR37 or A strain RGT18
  source 1..102: mol_type = other DNA
taaacttagtttaataactatttaggtaaagaccctaataataaaggcaasatacctagatctcttagagagcttaatataaaaacctttataaagcttctt

SEQ ID NO: 331 - DNA, 102 bp, synthetic construct
  misc_feature 1..102: note = Epichloe festucae
  misc_feature 51: note = Variation - S is G strain AR37 or A strain RGT18
  source 1..102: mol_type = other DNA
atataagaattcccttacttttacctaataatttatagataaattattctsaaaatacaaacattttatataagtatatattaataatattattgtattttt

SEQ ID NO: 332 - DNA, 102 bp, synthetic construct
  misc_feature 1..102: note = Epichloe festucae
  misc_feature 51: note = Variation - S is C strain AR37 or T strain RGT18
  source 1..102: mol_type = other DNA
aaataataggctaataactaggataaccttaaggataactagaataaattstaaacttaaatacttatattacttaaggactttataaactataatacttaa

SEQ ID NO: 333 - DNA, 102 bp, synthetic construct
  misc_feature 1..102: note = Epichloe festucae
  misc_feature 51: note = Variation - S is C strain AR37 or T strain RGT18
  source 1..102: mol_type = other DNA
gggatgcctagtggtctctcttaactagtagctagtgaaaaaatcctattstattaaataaagaataaacctccttactataggtgttatttataatgttac

SEQ ID NO: 334 - DNA, 102 bp, synthetic construct
  misc_feature 1..102: note = Epichloe festucae
  misc_feature 51: note = Variation - S is T strain AR37 or A strain RGT18
  source 1..102: mol_type = other DNA
atagattttattatagaattacctattacctaagtaagtaaataagagacsaatataatcctagtaattataaactaatttactaagtactttatattctta

SEQ ID NO: 335 - DNA, 102 bp, synthetic construct
  misc_feature 1..102: note = Epichloe festucae
  misc_feature 51: note = Variation - S is G strain AR37 or A strain RGT18
  source 1..102: mol_type = other DNA
aactatattagtgaatctagactactagagaggtcttaagagccacttttsattttccgtaaaatttatttatatgtaaaatccaaaaaattaacttaccac

SEQ ID NO: 336 - DNA, 102 bp, synthetic construct
  misc_feature 1..102: note = Epichloe festucae
  misc_feature 51: note = Variation - S is T strain AR37 or C strain RGT18
  source 1..102: mol_type = other DNA
agattaataattccctagtaagaggcaagggaaaagctagtctatagttasatagtataagaggcctcctaatatactaagactaggtagttattctagtta

SEQ ID NO: 337 - DNA, 102 bp, synthetic construct
  misc_feature 1..102: note = Epichloe festucae
  misc_feature 51: note = Variation - S is T strain AR37 or A strain RGT18
  source 1..102: mol_type = other DNA
taagatataaaggaatatataatttatatagtaagagttagagatttaatsaaaaaaaaagggggagagagagaaaaaaggaataaaaggaaagagagagaa

SEQ ID NO: 338 - DNA, 102 bp, synthetic construct
  misc_feature 1..102: note = Epichloe festucae
  misc_feature 51: note = Variation - S is A strain AR37 or G strain RGT18
  source 1..102: mol_type = other DNA
ttattaagatagtaataactttaactaagtaatactaattagactaaggtsagattagttaagctagcgaaattatttaatagatatctataaattcctaag

SEQ ID NO: 339 - DNA, 102 bp, synthetic construct
  misc_feature 1..102: note = Epichloe festucae
  misc_feature 51: note = Variation - S is G strain AR37 or C strain RGT18
  source 1..102: mol_type = other DNA
aaattataatacctaggataaagctaactatttctaacatattaatattastaaaggagttagtaaactttatagacctctttaataaggctaaagctaata

SEQ ID NO: 340 - DNA, 102 bp, synthetic construct
  misc_feature 1..102: note = Epichloe festucae
  misc_feature 51: note = Variation - S is G strain AR37 or C strain RGT18
  source 1..102: mol_type = other DNA
ttaaggatataaaataaaagctaatctctagatttattaaactattttaascacttaatactataaggaaataagtatattaacttatattacttaaaaagt

SEQ ID NO: 341 - DNA, 102 bp, synthetic construct
  misc_feature 1..102: note = Epichloe festucae
  misc_feature 51: note = Variation - S is C strain AR37 or T strain RGT18
  source 1..102: mol_type = other DNA
tcttagtttatatatagttattatatttatttaatatcttaatttactaastactttttatagctttaataaagaaaaaatcctttaattttagtataaagt

SEQ ID NO: 342 - DNA, 102 bp, synthetic construct
  misc_feature 1..102: note = Epichloe festucae
  misc_feature 51: note = Variation - S is A strain AR37 or G strain RGT18
  source 1..102: mol_type = other DNA
ctcgctccgattcgtatgggtgaccgagttccccatgttcaagcccgttgsagaaggcgagcctggccaaggcggcgcagctggcatctcagcagcacacca

SEQ ID NO: 343 - DNA, 102 bp, synthetic construct
  misc_feature 1..102: note = Epichloe festucae
  misc_feature 51: note = Variation - S is A strain AR37 or T strain RGT18
  source 1..102: mol_type = other DNA
attaatcttagcaaggctttagcttatactagactagtagttaattagccsaaggctcctatatctagtataattcctctaaagatctctttagaatagcat

SEQ ID NO: 344 - DNA, 102 bp, synthetic construct
  misc_feature 1..102: note = Epichloe festucae
  misc_feature 51: note = Variation - S is T strain AR37 or C strain RGT18
  source 1..102: mol_type = other DNA
tattacctaggacttaattataaaatatatttaatattactagtcttaaascttttaaaggggatctaataaatatagaaaatatatccttactataagata

SEQ ID NO: 345 - DNA, 102 bp, synthetic construct
  misc_feature 1..102: note = Epichloe festucae
  misc_feature 51: note = Variation - S is A strain AR37 or G strain RGT18
  source 1..102: mol_type = other DNA
ccccccctccttcttaattactctttattattataaaaacttattactaasgtgtgtatatactagatagaacctaggcatattaattttttatagctaaat

SEQ ID NO: 346 - DNA, 102 bp, synthetic construct
  misc_feature 1..102: note = Epichloe festucae
  misc_feature 51: note = Variation - S is T strain AR37 or C strain RGT18
  source 1..102: mol_type = other DNA
tactactaacagagcggggtagcttgcgatgcatctaatcgcatcgcgtgsatccctttggtggctccactctttggccacggtcggactatctattgtccg

SEQ ID NO: 347 - DNA, 102 bp, synthetic construct
  misc_feature 1..102: note = Epichloe festucae
  misc_feature 51: note = Variation - S is A strain AR37 or G strain RGT18
  source 1..102: mol_type = other DNA
cctccgtttagagttagtgctttactaatatagctatagcacgttcgctasgcaatagtcatagcacaaagagttatctgcctaggacgtaacctaggttct

SEQ ID NO: 348 - DNA, 102 bp, synthetic construct
  misc_feature 1..102: note = Epichloe festucae
  misc_feature 51: note = Variation - S is T strain AR37 or C strain RGT18
  source 1..102: mol_type = other DNA
ctagcataggctatgtaaataataaagaggctagctagctataagatagcsatatgcttatagagcaaggtatttattaaagactatgcatattattagtgc

SEQ ID NO: 349 - DNA, 102 bp, synthetic construct
  misc_feature 1..102: note = Epichloe festucae
  misc_feature 51: note = Variation - S is G strain AR37 or A strain RGT18
  source 1..102: mol_type = other DNA
gtggaccttttctccttctatatttacatgcgagatcagcaaagatcggtsgattatctggacttttggtaagcaggatgatttgaaggtctttattttgac

SEQ ID NO: 350 - DNA, 102 bp, synthetic construct
  misc_feature 1..102: note = Epichloe festucae
  misc_feature 51: note = Variation - S is C strain AR37 or A strain RGT18
  source 1..102: mol_type = other DNA
tcaccgtcacatgtttcgttgaacatgtagacgtagcatgttgcagggggsatggcgggaagcttgtcagagtgtgaggcggcagacgagcctgtcgtgttg

SEQ ID NO: 351 - DNA, 102 bp, synthetic construct
  misc_feature 1..102: note = Epichloe festucae
  misc_feature 51: note = Variation - S is G strain AR37 or T strain RGT18
  source 1..102: mol_type = other DNA
ataataaatcctaatctctaggaagacctttagggaataatattagtatasacccttaagataaactataaagagacttagactttttctagtatttcttat

SEQ ID NO: 352 - DNA, 102 bp, synthetic construct
  misc_feature 1..102: note = Epichloe festucae
  misc_feature 51: note = Variation - S is G strain AR37 or T strain RGT18
  source 1..102: mol_type = other DNA
cgtgggtatcgcctgatgaacaactttcttcactttttctttttttttttsgggttcttgtcatgacataaccatttgaagtttaccagcttgttgtggtgg

SEQ ID NO: 353 - DNA, 102 bp, synthetic construct
  misc_feature 1..102: note = Epichloe festucae
  misc_feature 51: note = Variation - S is A strain AR37 or G strain RGT18
  source 1..102: mol_type = other DNA
atagggctctagccgtatttatcttatcttgccttatagttagtgtgtatstagttaagtgtaaagagaatcttttagtaattatattagtattttttcttt

SEQ ID NO: 354 - DNA, 102 bp, synthetic construct
  misc_feature 1..102: note = Epichloe festucae
  misc_feature 51: note = Variation - S is A strain AR37 or G strain RGT18
  source 1..102: mol_type = other DNA
ctcctaatatataattataggtaaatattctttaatttagtctatacctasaattatccctttacttatattagtaataaagtaactaacttagtaaacctt

SEQ ID NO: 355 - DNA, 102 bp, synthetic construct
  misc_feature 1..102: note = Epichloe festucae
  misc_feature 51: note = Variation - S is C strain AR37 or T strain RGT18
  source 1..102: mol_type = other DNA
ttattatctcttcctttaggtgctttaaagttataaggtattatagttttstataatataattagtatatactatatattataaaaaagctagatattactt

SEQ ID NO: 356 - DNA, 102 bp, synthetic construct
  misc_feature 1..102: note = Epichloe festucae
  misc_feature 51: note = Variation - S is A strain AR37 or C strain RGT18
  source 1..102: mol_type = other DNA
atagctatattttaattcctagggttagtaaaggtacttatagtaattacstttagaataggtcttatatagtaagctataagtagggttttacttctaggt

SEQ ID NO: 357 - DNA, 102 bp, synthetic construct
  misc_feature 1..102: note = Epichloe festucae
  misc_feature 51: note = Variation - S is A strain AR37 or G strain RGT18
  source 1..102: mol_type = other DNA
tataagggcttaggctttacctaagcatattatagatagaaggaagggtasgagtaagtaagaataggtaaggaggagcttatataagaagctaagggggta

SEQ ID NO: 358 - DNA, 102 bp, synthetic construct
  misc_feature 1..102: note = Epichloe festucae
  misc_feature 51: note = Variation - S is T strain AR37 or C strain RGT18
  source 1..102: mol_type = other DNA
ttacgcactaagattaggggctagctacctctaaccttattaattagtatstatcttcctttttataaaagggaagccttttatttatactaatttcctttt

SEQ ID NO: 359 - DNA, 102 bp, synthetic construct
  misc_feature 1..102: note = Epichloe festucae
  misc_feature 51: note = Variation - S is T strain AR37 or C strain RGT18
  source 1..102: mol_type = other DNA
actattataaagactaaagtatttatcgttaaatactagctattccctttscttaaatataaacttcctagtctaaatactattttaactaccttttattag

SEQ ID NO: 360 - DNA, 102 bp, synthetic construct
  misc_feature 1..102: note = Epichloe festucae
  misc_feature 51: note = Variation - S is A strain AR37 or G strain RGT18
  source 1..102: mol_type = other DNA
tagccttatatatattaagtatattaatattacttacgcttaggacttatstctattagtattagattaggtccttagaattatattagtaatatatattag

SEQ ID NO: 361 - DNA, 102 bp, synthetic construct
  misc_feature 1..102: note = Epichloe festucae
  misc_feature 51: note = Variation - S is A strain AR37 or T strain RGT18
  source 1..102: mol_type = other DNA
aaataaactattagtataattactatagaaagtataggattaagatctagstttataagtaagattaataattccctagtaagagataagggaaaagctagt

SEQ ID NO: 362 - DNA, 102 bp, synthetic construct
  misc_feature 1..102: note = Epichloe festucae
  misc_feature 51: note = Variation - S is A strain AR37 or T strain RGT18
  source 1..102: mol_type = other DNA
aaagttagtatagcctagtataaaaaagtcagtaatttatagctataagasaataaaatacttagtaactcactatcttatatatattgctatatttattat

SEQ ID NO: 363 - DNA, 102 bp, synthetic construct
  misc_feature 1..102: note = Epichloe festucae
  misc_feature 51: note = Variation - S is A strain AR37 or G strain RGT18
  source 1..102: mol_type = other DNA
aaaaaaatagataacctatattaatttttataattagtttaaataaataasgtacttaatactatagttctaaatagtataactaaagggcttatattatag

SEQ ID NO: 364 - DNA, 102 bp, synthetic construct
  misc_feature 1..102: note = Epichloe festucae
  misc_feature 51: note = Variation - S is G strain AR37 or T strain RGT18
  source 1..102: mol_type = other DNA
tccaatgcagtcattcaatcgacgtcaccagcagcaaattgctgggcaggsgggaaagaatgacgatgatgatttccttgtcgcataatccgttcactaaaa

SEQ ID NO: 365 - DNA, 102 bp, synthetic construct
  misc_feature 1..102: note = Epichloe festucae
  misc_feature 51: note = Variation - S is T strain AR37 or C strain RGT18
  source 1..102: mol_type = other DNA
taaagttatatatatatatctaagctattttaagtatagtaactataggasttactaataatataaatatagtaatatttaaaaagaatatagcctagactt

SEQ ID NO: 366 - DNA, 102 bp, synthetic construct
  misc_feature 1..102: note = Epichloe festucae
  misc_feature 51: note = Variation - S is A strain AR37 or G strain RGT18
  source 1..102: mol_type = other DNA
tcttttttttttttttttgctggacttgcgacaggtcatgcggtagcatgsgacggtctggggagtcgcaagtcgtggtggttcaaaactaaaaactcattc

SEQ ID NO: 367 - DNA, 102 bp, synthetic construct
  misc_feature 1..102: note = Epichloe festucae
  misc_feature 51: note = Variation - S is T strain AR37 or A strain RGT18
  source 1..102: mol_type = other DNA
acagtgatggagatgttaagaaagatataggattaggcagtaactattaasaagctaatagaggagtaaaaaagacgtaaagaacatgctaggaaggtaaga

SEQ ID NO: 368 - DNA, 102 bp, synthetic construct
  misc_feature 1..102: note = Epichloe festucae
  misc_feature 51: note = Variation - S is A strain AR37 or G strain RGT18
  source 1..102: mol_type = other DNA
atagatttaacccttatctattaagtctataatctagtgcctaacctctasaagctagtcccttagtatattatatagtagtatattatatagtaatcccta

SEQ ID NO: 369 - DNA, 102 bp, synthetic construct
  misc_feature 1..102: note = Epichloe festucae
  misc_feature 51: note = Variation - S is C strain AR37 or T strain RGT18
  source 1..102: mol_type = other DNA
tgcactattaggacgcgaatccattgaacaacctctttttttttttttttstttttttttttttccccttgctcgcaggttcccttgcagggtgtcactggc

SEQ ID NO: 370 - DNA, 102 bp, synthetic construct
  misc_feature 1..102: note = Epichloe festucae
  misc_feature 51: note = Variation - S is G strain AR37 or T strain RGT18
  source 1..102: mol_type = other DNA
ttcgagaacgggcacttctgcgatggcccgatgggtaactcgtatacaaastagcgagcgtggtccccaacgtgggatccccccttcgtcgccaggacgtgc

SEQ ID NO: 371 - DNA, 102 bp, synthetic construct
  misc_feature 1..102: note = Epichloe festucae
  misc_feature 51: note = Variation - S is T strain AR37 or C strain RGT18
  source 1..102: mol_type = other DNA
aagggaatagctagcgtttaactagctaaagaataccttttaataagtacsttttctttattattataacctaagttagctagtgtgtattaagataaatac

SEQ ID NO: 372 - DNA, 102 bp, synthetic construct
  misc_feature 1..102: note = Epichloe festucae
  misc_feature 51: note = Variation - S is G strain AR37 or A strain RGT18
  source 1..102: mol_type = other DNA
taaataagtaggtatagttttccatgcctaattttactaaagtttataggstataacctaattcttataatacttcaaaggcattttatttagtaaataaac

SEQ ID NO: 373 - DNA, 102 bp, synthetic construct
  misc_feature 1..102: note = Epichloe festucae
  misc_feature 51: note = Variation - S is G strain AR37 or A strain RGT18
  source 1..102: mol_type = other DNA
aatataatcttactatagaataccttataaataatagaataagaatatagstatctctataataagataactagtagttagctatataagcgctatttaata

SEQ ID NO: 374 - DNA, 102 bp, synthetic construct
  misc_feature 1..102: note = Epichloe festucae
  misc_feature 51: note = Variation - S is C strain AR37 or T strain RGT18
  source 1..102: mol_type = other DNA
cctcaaggcgtcgaattggatccagcctgtggttcatgtcccgcggtagtsgagaatcgagaagccatggcgcaagccaagtctgccgcaaagtccccgttc

SEQ ID NO: 375 - DNA, 102 bp, synthetic construct
  misc_feature 1..102: note = Epichloe festucae
  misc_feature 51: note = Variation - S is C strain AR37 or T strain RGT18
  source 1..102: mol_type = other DNA
accggcacaatgacgtggttccagaaacaatttactctgcccgccaagtcscgcggctcctacctcatcactgatcagatcgttggggctcttcctgagatt

SEQ ID NO: 376 - DNA, 102 bp, synthetic construct
  misc_feature 1..102: note = Epichloe festucae
  misc_feature 51: note = Variation - S is G strain AR37 or A strain RGT18
  source 1..102: mol_type = other DNA
ggagttatattataatagtttattaactagaagtattctataaccttttasttactatataatactaagaaccctttactaataatatcttataacttaata

SEQ ID NO: 377 - DNA, 102 bp, synthetic construct
  misc_feature 1..102: note = Epichloe festucae
  misc_feature 51: note = Variation - S is A strain AR37 or G strain RGT18
  source 1..102: mol_type = other DNA
aataatagttaatttatatagagattttagaattataaggggtagcccttsatttcctgttttcctatataaattagctctttagcttgtctctctatatct

SEQ ID NO: 378 - DNA, 102 bp, synthetic construct
  misc_feature 1..102: note = Epichloe festucae
  misc_feature 51: note = Variation - S is G strain AR37 or A strain RGT18
  source 1..102: mol_type = other DNA
cttagtaagaggtatatagttttatataagaactaggtaaaacactaaatscttatatctaataagctaagtatttagcttctaagataaaatctaatatat

SEQ ID NO: 379 - DNA, 102 bp, synthetic construct
  misc_feature 1..102: note = Epichloe festucae
  misc_feature 51: note = Variation - S is A strain AR37 or G strain RGT18
  source 1..102: mol_type = other DNA
aacctttagtaaagttaataaatctctccttctaataggtaaaaagcagtsgtttctcttacctctagaagctactaagggtagccctatttacgtaccact

SEQ ID NO: 380 - DNA, 102 bp, synthetic construct
  misc_feature 1..102: note = Epichloe festucae
  misc_feature 51: note = Variation - S is A strain AR37 or T strain RGT18
  source 1..102: mol_type = other DNA
atcttgtgtcgctggttggggagattggcaatgccaatcggcgaggcactstccgcagctggggccatcttggacaaaagggatttgtgagttggaaaggtg

SEQ ID NO: 381 - DNA, 102 bp, synthetic construct
  misc_feature 1..102: note = Epichloe festucae
  misc_feature 51: note = Variation - S is T strain AR37 or C strain RGT18
  source 1..102: mol_type = other DNA
gtttcttaaaatactattaagaaagtaaaagaaaactatacttacctagcsttccttatttcctttctttaatatttcctagtaataatattatttagatta

SEQ ID NO: 382 - DNA, 102 bp, synthetic construct
  misc_feature 1..102: note = Epichloe festucae
  misc_feature 51: note = Variation - S is T strain AR37 or C strain RGT18
  source 1..102: mol_type = other DNA
atagtatactttttctcttacttataagctttaataatctctagctatatsttataggaaactaagctaggtagtattactaaagtatatataaataatatt

SEQ ID NO: 383 - DNA, 102 bp, synthetic construct
  misc_feature 1..102: note = Epichloe festucae
  misc_feature 51: note = Variation - S is G strain AR37 or A strain RGT18
  source 1..102: mol_type = other DNA
agcactctctatatcttttactagaacctattagttatatttacttagctsacccttttattttactaggtatttattactttcttagttttttctatagtc

SEQ ID NO: 384 - DNA, 102 bp, synthetic construct
  misc_feature 1..102: note = Epichloe festucae
  misc_feature 51: note = Variation - S is C strain AR37 or G strain RGT18
  source 1..102: mol_type = other DNA
actatatctaggatatagctatattactacttttaagtaactttaattaasctatagtaaagttattaccttactatactttatataataagacttaaatta

SEQ ID NO: 385 - DNA, 102 bp, synthetic construct
  misc_feature 1..102: note = Epichloe festucae
  misc_feature 51: note = Variation - S is C strain AR37 or T strain RGT18
  source 1..102: mol_type = other DNA
ataatagcattttagagtctttattttattaatcctatttaccttagtagsgctttacttactaaggagggggcctttatgtatttctagggtaattaattt

SEQ ID NO: 386 - DNA, 102 bp, synthetic construct
  misc_feature 1..102: note = Epichloe festucae
  misc_feature 51: note = Variation - S is C strain AR37 or T strain RGT18
  source 1..102: mol_type = other DNA
tttacccctagataaatagctagataaaacgtttaaactaggtcttaaaasattatttaagggcttttacttatactaaataaactaattaggtaatttaag

SEQ ID NO: 387 - DNA, 102 bp, synthetic construct
  misc_feature 1..102: note = Epichloe festucae
  misc_feature 51: note = Variation - S is A strain AR37 or G strain RGT18
  source 1..102: mol_type = other DNA
gagaaactgagctagccttcgagctagttgttggctttaagctggttgctsgcttcgagctagttgctagcttcgagctagttgctagctttgaactggtcg

SEQ ID NO: 388 - DNA, 102 bp, synthetic construct
  misc_feature 1..102: note = Epichloe festucae
  misc_feature 51: note = Variation - S is C strain AR37 or T strain RGT18
  source 1..102: mol_type = other DNA
acactacacgttttagtgcaatactctagttatatataatattatactttsttaataatactatttaacttaatactttatttccctaatataacttaaaga

SEQ ID NO: 389 - DNA, 102 bp, synthetic construct
  misc_feature 1..102: note = Epichloe festucae
  misc_feature 51: note = Variation - S is C strain AR37 or T strain RGT18
  source 1..102: mol_type = other DNA
ttttattataatttagttatttagttataaatttataaagttttaccttasttagaaaattagctataagtaaaggtatagggtatatataaaagatatttt

SEQ ID NO: 390 - DNA, 102 bp, synthetic construct
  misc_feature 1..102: note = Epichloe festucae
  misc_feature 51: note = Variation - S is G strain AR37 or A strain RGT18
  source 1..102: mol_type = other DNA
ttattacacattacattacattacattcattacaaatgtaatatcaggggsaaaaaaagtggggtatattaaggtcttataatattgtatagaattttctct

SEQ ID NO: 391 - DNA, 102 bp, synthetic construct
  misc_feature 1..102: note = Epichloe festucae
  misc_feature 51: note = Variation - S is A strain AR37 or G strain RGT18
  source 1..102: mol_type = other DNA
agtaagctttagacctttctttttcttagctagcttattttatttccttasttaagtcctagctatatattactacatataccctagttattagtatattac

SEQ ID NO: 392 - DNA, 102 bp, synthetic construct
  misc_feature 1..102: note = Epichloe festucae
  misc_feature 51: note = Variation - S is A strain AR37 or G strain RGT18
  source 1..102: mol_type = other DNA
gataggcctaatagaatactaaaaaattattaatcttagtatatcttagasgctttaaaataatttaatatactagatagtaagtatatcttagaggcttta

SEQ ID NO: 393 - DNA, 102 bp, synthetic construct
  misc_feature 1..102: note = Epichloe festucae
  misc_feature 51: note = Variation - S is T strain AR37 or A strain RGT18
  source 1..102: mol_type = other DNA
gttttaagttatattagtaaaataaagtattaagttaaatagtattattasaaaggtataatcttatatataaccttacttagttatagtaaaattattaaa

SEQ ID NO: 394 - DNA, 102 bp, synthetic construct
  misc_feature 1..102: note = Epichloe festucae
  misc_feature 51: note = Variation - S is C strain AR37 or G strain RGT18
  source 1..102: mol_type = other DNA
tttaacggtcagaggccttgtcagacagtcggattaattagtctaacgacsgaagcttttgttagcggttagagacctcgttagaagaccttctattagtca

SEQ ID NO: 395 - DNA, 102 bp, synthetic construct
  misc_feature 1..102: note = Epichloe festucae
  misc_feature 51: note = Variation - S is A strain AR37 or G strain RGT18
  source 1..102: mol_type = other DNA
tataatagaatttaagaaatttgctaaaagctagataaattcgctagtttsctagactaagagaatgaatttagactaaattaaaacggaaatagttagtat

SEQ ID NO: 396 - DNA, 102 bp, synthetic construct
  misc_feature 1..102: note = Epichloe festucae
  misc_feature 51: note = Variation - S is C strain AR37 or T strain RGT18
  source 1..102: mol_type = other DNA
aggcatttgattcagccagcattgacgacacacatcacatgcttgctttgsacatgtgaacaacaggaacagaaaaggacttcgacagtggcgaccgagtgt

SEQ ID NO: 397 - DNA, 102 bp, synthetic construct
  misc_feature 1..102: note = Epichloe festucae
  misc_feature 51: note = Variation - S is A strain AR37 or G strain RGT18
  source 1..102: mol_type = other DNA
agggagcgttagtttagacctatcctaattcttatataagcgtatgtagtsattaagggacccctaataagggggaaggctattagctttagccttattaaa

SEQ ID NO: 398 - DNA, 102 bp, synthetic construct
  misc_feature 1..102: note = Epichloe festucae
  misc_feature 51: note = Variation - S is A strain AR37 or T strain RGT18
  source 1..102: mol_type = other DNA
aatttataatatttacctttttttaaggattttactataactagggttatstataatattatacctttttaataatactattatacttattactttatttta

SEQ ID NO: 399 - DNA, 102 bp, synthetic construct
  misc_feature 1..102: note = Epichloe festucae
  misc_feature 51: note = Variation - S is G strain AR37 or C strain RGT18
  source 1..102: mol_type = other DNA
gactagtactatattatagttaactactataactataactatatataactsctataaaactagcctagagatatataggaagtgaggctagccttagataac

SEQ ID NO: 400 - DNA, 102 bp, synthetic construct
  misc_feature 1..102: note = Epichloe festucae
  misc_feature 51: note = Variation - S is T strain AR37 or A strain RGT18
  source 1..102: mol_type = other DNA
attagtaatattatattacctatatataatacactaggcttctatttactsacctataactctaatatacccttaaggatcttaaggctaaaattactataa

SEQ ID NO: 401 - DNA, 102 bp, synthetic construct
  misc_feature 1..102: note = Epichloe festucae
  misc_feature 51: note = Variation - S is T strain AR37 or C strain RGT18
  source 1..102: mol_type = other DNA
ttttctgctttgcgaattcgccataatcgagtcgcgccgctcgcacgggasttgtgaacagaaggacgtgcgcacttctactccatcgggcgggtagaagct

SEQ ID NO: 402 - DNA, 102 bp, synthetic construct
  misc_feature 1..102: note = Epichloe festucae
  misc_feature 51: note = Variation - S is G strain AR37 or A strain RGT18
  source 1..102: mol_type = other DNA
aaggttaaggtcttttaactatagctaccttataataagtaatttaagaasagagaaaatcactatagcctaagactaaagaccctaaagactctaaggact

SEQ ID NO: 403 - DNA, 102 bp, synthetic construct
  misc_feature 1..102: note = Epichloe festucae
  misc_feature 51: note = Variation - S is C strain AR37 or T strain RGT18
  source 1..102: mol_type = other DNA
tctaggcatgttttcctttattatttagtagcataacctaggcctttaggsaatagtttttatagtaactaataaggttaggccttttttatagcatattta

SEQ ID NO: 404 - DNA, 102 bp, synthetic construct
  misc_feature 1..102: note = Epichloe festucae
  misc_feature 51: note = Variation - S is T strain AR37 or G strain RGT18
  source 1..102: mol_type = other DNA
atagacctttttaataaggctagagctaatagcttacctccttattaagastctcttaattactatatatacttatactaaaactaggataagtctaaacta

SEQ ID NO: 405 - DNA, 102 bp, synthetic construct
  misc_feature 1..102: note = Epichloe festucae
  misc_feature 51: note = Variation - S is T strain AR37 or C strain RGT18
  source 1..102: mol_type = other DNA
aagttcctaggtattataagttagctagatataaagagatactatagtctstagctataaaacttaaggcactctagtaaggtaagtaaggataagtatata

SEQ ID NO: 406 - DNA, 102 bp, synthetic construct
  misc_feature 1..102: note = Epichloe festucae
  misc_feature 51: note = Variation - S is A strain AR37 or G strain RGT18
  source 1..102: mol_type = other DNA
aggagacactctattccttattttaggcatactagtttataaaggtaaatstttatatagcgttttataagctatagattactaagggctaggagcacttta

SEQ ID NO: 407 - DNA, 102 bp, synthetic construct
  misc_feature 1..102: note = Epichloe festucae
  misc_feature 51: note = Variation - S is A strain AR37 or G strain RGT18
  source 1..102: mol_type = other DNA
tagaggtaacttactactaacttactaagtattatattagccttattatasgctttaactatactaatactacctattatattatatttagtttaactagta

SEQ ID NO: 408 - DNA, 102 bp, synthetic construct
  misc_feature 1..102: note = Epichloe festucae
  misc_feature 51: note = Variation - S is T strain AR37 or C strain RGT18
  source 1..102: mol_type = other DNA
gtccgcataacttcttctactatagactttaggataagggggcctaaggtsactctataacccttaaactataataacactgttttaattagggtttcctag

SEQ ID NO: 409 - DNA, 102 bp, synthetic construct
  misc_feature 1..102: note = Epichloe festucae
  misc_feature 51: note = Variation - S is T strain AR37 or C strain RGT18
  source 1..102: mol_type = other DNA
cttagccctaatacttagattaataaccttactatatatagaatctagctstataataagttttaattaaagttatagtgccttatagtattactttactat

SEQ ID NO: 410 - DNA, 102 bp, synthetic construct
  misc_feature 1..102: note = Epichloe festucae
  misc_feature 51: note = Variation - S is C strain AR37 or T strain RGT18
  source 1..102: mol_type = other DNA
cctaagatacctaagattaagtgtcttttcccttaggctttattatctaasctagctaaggcctatgcctctaagcgctatatttagtataagaagagaggt

SEQ ID NO: 411 - DNA, 102 bp, synthetic construct
  misc_feature 1..102: note = Epichloe festucae
  misc_feature 51: note = Variation - S is T strain AR37 or C strain RGT18
  source 1..102: mol_type = other DNA
ttatataattccttaggaatatctttaatagttttatatacttttacctcsttattatctttaagggtaataaacttattttctataactcctataatagta

SEQ ID NO: 412 - DNA, 102 bp, synthetic construct
  misc_feature 1..102: note = Epichloe festucae
  misc_feature 51: note = Variation - S is T strain AR37 or A strain RGT18
  source 1..102: mol_type = other DNA
tataacttcttatatagtgatttagtgcctttacctttaatctcttagatsatataagaattaaagatctagtagcctttatactttactagattaaatatt

SEQ ID NO: 413 - DNA, 102 bp, synthetic construct
  misc_feature 1..102: note = Epichloe festucae
  misc_feature 51: note = Variation - S is G strain AR37 or A strain RGT18
  source 1..102: mol_type = other DNA
ggatttactattataaggttatactaagtttactttaagagctactattasgtgtaaggtaagatttctaaagaaggttaattctttttatctagagtccga

SEQ ID NO: 414 - DNA, 102 bp, synthetic construct
  misc_feature 1..102: note = Epichloe festucae
  misc_feature 51: note = Variation - S is G strain AR37 or A strain RGT18
  source 1..102: mol_type = other DNA
tacaattattagtagcttcttacctcttttccctttaatctaggttagctsgattaaatcccttcgttctgattaattaatctaggttatctaactaatcta

SEQ ID NO: 415 - DNA, 102 bp, synthetic construct
  misc_feature 1..102: note = Epichloe festucae
  misc_feature 51: note = Variation - S is A strain AR37 or G strain RGT18
  source 1..102: mol_type = other DNA
gcacgattcattgcaggggccggccacctgcccccacgtgcgctgcgcccscctgcgcccacctgcgcccacctgcctgcgcccacctgcccccacctcgaa

SEQ ID NO: 416 - DNA, 102 bp, synthetic construct
  misc_feature 1..102: note = Epichloe festucae
  misc_feature 51: note = Variation - S is A strain AR37 or T strain RGT18
  source 1..102: mol_type = other DNA
tccaggttcaagtgcgcgcgcaccggaaaaacaatatgcatcgcccacgcsggccaccatgcgtgctgcgatcaaacagaagagcaacgattcatcggtggg

SEQ ID NO: 417 - DNA, 102 bp, synthetic construct
  misc_feature 1..102: note = Epichloe festucae
  misc_feature 51: note = Variation - S is C strain AR37 or T strain RGT18
  source 1..102: mol_type = other DNA
tattaatattataaagcttagtaatagggcactttccttagaataaaaagsacttcttctaattctaatagattcttacttttataagaattattactaata

SEQ ID NO: 418 - DNA, 102 bp, synthetic construct
  misc_feature 1..102: note = Epichloe festucae
  misc_feature 51: note = Variation - S is T strain AR37 or A strain RGT18
  source 1..102: mol_type = other DNA
tgtagttagtgtagtttaggggaaaaaatttatattatattatattgtagstttttcctgcttgtagttagtgtagtttgtagtgcaatactctgctcttag

SEQ ID NO: 419 - DNA, 102 bp, synthetic construct
  misc_feature 1..102: note = Epichloe festucae
  misc_feature 51: note = Variation - S is A strain AR37 or G strain RGT18
  source 1..102: mol_type = other DNA
aggttatggcagttattaactattattaactaatagaatttaatctagatsacttttacaatatcttatatactaatagaattgattttagtgacattatac

SEQ ID NO: 420 - DNA, 102 bp, synthetic construct
  misc_feature 1..102: note = Epichloe festucae
  misc_feature 51: note = Variation - S is A strain AR37 or G strain RGT18
  source 1..102: mol_type = other DNA
aaaaaaggaaaatattaccttaaaggcctatatataatttagctaagagasagctaaaggtccttagagagtaccttataagtatatagcttaaagggtaaa

SEQ ID NO: 421 - DNA, 102 bp, synthetic construct
  misc_feature 1..102: note = Epichloe festucae
  misc_feature 51: note = Variation - S is G strain AR37 or A strain RGT18
  source 1..102: mol_type = other DNA
ataattagactatcttaatagtatatttataattagactatcttaatagtstatttactaggttacttttccctagtctatacctaattataaagtaaaagg

SEQ ID NO: 422 - DNA, 102 bp, synthetic construct
  misc_feature 1..102: note = Epichloe festucae
  misc_feature 51: note = Variation - S is T strain AR37 or C strain RGT18
  source 1..102: mol_type = other DNA
gaaagcaacggctaaaaacgacaagaattttctcgtagtgggagcccacgsaccagtttatgctcgccattgttattgtgcccccttcttcgtagaatctac

SEQ ID NO: 423 - DNA, 102 bp, synthetic construct
  misc_feature 1..102: note = Epichloe festucae
  misc_feature 51: note = Variation - S is C strain AR37 or G strain RGT18
  source 1..102: mol_type = other DNA
aattactttctctatagtatagtaaaagtaataaactactataacctaggstatatacctagggttagagagctagagctaaaggacttatcttacctccta

SEQ ID NO: 424 - DNA, 102 bp, synthetic construct
  misc_feature 1..102: note = Epichloe festucae
  misc_feature 51: note = Variation - S is A strain AR37 or G strain RGT18
  source 1..102: mol_type = other DNA
attatagatttaagtaagaaagctatagataagttactaatagttataagsacccacttatggacccacttttattaaaaccgattaaaaaccctctcttta

SEQ ID NO: 425 - DNA, 102 bp, synthetic construct
  misc_feature 1..102: note = Epichloe festucae
  misc_feature 51: note = Variation - S is T strain AR37 or A strain RGT18
  source 1..102: mol_type = other DNA
agtttagcaattccagtggtagcaagaatagcattaacaggacctttaggscctaaggacctaatatctatagcagtagtagcaattagagtagcaattata

SEQ ID NO: 426 - DNA, 102 bp, synthetic construct
  misc_feature 1..102: note = Epichloe festucae
  misc_feature 51: note = Variation - S is G strain AR37 or C strain RGT18
  source 1..102: mol_type = other DNA
ccacccaccatcatcagaagtgggcaacaatgtatctccatcacagatccsaaaccaccacgtctcattcgtctcgtctcaacgagtcaatcgcccccttca

SEQ ID NO: 427 - DNA, 102 bp, synthetic construct
  misc_feature 1..102: note = Epichloe festucae
  misc_feature 51: note = Variation - S is T strain AR37 or C strain RGT18
  source 1..102: mol_type = other DNA
aagtattaagaaataatatagtttaactaaagtaaaagtagctataattasatagagtgttaggaagctctaaaaaatagtttaatctaataacacggtggt

SEQ ID NO: 428 - DNA, 102 bp, synthetic construct
  misc_feature 1..102: note = Epichloe festucae
  misc_feature 51: note = Variation - S is C strain AR37 or A strain RGT18
  source 1..102: mol_type = other DNA
taaatcttaaactataaattaaaatattataaactatttatactttatagstaaaaatattctaatagtaaggcttctaaatatttatagctgatactttac

SEQ ID NO: 429 - DNA, 102 bp, synthetic construct
  misc_feature 1..102: note = Epichloe festucae
  misc_feature 51: note = Variation - S is A strain AR37 or T strain RGT18
  source 1..102: mol_type = other DNA
aaaaccttccgttgcgttgcgttaaatatttaacgtagtggttctattagsccctaaccgtagagctgcacctgtacagctgttgccagccagcaactagct

SEQ ID NO: 430 - DNA, 102 bp, synthetic construct
  misc_feature 1..102: note = Epichloe festucae
  misc_feature 51: note = Variation - S is G strain AR37 or A strain RGT18
  source 1..102: mol_type = other DNA
agcaaaatagcctaggataggcatattattagactagatttacactaggasggggtatagttacccttattttagtaaatctttcctttatctttcttttct

SEQ ID NO: 431 - DNA, 102 bp, synthetic construct
  misc_feature 1..102: note = Epichloe festucae
  misc_feature 51: note = Variation - S is C strain AR37 or T strain RGT18
  source 1..102: mol_type = other DNA
gattagttaagatcttattagaataaagcttaaaaagaataatcctacctstttactattagctataggctaggaaaataagcagtttaaagtaaaaacacc

SEQ ID NO: 432 - DNA, 102 bp, synthetic construct
  misc_feature 1..102: note = Epichloe festucae
  misc_feature 51: note = Variation - S is C strain AR37 or T strain RGT18
  source 1..102: mol_type = other DNA
tagactattttaagtacttaatactataggaaaataagcttactaacttasactacctaagaagtatagctaactatataatatattttatattagcttact

SEQ ID NO: 433 - DNA, 102 bp, synthetic construct
  misc_feature 1..102: note = Epichloe festucae
  misc_feature 51: note = Variation - S is T strain AR37 or C strain RGT18
  source 1..102: mol_type = other DNA
ttcctataataattatattatctatatatagaagaagtataatattattasattaaaaaatacagagtttgcttaatagcctcttaaagccttactatttaa

SEQ ID NO: 434 - DNA, 102 bp, synthetic construct
  misc_feature 1..102: note = Epichloe festucae
  misc_feature 51: note = Variation - S is T strain AR37 or C strain RGT18
  source 1..102: mol_type = other DNA
ttaatagattaccttagagggaattaactagtaatatttaaactaaaaccstataagttagtagtatttaaagaactttaataaagattttaaaaagcgcta

SEQ ID NO: 435 - DNA, 102 bp, synthetic construct
  misc_feature 1..102: note = Epichloe festucae
  misc_feature 51: note = Variation - S is C strain AR37 or G strain RGT18
  source 1..102: mol_type = other DNA
tacactatataaatagtgtttactagcttatatagtgctttataaatatasctttaaaaagtaactaaggtattagttagcctaaagggtattataagatat

SEQ ID NO: 436 - DNA, 102 bp, synthetic construct
  misc_feature 1..102: note = Epichloe festucae
  misc_feature 51: note = Variation - S is G strain AR37 or A strain RGT18
  source 1..102: mol_type = other DNA
ctttaagtgtaaagttactagatattatactataaactatattataactasaaataatttattataataataggaattcttatagttaaaattaataatact

SEQ ID NO: 437 - DNA, 102 bp, synthetic construct
  misc_feature 1..102: note = Epichloe festucae
  misc_feature 51: note = Variation - S is G strain AR37 or A strain RGT18
  source 1..102: mol_type = other DNA
tatatatagtacactaggcttttatttactaacccttatctctattatatsttaaaggatattaaggcaaagattaccttaggtatatatattattaaacct

SEQ ID NO: 438 - DNA, 102 bp, synthetic construct
  misc_feature 1..102: note = Epichloe festucae
  misc_feature 51: note = Variation - S is C strain AR37 or T strain RGT18
  source 1..102: mol_type = other DNA
aactattttactagctaatataaagtaaatatagtattttattacctttastatatataggctattatagcttatactaaataagtacttttttaaaggtac

SEQ ID NO: 439 - DNA, 102 bp, synthetic construct
  misc_feature 1..102: note = Epichloe festucae
  misc_feature 51: note = Variation - S is G strain AR37 or C strain RGT18
  source 1..102: mol_type = other DNA
attaagatatagataaaaatacctatatataaagagaaaatatataaaagsttataaaatttcttagtaaacttaaataaattatttaaattaaattactat

SEQ ID NO: 440 - DNA, 102 bp, synthetic construct
  misc_feature 1..102: note = Epichloe festucae
  misc_feature 51: note = Variation - S is T strain AR37 or C strain RGT18
  source 1..102: mol_type = other DNA
gcttagtattaaaccacttcttataatttaaatatactttatataagtatstaatatactctttatatttctcttaagataatatatttaaaagagatataa

SEQ ID NO: 441 - DNA, 102 bp, synthetic construct
  misc_feature 1..102: note = Epichloe festucae
  misc_feature 51: note = Variation - S is A strain AR37 or G strain RGT18
  source 1..102: mol_type = other DNA
acgctgcggttgtactcgttagaacagcagcgcgaccgtcacggcggaggscataacttgcacatacaggcaacgatcatctacgacctttatgacactgcg

SEQ ID NO: 442 - DNA, 102 bp, synthetic construct
  misc_feature 1..102: note = Epichloe festucae
  misc_feature 51: note = Variation - S is G strain AR37 or C strain RGT18
  source 1..102: mol_type = other DNA
atattaacactctttacctaattatatcttactagcttagatattttaccsttttaggttttattatctttatttattttaactacttaatatacttagagt

SEQ ID NO: 443 - DNA, 102 bp, synthetic construct
  misc_feature 1..102: note = Epichloe festucae
  misc_feature 51: note = Variation - S is C strain AR37 or T strain RGT18
  source 1..102: mol_type = other DNA
ttattaactttataataaacttactagcatttagattaattaggaaaattstagataatattatgctccttagttaggattaattagttactttttatatta

SEQ ID NO: 444 - DNA, 102 bp, synthetic construct
  misc_feature 1..102: note = Epichloe festucae
  misc_feature 51: note = Variation - S is A strain AR37 or G strain RGT18
  source 1..102: mol_type = other DNA
tatatagttcttttataaggatataaggctagtaaagtagtaggtaactasgtatataacgctatcctagccttactaggaaaggttagcttttactactat

SEQ ID NO: 445 - DNA, 102 bp, synthetic construct
  misc_feature 1..102: note = Epichloe festucae
  misc_feature 51: note = Variation - S is A strain AR37 or G strain RGT18
  source 1..102: mol_type = other DNA
taagtttataaaggtaatatataataagactattatatatactattataasagttatagaagataaatttattacccttaaagataagaaaaaagtaaaagt

SEQ ID NO: 446 - DNA, 102 bp, synthetic construct
  misc_feature 1..102: note = Epichloe festucae
  misc_feature 51: note = Variation - S is C strain AR37 or A strain RGT18
  source 1..102: mol_type = other DNA
ttatatatttttaataaagcttattaagcctttagagtttattttagtttstttcttaagactttttctttttaaattaatagcttttctaattatattatc

SEQ ID NO: 447 - DNA, 102 bp, synthetic construct
  misc_feature 1..102: note = Epichloe festucae
  misc_feature 51: note = Variation - S is A strain AR37 or T strain RGT18
  source 1..102: mol_type = other DNA
cttctcccgacccttgtatcccctaccaaaaaaaaaaaaaaaaaaaaaaasgtcccatcgacatgccccttcagtccgtagcgatattccacagcccatcgc

SEQ ID NO: 448 - DNA, 102 bp, synthetic construct
  misc_feature 1..102: note = Epichloe festucae
  misc_feature 51: note = Variation - S is A strain AR37 or G strain RGT18
  source 1..102: mol_type = other DNA
agctagctatagtttacattaggactaatacttagttagtctaaggtatasgtttagctagctatagtttatattagaactagtacttattctctatagtaa

SEQ ID NO: 449 - DNA, 102 bp, synthetic construct
  misc_feature 1..102: note = Epichloe festucae
  misc_feature 51: note = Variation - S is T strain AR37 or C strain RGT18
  source 1..102: mol_type = other DNA
ctagataaatactagctaggggcaggtatataaaggttttaatctctaacstagcactaataatatatatagtctttaataaataccttactctacaagcac

SEQ ID NO: 450 - DNA, 102 bp, synthetic construct
  misc_feature 1..102: note = Epichloe festucae
  misc_feature 51: note = Variation - S is C strain AR37 or A strain RGT18
  source 1..102: mol_type = other DNA
actagatagtagcccttaattaatctagaatagtacaaattaaacgctttsctaatctattttgcttatagatatagggactagaagttataaatttaatcc

SEQ ID NO: 451 - DNA, 102 bp, synthetic construct
  misc_feature 1..102: note = Epichloe festucae
  misc_feature 51: note = Variation - S is A strain AR37 or G strain RGT18
  source 1..102: mol_type = other DNA
atatataagtagtttactacgcttctctaagctttaataccttattactasgataaaatctagtaatatatttaaattactaggttaagtaataaatctctt

SEQ ID NO: 452 - DNA, 102 bp, synthetic construct
  misc_feature 1..102: note = Epichloe festucae
  misc_feature 51: note = Variation - S is G strain AR37 or A strain RGT18
  source 1..102: mol_type = other DNA
tccttaatattcttatattatctaatagtaatattttctaaccttagctasataatctccttaagtatagtaataactatagctatattttattatttttct

SEQ ID NO: 453 - DNA, 102 bp, synthetic construct
  misc_feature 1..102: note = Epichloe festucae
  misc_feature 51: note = Variation - S is C strain AR37 or A strain RGT18
  source 1..102: mol_type = other DNA
attaaacctaactaagccacaaagctaagggattagcctatacctataagsttacttaacctcttaattaacttactagggatgtaagctagtaatagggag

SEQ ID NO: 454 - DNA, 102 bp, synthetic construct
  misc_feature 1..102: note = Epichloe festucae
  misc_feature 51: note = Variation - S is T strain AR37 or C strain RGT18
  source 1..102: mol_type = other DNA
taaggtcttataaagccattccctatgtctatttattagttatatataaasaatttaccactctctcctatagttataaatctaaatctttatttactatat

SEQ ID NO: 455 - DNA, 102 bp, synthetic construct
  misc_feature 1..102: note = Epichloe festucae
  misc_feature 51: note = Variation - S is C strain AR37 or A strain RGT18
  source 1..102: mol_type = other DNA
attaaatcttactaacttacttttaagaagactagattttataagtaaggsaagaaaagagaaagtaataactatataacttcttacctttttatttaaatt

SEQ ID NO: 456 - DNA, 102 bp, synthetic construct
  misc_feature 1..102: note = Epichloe festucae
  misc_feature 51: note = Variation - S is C strain AR37 or G strain RGT18
  source 1..102: mol_type = other DNA
gattgttgagatggcgtacctgcgtacgttcgacccttatcaaaacaaaasaaaagaaaaagcatcggtccgctatgcgcggaccgggcaaacccaaagaaa

SEQ ID NO: 457 - DNA, 102 bp, synthetic construct
  misc_feature 1..102: note = Epichloe festucae
  misc_feature 51: note = Variation - S is A strain AR37 or C strain RGT18
  source 1..102: mol_type = other DNA
aaacttttatttattatctttaatagtatcttatagtaagaacgcattttstatatttattaagtcccctttaaaaggtttaagactagtaatattaaatat

SEQ ID NO: 458 - DNA, 102 bp, synthetic construct
  misc_feature 1..102: note = Epichloe festucae
  misc_feature 51: note = Variation - S is G strain AR37 or A strain RGT18
  source 1..102: mol_type = other DNA
agtattattaatatactcctaaaaagttactaatatattaactagtttaastagtattactagatatttaaagtaactatattaataataaaacactatttt

SEQ ID NO: 459 - DNA, 102 bp, synthetic construct
  misc_feature 1..102: note = Epichloe festucae
  misc_feature 51: note = Variation - S is C strain AR37 or G strain RGT18
  source 1..102: mol_type = other DNA
ctactctttatattatctttatttaattatctcttatttatttagcactastcttaactcctttatgttcttagagataattaattatataggataatttta

SEQ ID NO: 460 - DNA, 102 bp, synthetic construct
  misc_feature 1..102: note = Epichloe festucae
  misc_feature 51: note = Variation - S is C strain AR37 or T strain RGT18
  source 1..102: mol_type = other DNA
cctttagatattatatactaggataagttccctagttttaattaatctttsctaagagaaatagcttagttcttattagtttagtttataaggcattgccta

SEQ ID NO: 461 - DNA, 102 bp, synthetic construct
  misc_feature 1..102: note = Epichloe festucae
  misc_feature 51: note = Variation - S is G strain AR37 or A strain RGT18
  source 1..102: mol_type = other DNA
atttaaataagaaaatcttgtttttatatatattttacttatttaattatsaatttctaaaactttagcttatttagaataataagctaagaataggctaag

SEQ ID NO: 462 - DNA, 102 bp, synthetic construct
  misc_feature 1..102: note = Epichloe festucae
  misc_feature 51: note = Variation - S is T strain AR37 or C strain RGT18
  source 1..102: mol_type = other DNA
aagttattttatataactattaatcttttacttctaaaaagatctcctagsttagcaaagagtctagaatactagattattctaatctagtttatgtgtaaa

SEQ ID NO: 463 - DNA, 102 bp, synthetic construct
  misc_feature 1..102: note = Epichloe festucae
  misc_feature 51: note = Variation - S is A strain AR37 or G strain RGT18
  source 1..102: mol_type = other DNA
taaattaaaactagaataatactaataatagaatacttatagtatttagtsatattttattataaatttctatataaaatattagtaattaaactagtatta

SEQ ID NO: 464 - DNA, 102 bp, synthetic construct
  misc_feature 1..102: note = Epichloe festucae
  misc_feature 51: note = Variation - S is T strain AR37 or G strain RGT18
  source 1..102: mol_type = other DNA
ttatattacttaaatatattactttaagtattaagaaactatataacttasaagtctctttattcttattatagatattatccttataatatttaattatta

SEQ ID NO: 465 - DNA, 102 bp, synthetic construct
  misc_feature 1..102: note = Epichloe festucae
  misc_feature 51: note = Variation - S is A strain AR37 or T strain RGT18
  source 1..102: mol_type = other DNA
ataataagacgcttgaaaagcttgtgaaagacttgctaggacctaaatggsaaccatgcccggcgtggctcaaatgtttgtcgatctgtcacacatgccatt

SEQ ID NO: 466 - DNA, 102 bp, synthetic construct
  misc_feature 1..102: note = Epichloe festucae
  misc_feature 51: note = Variation - S is G strain AR37 or A strain RGT18
  source 1..102: mol_type = other DNA
ataatagcgaagttagggataaaagataatattataactataatagcttasattaccttataaataagtatagtaagctaaggaaagagccctaagatagct

SEQ ID NO: 467 - DNA, 102 bp, synthetic construct
  misc_feature 1..102: note = Epichloe festucae
  misc_feature 51: note = Variation - S is G strain AR37 or T strain RGT18
  source 1..102: mol_type = other DNA
ctgttactcttcccagaccgttgactagcgctgcgaccttttttttttttstttttttttttttttgtttcgagaaaggacatgagttgatgaggggccaac

SEQ ID NO: 468 - DNA, 102 bp, synthetic construct
  misc_feature 1..102: note = Epichloe festucae
  misc_feature 51: note = Variation - S is A strain AR37 or G strain RGT18
  source 1..102: mol_type = other DNA
tgctactataaatatttataattaaactaatagaagattttaacttaaatsctctatagtaattaattagtttaaaagctagaaaactttattctaattact

SEQ ID NO: 469 - DNA, 102 bp, synthetic construct
  misc_feature 1..102: note = Epichloe festucae
  misc_feature 51: note = Variation - S is A strain AR37 or G strain RGT18
  source 1..102: mol_type = other DNA
atctctttatatattatagttagtttactaataacttattagttttattasaataaaacacttatagcttactatatagagtaagctatactatagctagct

SEQ ID NO: 470 - DNA, 102 bp, synthetic construct
  misc_feature 1..102: note = Epichloe festucae
  misc_feature 51: note = Variation - S is G strain AR37 or A strain RGT18
  source 1..102: mol_type = other DNA
gaaaataagccttattactaaaggataaggactttaaatgtatagcttatsattaatctaaggtagtacaaagacctaggaagttagctatccctaaccccc

SEQ ID NO: 471 - DNA, 102 bp, synthetic construct
  misc_feature 1..102: note = Epichloe festucae
  misc_feature 51: note = Variation - S is T strain AR37 or A strain RGT18
  source 1..102: mol_type = other DNA
tatctcaaagcgttatgcaggggactaatataatgagccgagtattatatsgagaaagaaggcaacccgcaactggtctagtcaacaatggtggttccatct

SEQ ID NO: 472 - DNA, 102 bp, synthetic construct
  misc_feature 1..102: note = Epichloe festucae
  misc_feature 51: note = Variation - S is G strain AR37 or A strain RGT18
  source 1..102: mol_type = other DNA
aggagagagctcttagaatacctataataagatagctaatagtagcttagsatagaataaataataaggacttattattaagaagtagtattataatagaga

SEQ ID NO: 473 - DNA, 102 bp, synthetic construct
  misc_feature 1..102: note = Epichloe festucae
  misc_feature 51: note = Variation - S is C strain AR37 or T strain RGT18
  source 1..102: mol_type = other DNA
aaatcggaagggccaagctttgaactgactctgctcctgggccatgtctcsatgctcacttccctcgttgtcgcggagagccaaggaaagaagtacatcttg

SEQ ID NO: 474 - DNA, 102 bp, synthetic construct
  misc_feature 1..102: note = Epichloe festucae
  misc_feature 51: note = Variation - S is C strain AR37 or T strain RGT18
  source 1..102: mol_type = other DNA
gcatggaccggtaacgtttttcctgaaagaatgagccaagtcagttagagscagattggaggcacgaggcaaagtgccgtttgaagaacgtttggcgcaatc

SEQ ID NO: 475 - DNA, 102 bp, synthetic construct
  misc_feature 1..102: note = Epichloe festucae
  misc_feature 51: note = Variation - S is C strain AR37 or T strain RGT18
  source 1..102: mol_type = other DNA
accatgcccatccgttgcatgaataattgcacccctctccagaagcagacsgacgatgctcgcatgtccttcacaagcagcccatgagagaggagtacggcc

SEQ ID NO: 476 - DNA, 102 bp, synthetic construct
  misc_feature 1..102: note = Epichloe festucae
  misc_feature 51: note = Variation - S is A strain AR37 or G strain RGT18
  source 1..102: mol_type = other DNA
ctatagggtaacctgcttacgtcaccctagcttacctaattactagtggcsctgcggttgtggctacgcttgcagccataacgcaattaaataatccataat

SEQ ID NO: 477 - DNA, 102 bp, synthetic construct
  misc_feature 1..102: note = Epichloe festucae
  misc_feature 51: note = Variation - S is C strain AR37 or G strain RGT18
  source 1..102: mol_type = other DNA
tctctccgaattcttctcaccgacctcaacttgcagacagaacctcccccscccccccccccccccgcccccacccccaccatgtcgtcagccctcatctcc

SEQ ID NO: 478 - DNA, 102 bp, synthetic construct
  misc_feature 1..102: note = Epichloe festucae
  misc_feature 51: note = Variation - S is A strain AR37 or G strain RGT18
  source 1..102: mol_type = other DNA
gtagctttatataagtaagtaaattactaattatatctcttaaatatatasaaggtttagtaaatttattataataaagcctcttattataaataaagctat

SEQ ID NO: 479 - DNA, 102 bp, synthetic construct
  misc_feature 1..102: note = Epichloe festucae
  misc_feature 51: note = Variation - S is T strain AR37 or A strain RGT18
  source 1..102: mol_type = other DNA
aataaaattaaggctttagctaagctaactaatcttctaatttaccctttsagctatatacttaactaatcttttaatttaccctttaagctatatacttat

SEQ ID NO: 480 - DNA, 102 bp, synthetic construct
  misc_feature 1..102: note = Epichloe festucae
  misc_feature 51: note = Variation - S is C strain AR37 or A strain RGT18
  source 1..102: mol_type = other DNA
gagactatagtataagttaaaatataccctagtctaattacctaactatastagcttactattaaagtattatactagatattaagtcttactaattagaga

SEQ ID NO: 481 - DNA, 102 bp, synthetic construct
  misc_feature 1..102: note = Epichloe festucae
  misc_feature 51: note = Variation - S is T strain AR37 or A strain RGT18
  source 1..102: mol_type = other DNA
atatttactatacttaaatatttactaatattacttataaggtaaaatatsataaatatactataatagtattactaagtaatactataaatttaaagacct

SEQ ID NO: 482 - DNA, 102 bp, synthetic construct
  misc_feature 1..102: note = Epichloe festucae
  misc_feature 51: note = Variation - S is G strain AR37 or A strain RGT18
  source 1..102: mol_type = other DNA
aggggtgcatgctcgagaaactgcccaacttgttctattccatgggctacstcgacgcgagctggacgctcggcgccgacgccaccgcccagctcgtctgcc

SEQ ID NO: 483 - DNA, 102 bp, synthetic construct
  misc_feature 1..102: note = Epichloe festucae
  misc_feature 51: note = Variation - S is A strain AR37 or T strain RGT18
  source 1..102: mol_type = other DNA
taatagctctattaatattagaagctaaagctaacgctatctgcgagaccstccgggagctacagtggcttcagggcttgattaatattagaagctaaagct

SEQ ID NO: 484 - DNA, 102 bp, synthetic construct
  misc_feature 1..102: note = Epichloe festucae
  misc_feature 51: note = Variation - S is T strain AR37 or A strain RGT18
  source 1..102: mol_type = other DNA
ttatagtaagctttaaggagtaatttaagtaagaaaagagtttaattattsgtctagtaaatttaggaggatttagatgcctataactaggtgctttaggat

SEQ ID NO: 485 - DNA, 102 bp, synthetic construct
  misc_feature 1..102: note = Epichloe festucae
  misc_feature 51: note = Variation - S is G strain AR37 or T strain RGT18
  source 1..102: mol_type = other DNA
tattttaaaagcaaggacgcggggtttggaaagagaacggaagtctggggsttttttttttttttttttttttgctagccatgctttagtaaattttttttt

SEQ ID NO: 486 - DNA, 102 bp, synthetic construct
  misc_feature 1..102: note = Epichloe festucae
  misc_feature 51: note = Variation - S is C strain AR37 or T strain RGT18
  source 1..102: mol_type = other DNA
taataaaaaagggagttattacctaacttactatagtaataagggataagsacttagataagggtaataaactatttatatatttctttatatatagtgttt

SEQ ID NO: 487 - DNA, 102 bp, synthetic construct
  misc_feature 1..102: note = Epichloe festucae
  misc_feature 51: note = Variation - S is A strain AR37 or T strain RGT18
  source 1..102: mol_type = other DNA
aattatgttataaaaaatcagatgcattggctatagccaatgaggtaaaastttttttttttaaaatcaataaatcaataattgttagtatctattaggata

SEQ ID NO: 488 - DNA, 102 bp, synthetic construct
  misc_feature 1..102: note = Epichloe festucae
  misc_feature 51: note = Variation - S is A strain AR37 or T strain RGT18
  source 1..102: mol_type = other DNA
taaggagagtatttgttgtgctgaagtctgacggtggtggtggtggtgacsgcagaataggcaaggagaagccaggagaagcataagctccggaaccgggtt

SEQ ID NO: 489 - DNA, 102 bp, synthetic construct
  misc_feature 1..102: note = Epichloe festucae
  misc_feature 51: note = Variation - S is T strain AR37 or G strain RGT18
  source 1..102: mol_type = other DNA
aaaggtcctaatatcttaagataagggtaacttatatagctctattatagsctaataagtaagtattttaaatataggttttctaaatgctagtaaaggtag

SEQ ID NO: 490 - DNA, 102 bp, synthetic construct
  misc_feature 1..102: note = Epichloe festucae
  misc_feature 51: note = Variation - S is A strain AR37 or T strain RGT18
  source 1..102: mol_type = other DNA
aaaaatagtttactaaggtaactatagctatatttatttatacttataaasgactaggaagagcttatttaactagacctagagattactatatagcctaag

SEQ ID NO: 491 - DNA, 102 bp, synthetic construct
  misc_feature 1..102: note = Epichloe festucae
  misc_feature 51: note = Variation - S is G strain AR37 or A strain RGT18
  source 1..102: mol_type = other DNA
ttaaaggactcttatagttcttataagtagagcttaaagtaataactaatscttaaatccttactaaacatatataactatttaaatttaatattatattag

SEQ ID NO: 492 - DNA, 102 bp, synthetic construct
  misc_feature 1..102: note = Epichloe festucae
  misc_feature 51: note = Variation - S is A strain AR37 or G strain RGT18
  source 1..102: mol_type = other DNA
tcaacatggcgcaggcaaagaagaacctcctgctccttacgattagggaasttgacgcagaatggaaaaggagaaagtcaggtaggatatttgcgtatcggc

SEQ ID NO: 493 - DNA, 102 bp, synthetic construct
  misc_feature 1..102: note = Epichloe festucae
  misc_feature 51: note = Variation - S is T strain AR37 or A strain RGT18
  source 1..102: mol_type = other DNA
aagaactatattcgtatttcttaagatctatatatacttactttagtgtasaatttacactataaagttaattaactataaatataatattaggttatataa

SEQ ID NO: 494 - DNA, 102 bp, synthetic construct
  misc_feature 1..102: note = Epichloe festucae
  misc_feature 51: note = Variation - S is A strain AR37 or T strain RGT18
  source 1..102: mol_type = other DNA
ttaattttattctattagtttagggtattttttatttaaaataataataasaaaatataaaaatataaaataattaataataatagtaaataaaataataag

SEQ ID NO: 495 - DNA, 102 bp, synthetic construct
  misc_feature 1..102: note = Epichloe festucae
  misc_feature 51: note = Variation - S is C strain AR37 or T strain RGT18
  source 1..102: mol_type = other DNA
gatggcgttgaccccacgcggacatacaccaacgacctgtggcagattgtsgaggtgtttggcattgaagctgcccgttctgctctggtgaaggagctgacc

SEQ ID NO: 496 - DNA, 102 bp, synthetic construct
  misc_feature 1..102: note = Epichloe festucae
  misc_feature 51: note = Variation - S is T strain AR37 or C strain RGT18
  source 1..102: mol_type = other DNA
ccagagtattgcactacaattgatttgtagtgtattttttatttaacaaasaatatatatctaatcttagaaaatatgtaaagatataaaacttcttttttt

SEQ ID NO: 497 - DNA, 102 bp, synthetic construct
  misc_feature 1..102: note = Epichloe festucae
  misc_feature 51: note = Variation - S is C strain AR37 or A strain RGT18
  source 1..102: mol_type = other DNA
attagtaatttagtattactagaattttatattaagattataatagaatcstactattaatttaactaggtttaacctgatttttactataatagtaacatt

SEQ ID NO: 498 - DNA, 102 bp, synthetic construct
  misc_feature 1..102: note = Epichloe festucae
  misc_feature 51: note = Variation - S is G strain AR37 or A strain RGT18
  source 1..102: mol_type = other DNA
tagtgtttagctttgctaaagcctaatcttatataaagtaattaagatagsaaacaggagtttaatagtttcctaggatagattagtgttaataaaggataa

SEQ ID NO: 499 - DNA, 102 bp, synthetic construct
  misc_feature 1..102: note = Epichloe festucae
  misc_feature 51: note = Variation - S is T strain AR37 or C strain RGT18
  source 1..102: mol_type = other DNA
agatctttaaaataagtctaggtaaggatatattagtaaagtttaagtttsctcttttatcctagtaattataatcttttcctatctataatatttaatagc

SEQ ID NO: 500 - DNA, 102 bp, synthetic construct
  misc_feature 1..102: note = Epichloe festucae
  misc_feature 51: note = Variation - S is T strain AR37 or C strain RGT18
  source 1..102: mol_type = other DNA
ttccttctaaaatcctatataagcttagatagtaatcctaaatagcttagsacctaattaatactcttaaagtaacttagtgttataattattagctatagg

SEQ ID NO: 501 - DNA, 102 bp, synthetic construct
  misc_feature 1..102: note = Epichloe festucae
  misc_feature 51: note = Variation - S is C strain AR37 or T strain RGT18
  source 1..102: mol_type = other DNA
cccaagcgacccaggcggccataatcttaaacagcatttcccttttgcaasacgctcgaatgttttcctaaaaagtgaacaagtaatcattgtctagatagg

SEQ ID NO: 502 - DNA, 102 bp, synthetic construct
  misc_feature 1..102: note = Epichloe festucae
  misc_feature 51: note = Variation - S is A strain AR37 or C strain RGT18
  source 1..102: mol_type = other DNA
taataagataatagcatagaattattactctctcctattaattaagaaaasactttacttcttattttaggtatattagtttataaaggtaaatatttatat

SEQ ID NO: 503 - DNA, 102 bp, synthetic construct
  misc_feature 1..102: note = Epichloe festucae
  misc_feature 51: note = Variation - S is T strain AR37 or C strain RGT18
  source 1..102: mol_type = other DNA
tactatataaataactagattagagaattaactaataaaactaaggatagsaaggactatagtatagacttagtaatatacttaaatagtgtgggttatacg

SEQ ID NO: 504 - DNA, 102 bp, synthetic construct
  misc_feature 1..102: note = Epichloe festucae
  misc_feature 51: note = Variation - S is T strain AR37 or C strain RGT18
  source 1..102: mol_type = other DNA
ccttaataaaattagctatattttctcctaaaaactactaaatattatacstattttatatagtaataagagaagtttaatatactattatttctctaagaa

SEQ ID NO: 505 - DNA, 102 bp, synthetic construct
  misc_feature 1..102: note = Epichloe festucae
  misc_feature 51: note = Variation - S is T strain AR37 or A strain RGT18
  source 1..102: mol_type = other DNA
ataaagagattaaatagtaaagctattttataaagagattaagctataatstaaagccttagagggcattatatttaatagagaattagtctttataagtta

SEQ ID NO: 506 - DNA, 102 bp, synthetic construct
  misc_feature 1..102: note = Epichloe festucae
  misc_feature 51: note = Variation - S is T strain AR37 or C strain RGT18
  source 1..102: mol_type = other DNA
attattaggtactgcattttcagtattaataagattagaattaagtggacsaggagttcaattcatatcaaataaccaattatataatagtatcgttacagc

SEQ ID NO: 507 - DNA, 102 bp, synthetic construct
  misc_feature 1..102: note = Epichloe festucae
  misc_feature 51: note = Variation - S is G strain AR37 or A strain RGT18
  source 1..102: mol_type = other DNA
aataatctagtattctaaaatctttactaagctaggagatctttttaaaastagaaaattaatagttatataaaataactttaagatctaatattataaggt

SEQ ID NO: 508 - DNA, 102 bp, synthetic construct
  misc_feature 1..102: note = Epichloe festucae
  misc_feature 51: note = Variation - S is T strain AR37 or C strain RGT18
  source 1..102: mol_type = other DNA
ctaaccatctgctatctagtccaattcgctcttcttcgtgtctacgcagtsaaacttgctcctctccctctcccaagcggcgtgacttaacttcttagtcac

SEQ ID NO: 509 - DNA, 102 bp, synthetic construct
  misc_feature 1..102: note = Epichloe festucae
  misc_feature 51: note = Variation - S is G strain AR37 or A strain RGT18
  source 1..102: mol_type = other DNA
agttatcttctataataatctattctcctagctaaatggcaattttgcctsgttttctatgggtaattaggtattaccttctagcactattttaacgtgctt

SEQ ID NO: 510 - DNA, 102 bp, synthetic construct
  misc_feature 1..102: note = Epichloe festucae
  misc_feature 51: note = Variation - S is T strain AR37 or C strain RGT18
  source 1..102: mol_type = other DNA
tcaacaacaacctccaatatagacagttgtgacaccccagtaaaatctctsccaattaatgcaatagggtatcaaaacaagaggctcaaaagacaaaggaga

SEQ ID NO: 511 - DNA, 102 bp, synthetic construct
  misc_feature 1..102: note = Epichloe festucae
  misc_feature 51: note = Variation - S is C strain AR37 or T strain RGT18
  source 1..102: mol_type = other DNA
aactttaagaaaaaccttctaattattttatttactattattattaattastttatatttttattattaatttaattaaaaaataccctaaactaatataat

SEQ ID NO: 512 - DNA, 102 bp, synthetic construct
  misc_feature 1..102: note = Epichloe festucae
  misc_feature 51: note = Variation - S is T strain AR37 or C strain RGT18
  source 1..102: mol_type = other DNA
tctataggaatccttattttcttattataaagaaagataaagggatttacstaattctatttactataaagtataataaggtaataatataagatatgctaa

SEQ ID NO: 513 - DNA, 102 bp, synthetic construct
  misc_feature 1..102: note = Epichloe festucae
  misc_feature 51: note = Variation - S is C strain AR37 or T strain RGT18
  source 1..102: mol_type = other DNA
atattataatattgcaatttttagcaatatagcctttattttttgccttasgtaaagattttaaccaagtcttgtataatccttggttattcttgataataa

SEQ ID NO: 514 - DNA, 102 bp, synthetic construct
  misc_feature 1..102: note = Epichloe festucae
  misc_feature 51: note = Variation - S is G strain AR37 or C strain RGT18
  source 1..102: mol_type = other DNA
gtttgacatggaatgcaagcagcaggacattttcgacttctccattcgtcscactgttgacgacatcttgaacggctacaatggcactgtcttcgcctacgg

SEQ ID NO: 515 - DNA, 102 bp, synthetic construct
  misc_feature 1..102: note = Epichloe festucae
  misc_feature 51: note = Variation - S is T strain AR37 or C strain RGT18
  source 1..102: mol_type = other DNA
ggatgatgtggagaagtagactcacttctaagactgcgatacggaatagtsagggaaagcggagctttgccgcaaatggacaaatggacaaatagacgaata

SEQ ID NO: 516 - DNA, 102 bp, synthetic construct
  misc_feature 1..102: note = Epichloe festucae
  misc_feature 51: note = Variation - S is C strain AR37 or T strain RGT18
  source 1..102: mol_type = other DNA
tagttagttttctcatatagataataagattaataattaactaaatatccsggatagatataataaggttatatcctataagcctaagggttaatagattaa

SEQ ID NO: 517 - DNA, 102 bp, synthetic construct
  misc_feature 1..102: note = Epichloe festucae
  misc_feature 51: note = Variation - S is A strain AR37 or G strain RGT18
  source 1..102: mol_type = other DNA
tagctagtagcttgctagtgttacataaacctagccctagagccttactascctataaggtgcataggtatacctattattgtaagtaaggccttataatta

SEQ ID NO: 518 - DNA, 102 bp, synthetic construct
  misc_feature 1..102: note = Epichloe festucae
  misc_feature 51: note = Variation - S is T strain AR37 or C strain RGT18
  source 1..102: mol_type = other DNA
atccttcttatttacatttgtaagggcttagactttgcctaagcattgtcsgtatagtagttagagaggggattagtaaaagcaattagggtaaggaaaagg

SEQ ID NO: 519 - DNA, 102 bp, synthetic construct
  misc_feature 1..102: note = Epichloe festucae
  misc_feature 51: note = Variation - S is G strain AR37 or A strain RGT18
  source 1..102: mol_type = other DNA
tttattactaagttaaatactttaattataagtaatttattactaagttasatactaagcacttaatttactctctaaagactagaatatactaaactaata

SEQ ID NO: 520 - DNA, 102 bp, synthetic construct
  misc_feature 1..102: note = Epichloe festucae
  misc_feature 51: note = Variation - S is A strain AR37 or C strain RGT18
  source 1..102: mol_type = other DNA
aaactcacttgaacatgtcggccgagatctgagtgatcctcgcccacgcastcacgccaggccgggcaggcgtcttctgcagcctcgtcttgatggtgtcga

SEQ ID NO: 521 - DNA, 102 bp, synthetic construct
  misc_feature 1..102: note = Epichloe festucae
  misc_feature 51: note = Variation - S is A strain AR37 or G strain RGT18
  source 1..102: mol_type = other DNA
atgtaatcaggccggctgtccacgaactctcccaaggaaagcgccctacasaagtgttccaaatgagacttggcgttgtcaaagtcaagtcttgccccagta

SEQ ID NO: 522 - DNA, 102 bp, synthetic construct
  misc_feature 1..102: note = Epichloe festucae
  misc_feature 51: note = Variation - S is G strain AR37 or A strain RGT18
  source 1..102: mol_type = other DNA
gagtagagagcagacaaacaaggaaaaaaaaaaaaaaaaaaaaaaaaaaasaaaaaaaaaaaaaaaaaaaaaaaaaaacccgtgtagcagttcaagtacaat

SEQ ID NO: 523 - DNA, 102 bp, synthetic construct
  misc_feature 1..102: note = Epichloe festucae
  misc_feature 51: note = Variation - S is G strain AR37 or A strain RGT18
  source 1..102: mol_type = other DNA
atatatatcttaactattagttttagtatttctaagtttaatagttaatasaagccctatatataattagtataggataattaaatataatatatatatcta

SEQ ID NO: 524 - DNA, 102 bp, synthetic construct
  misc_feature 1..102: note = Epichloe festucae
  misc_feature 51: note = Variation - S is G strain AR37 or C strain RGT18
  source 1..102: mol_type = other DNA
ccccaaaaagaaaagaaaagaaaaaaaagaacgcctcgcttactctgcctsccccacgctccaccacaatcacgcagcagatattactctgcctcccccacg

SEQ ID NO: 525 - DNA, 102 bp, synthetic construct
  misc_feature 1..102: note = Epichloe festucae
  misc_feature 51: note = Variation - S is A strain AR37 or G strain RGT18
  source 1..102: mol_type = other DNA
tatagggatacctatattatttatagggtaatcctttaaaccttaatttasatcttattattatactaaattattttccccctctaaagggttatcccctat

SEQ ID NO: 526 - DNA, 102 bp, synthetic construct; identical to SEQ ID NO: 390
  misc_feature 1..102: note = Epichloe festucae
  misc_feature 51: note = Variation - S is G strain AR37 or A strain RGT18
  source 1..102: mol_type = other DNA

SEQ ID NO: 527 - DNA, 102 bp, synthetic construct
  misc_feature 1..102: note = Epichloe festucae
  misc_feature 51: note = Variation - S is C strain AR37 or T strain RGT18
  source 1..102: mol_type = other DNA
ggtccgggcgggcaactcgagccgggaaaaagggggggggggggttttttstttttttttttgtaataaagattgcccgagatgaggtttgcctgggggggg

SEQ ID NO: 528 - DNA, 102 bp, synthetic construct
  misc_feature 1..102: note = Epichloe festucae
  misc_feature 51: note = Variation - S is T strain AR37 or C strain RGT18
  source 1..102: mol_type = other DNA
ttcaagctggtacgggggcttggattaaaattgccacatctaccctacctsccctaaattgaagcgacatcgaagcgacattgaagcgcgacatgaacaaaa

SEQ ID NO: 529 - DNA, 102 bp, synthetic construct
  misc_feature 1..102: note = Epichloe festucae
  misc_feature 51: note = Variation - S is G strain AR37 or C strain RGT18
  source 1..102: mol_type = other DNA
agtaatcatggctgcaatgcactgatcttgggtgtacgaattggccgccgstcatgagaggagattgaaatcttgtctattttttgggaattatcaatgctc

SEQ ID NO: 530 - DNA, 102 bp, synthetic construct
  misc_feature 1..102: note = Epichloe festucae
  misc_feature 51: note = Variation - S is T strain AR37 or C strain RGT18
  source 1..102: mol_type = other DNA
tatattaataagattagggaaaaatttaggtaagtaagaaaaggcactttscttactatactaatcctagtagtaaagtattataagtttaagggttactat

SEQ ID NO: 531 - DNA, 102 bp, synthetic construct
  misc_feature 1..102: note = Epichloe festucae
  misc_feature 51: note = Variation - S is A strain AR37 or G strain RGT18
  source 1..102: mol_type = other DNA
taaacttattaagggcctatatttatactatattctctaatagttcctatstaggctatatatagcccgcttacttaataagtatattatatctcttgccct

SEQ ID NO: 532 - DNA, 102 bp, synthetic construct
  misc_feature 1..102: note = Epichloe festucae
  misc_feature 51: note = Variation - S is A strain AR37 or G strain RGT18
  source 1..102: mol_type = other DNA
ccttagatattagctataattttacctatagtctatagtaattatatagtsaggtagtcttattaaaatataaataaaaatgcttatatataaaggggaaac

SEQ ID NO: 533 - DNA, 102 bp, synthetic construct
  misc_feature 1..102: note = Epichloe festucae
  misc_feature 51: note = Variation - S is A strain AR37 or G strain RGT18
  source 1..102: mol_type = other DNA
tattgagatgcatcaaaaatgtgacaacctaaaaaaaaaaaaaaaaaaaasaacgaaaagaactcgcaggatatcgtgtccaaagacgtgcggaattaaagt

SEQ ID NO: 534 - DNA, 102 bp, synthetic construct
  misc_feature 1..102: note = Epichloe festucae
  misc_feature 51: note = Variation - S is A strain AR37 or T strain RGT18
  source 1..102: mol_type = other DNA
tcttttgcgacaacctcaacttacaaccgccacgacgccaatgatcctcastgtcccacgagcaatatcgtcacccacgaaaacaaccagcgaacaatcttc

SEQ ID NO: 535 - DNA, 102 bp, synthetic construct
  misc_feature 1..102: note = Epichloe festucae
  misc_feature 51: note = Variation - S is C strain AR37 or T strain RGT18
  source 1..102: mol_type = other DNA
tgaactggatacagcataggtgtagtagacgtttctttttttttttttttsttttttttttaaaaaagcccattcgactgttgaagcttgtttctgtttcca

SEQ ID NO: 536 - DNA, 102 bp, synthetic construct
  misc_feature 1..102: note = Epichloe festucae
  misc_feature 51: note = Variation - S is C strain AR37 or T strain RGT18
  source 1..102: mol_type = other DNA
ttccggcggatcgggacgacgctcccagggcgtggagcttgagcgacgggsgttgggcgaggaggaggatgaagcgctggccgacggagcctgtggctccaa

SEQ ID NO: 537 - DNA, 102 bp, synthetic construct
  misc_feature 1..102: note = Epichloe festucae
  misc_feature 51: note = Variation - S is C strain AR37 or A strain RGT18
  source 1..102: mol_type = other DNA
tatttgacattgagacttggcatgatggaacttgaggacgactgctctctstagcaattcatcatggcaggtgtttgcgagattccatgtcatggttttcaa

SEQ ID NO: 538 - DNA, 102 bp, synthetic construct
  misc_feature 1..102: note = Epichloe festucae
  misc_feature 51: note = Variation - S is A strain AR37 or C strain RGT18
  source 1..102: mol_type = other DNA
tgtacacagcgaaatcggggaccgaaaaaaaaaaaaaaaaaaaaaaaaaasctaccctccgctcagtgaatacggaactaggatccatctcttgtttttgga

SEQ ID NO: 539 - DNA, 102 bp, synthetic construct
  misc_feature 1..102: note = Epichloe festucae
  misc_feature 51: note = Variation - S is A strain AR37 or G strain RGT18
  source 1..102: mol_type = other DNA
atctaggttagtgaactggaactgcttcttctcgcctgctccagcactagsccgtggaggagctgtcccttctggctggccacccgcgaggctcgcccttct

SEQ ID NO: 540 - DNA, 102 bp, synthetic construct
  misc_feature 1..102: note = Epichloe festucae
  misc_feature 51: note = Variation - S is A strain AR37 or G strain RGT18
  source 1..102: mol_type = other DNA
tagggttagagggctagagctaaaggactattcttactttctaagggttasagggctagagctaaaggactattcttacctcctagataaatatagtattct

SEQ ID NO: 541 - DNA, 102 bp, synthetic construct
  misc_feature 1..102: note = Epichloe festucae
  misc_feature 51: note = Variation - S is A strain AR37 or G strain RGT18
  source 1..102: mol_type = other DNA
ttcgacaagggtcagatacagctgcctcagccaacacgctctgtccagctsatttatcatacatgatgctgtttcatcatgtccacgcagaaacgcctcttg

SEQ ID NO: 542 - DNA, 102 bp, synthetic construct
  misc_feature 1..102: note = Epichloe festucae
  misc_feature 51: note = Variation - S is A strain AR37 or G strain RGT18
  source 1..102: mol_type = other DNA
ggagcgggtaggcagtcttggtaagataatggtggagttgcgccgcacgasccgacaaaccgccaaaagaggaggcaatggtgttgaactctacctgcttga

SEQ ID NO: 543 - DNA, 102 bp, synthetic construct
  misc_feature 1..102: note = Epichloe festucae
  misc_feature 51: note = Variation - S is G strain AR37 or A strain RGT18
  source 1..102: mol_type = other DNA
caaggatgggggactggttgcgtaagcaaaacagagcgaaacggagggggsagaccacaacaagatgcaccagactcatggcatggctcatcgggaagttcc

SEQ ID NO: 544 - DNA, 102 bp, synthetic construct
  misc_feature 1..102: note = Epichloe festucae
  misc_feature 51: note = Variation - S is G strain AR37 or T strain RGT18
  source 1..102: mol_type = other DNA
acagacagttcgatttgcttctgacaaggatgtgtgacgtttactcatttstcagtctgcgctactttatgagcttttgtgtttgtagcagagattgacgat

SEQ ID NO: 545 - DNA, 102 bp, synthetic construct
  misc_feature 1..102: note = Epichloe festucae
  misc_feature 51: note = Variation - S is T strain AR37 or A strain RGT18
  source 1..102: mol_type = other DNA
ataatatataaagaaagaatataataaactaatatttataatctattaatsaataattaatagtattattttaattaccttatatagcttaattaagctata

SEQ ID NO: 546 - DNA, 102 bp, synthetic construct
  misc_feature 1..102: note = Epichloe festucae
  misc_feature 51: note = Variation - S is T strain AR37 or C strain RGT18
  source 1..102: mol_type = other DNA
tactaataatattatagtactagtgccttagattcttaattaattatatcstataagacacacactatagcgcttaaggcttacctagctaccctagattag

SEQ ID NO: 547 - DNA, 102 bp, synthetic construct
  misc_feature 1..102: note = Epichloe festucae
  misc_feature 51: note = Variation - S is A strain AR37 or C strain RGT18
  source 1..102: mol_type = other DNA
gctacagctctagtttgcactctcaacatgaggtgaatagactgtcacccsacagctccgtcaacgagctacacattcacccactctttcggtctgactctc

SEQ ID NO: 548 - DNA, 102 bp, synthetic construct
  misc_feature 1..102: note = Epichloe festucae
  misc_feature 51: note = Variation - S is A strain AR37 or C strain RGT18
  source 1..102: mol_type = other DNA
tacaaagctatggcgcatcccggcgttcaggacggtgaaagctttacgggsaactattcaaactgaagagattttgtcgttcatctacttgcttagggtaga

SEQ ID NO: 549 - DNA, 102 bp, synthetic construct
  misc_feature 1..102: note = Epichloe festucae
  misc_feature 51: note = Variation - S is G strain AR37 or T strain RGT18
  source 1..102: mol_type = other DNA
gacaacaaggcggcaattgggagcagaagcagacgacaacggtgagggggsggtggagagggggagggggaagaagaagcaatcatcaaaggaccctgacga

SEQ ID NO: 550 - DNA, 102 bp, synthetic construct
  misc_feature 1..102: note = Epichloe festucae
  misc_feature 51: note = Variation - S is G strain AR37 or C strain RGT18
  source 1..102: mol_type = other DNA
aatggtcgagccaggccagatcgtaagaccggccagcgcatgcagcacatscagcacaaggaagcaccttcgcggcctggccggaatcactgtccagagtga

SEQ ID NO: 551 - DNA, 102 bp, synthetic construct
  misc_feature 1..102: note = Epichloe festucae
  misc_feature 51: note = Variation - S is G strain AR37 or C strain RGT18
  source 1..102: mol_type = other DNA
atactagcccacagtcataggtagcagtaacgtctgcttacattagaaaasttaattaacttaacagtagtaattataataatagctaaatctatctttata

SEQ ID NO: 552 - DNA, 102 bp, synthetic construct
  misc_feature 1..102: note = Epichloe festucae
  misc_feature 51: note = Variation - S is T strain AR37 or C strain RGT18
  source 1..102: mol_type = other DNA
tagagttattaaagagattataagtaaattattaattagagtttaatatastttaattaaactaagtactattaaaaacttacttaatcttataaagaatcc

SEQ ID NO: 553 - DNA, 102 bp, synthetic construct
  misc_feature 1..102: note = Epichloe festucae
  misc_feature 51: note = Variation - S is A strain AR37 or T strain RGT18
  source 1..102: mol_type = other DNA
ggccatgcggctgggttgggcgtcgtcgaggtctttgacacggggagtgtsgggaagggcgtacgggcaacgggggcatgaccagctttcaaaagacttgtt

SEQ ID NO: 554 - DNA, 102 bp, synthetic construct
  misc_feature 1..102: note = Epichloe festucae
  misc_feature 51: note = Variation - S is C strain AR37 or T strain RGT18
  source 1..102: mol_type = other DNA
aactatcaatattatctgtactattaatattatctgtactgttaatattasctgtactatcaatattagcaatacaatcaatattattaataccattaatat

SEQ ID NO: 555 - DNA, 102 bp, synthetic construct
  misc_feature 1..102: note = Epichloe festucae
  misc_feature 51: note = Variation - S is G strain AR37 or A strain RGT18
  source 1..102: mol_type = other DNA
tcaacaaccccagaccaaacgaaaaatgaacaaaaaaaaaaaaaaaaaaasaacaaaaaaaaaaaaaaaaaaggcctcctcttccttccaagtggatgcccg

SEQ ID NO: 556 - DNA, 102 bp, synthetic construct
  misc_feature 1..102: note = Epichloe festucae
  misc_feature 51: note = Variation - S is A strain AR37 or G strain RGT18
  source 1..102: mol_type = other DNA
ccactacattctccaggcggcgtcctctttcctcccctgcatggccctcgscccgcaagagaacgagcgcgtgctcgacatggccgccgcccccggtggcaa

SEQ ID NO: 557 - DNA, 102 bp, synthetic construct
  misc_feature 1..102: note = Epichloe festucae
  misc_feature 51: note = Variation - S is T strain AR37 or C strain RGT18
  source 1..102: mol_type = other DNA
gagacccgagcttggtcgctcgtactcgtactcggatgctgccattgtcasgcccaggcaccacggcacgtcgccgtcgctgagtcaaagccaagaattacc

SEQ ID NO: 558 - DNA, 102 bp, synthetic construct
  misc_feature 1..102: note = Epichloe festucae
  misc_feature 51: note = Variation - S is T strain AR37 or C strain RGT18
  source 1..102: mol_type = other DNA
aaggctagaataaaactagtataggatagctaagacttaccactacccccstaattaatatagtaatattataagtcctcttctagaatataaataagaagg

SEQ ID NO: 559 - DNA, 102 bp, synthetic construct
  misc_feature 1..102: note = Epichloe festucae
  misc_feature 51: note = Variation - S is T strain AR37 or A strain RGT18
  source 1..102: mol_type = other DNA
gagcgcactaacaaagaaaggggagggggggggcggaaagcaagaaaagasacgtggaggatcgagatctgcccccccagcactggaatgtcaacacgtacc

SEQ ID NO: 560 - DNA, 102 bp, synthetic construct
  misc_feature 1..102: note = Epichloe festucae
  misc_feature 51: note = Variation - S is C strain AR37 or T strain RGT18
  source 1..102: mol_type = other DNA
gcgcttgttgcgtcagcatggtatgtctcatcttgtctttttttttttttstttttttttttttcccctttcaagtcaaaagggcattcattcatcatcgag

SEQ ID NO: 561 - DNA, 102 bp, synthetic construct
  misc_feature 1..102: note = Epichloe festucae
  misc_feature 51: note = Variation - S is A strain AR37 or C strain RGT18
  source 1..102: mol_type = other DNA
atttgctctcatctgccacgcctgcagactggtcaacggccaagctccccscgggacgaagactctcgcagaaatcggcatgtggaggtgcagcgggtgcgg

SEQ ID NO: 562 - DNA, 102 bp, synthetic construct
  misc_feature 1..102: note = Epichloe festucae
  misc_feature 51: note = Variation - S is A strain AR37 or G strain RGT18
  source 1..102: mol_type = other DNA
gccttttgcgggaagtcgttgatttcaagcgtcgcgtggaacgccccggcstcgggacccttgttgtcgatgggctggccggaccggagctggccagccttt

SEQ ID NO: 563 - DNA, 102 bp, synthetic construct
  misc_feature 1..102: note = Epichloe festucae
  misc_feature 51: note = Variation - S is A strain AR37 or C strain RGT18
  source 1..102: mol_type = other DNA
ctaggtccgtcgcttgaggcaagtcccaccaaaccgtccccagcctgctgstctccttgcactgtgcaggcaggacatgcacgatggcgggttgagcctgca

SEQ ID NO: 564 - DNA, 102 bp, synthetic construct
  misc_feature 1..102: note = Epichloe festucae
  misc_feature 51: note = Variation - S is G strain AR37 or A strain RGT18
  source 1..102: mol_type = other DNA
acgtataagatgattgccgtttttttttttcagaacgcactcgggcgccasgagcatgagaaagaaaaggagaagagaaagaagaagagaaaggaagatgcg

SEQ ID NO: 565 - DNA, 102 bp, synthetic construct
  misc_feature 1..102: note = Epichloe festucae
  misc_feature 51: note = Variation - S is G strain AR37 or A strain RGT18
  source 1..102: mol_type = other DNA
caagctttagcaggggcatgcatcagggaccgggggggggggggggggggsggacaaacaatcatgtggtttcgtgaaagctggagaacggaagacgcgggg

SEQ ID NO: 566 - DNA, 102 bp, synthetic construct
  misc_feature 1..102: note = Epichloe festucae
  misc_feature 51: note = Variation - S is C strain AR37 or T strain RGT18
  source 1..102: mol_type = other DNA
gggaatctaaacacagagatatcagtcctgcaaatgttcatctcccccccsccccccttttttttttctttttttagaacggcaagctcccagtttcttcgt

SEQ ID NO: 567 - DNA, 102 bp, synthetic construct
  misc_feature 1..102: note = Epichloe festucae
  misc_feature 51: note = Variation - S is T strain AR37 or A strain RGT18
  source 1..102: mol_type = other DNA
caaaagtggcgttgaaggccgaccagatcgtgaccggcctccgagggaagscagtcagggtcgtgaagccgcggatcgaagtcgtagtccacgcaaacgacg

SEQ ID NO: 568 - DNA, 102 bp, synthetic construct
  misc_feature 1..102: note = Epichloe festucae
  misc_feature 51: note = Variation - S is A strain AR37 or T strain RGT18
  source 1..102: mol_type = other DNA
agtaaattaggtggttctcccccctatattactcttaggtagctagtaggsgaagctttagaattataagaataatagtagctaggtaagaggtataagggc

SEQ ID NO: 569 - DNA, 102 bp, synthetic construct
  misc_feature 1..102: note = Epichloe festucae
  misc_feature 51: note = Variation - S is A strain AR37 or C strain RGT18
  source 1..102: mol_type = other DNA
ggggaagcacaaagtccatgggaaaaaaaaaaaaaaaaaaaaaaaaaaaascgttcgaagagcaaccgtcgctccgtgagcagctggtttgggtattgcgat

SEQ ID NO: 570 - DNA, 102 bp, synthetic construct
  misc_feature 1..102: note = Epichloe festucae
  misc_feature 51: note = Variation - S is G strain AR37 or A strain RGT18
  source 1..102: mol_type = other DNA
attagtagtgctactagctctaaaaagttactaataaagttatagtaaaasttagtaaaccctaggaagctataaacctatagtaaaaattagtaaacctta

SEQ ID NO: 571 - DNA, 102 bp, synthetic construct
  misc_feature 1..102: note = Epichloe festucae
  misc_feature 51: note = Variation - S is G strain AR37 or A strain RGT18
  source 1..102: mol_type = other DNA
cagggcgttcctggcgctcatcttgaaaaccttgccaatctgtgatttcgscccgcaattgatcaatgtcttcgagctcctcctgaatagcgttagcacctt

SEQ ID NO: 572 - DNA, 102 bp, synthetic construct
  misc_feature 1..102: note = Epichloe festucae
  misc_feature 51: note = Variation - S is A strain AR37 or G strain RGT18
  source 1..102: mol_type = other DNA
aaatgatccgtacccatatgtaattgtaatgcagcatcccacgcctttgcsctaaatttatatggggcgccatggcaaaaaaaagatatcacctaatattat

SEQ ID NO: 573 - DNA, 102 bp, synthetic construct
  misc_feature 1..102: note = Epichloe festucae
  misc_feature 51: note = Variation - S is T strain AR37 or G strain RGT18
  source 1..102: mol_type = other DNA
acacgcaccaaatgagaaggagatccccgatcgatacccagcaccagcacsgtggaccggaaatgtatgtagagaggactcactgctcactgtcagaggaga

SEQ ID NO: 574 - DNA, 102 bp, synthetic construct
  misc_feature 1..102: note = Epichloe festucae
  misc_feature 51: note = Variation - S is A strain AR37 or G strain RGT18
  source 1..102: mol_type = other DNA
acgcctacaacattttcttggtgggcggccttggaggatatcgacggaccscctatgcctctcgatcggtacttggtgaagatcaataggcggacaaggaca

SEQ ID NO: 575 - DNA, 102 bp, synthetic construct
  misc_feature 1..102: note = Epichloe festucae
  misc_feature 51: note = Variation - S is A strain AR37 or G strain RGT18
  source 1..102: mol_type = other DNA
tgctctcggggatttcgggggcccgctgcctgcctggatgcaacattgagsctgaccgatgccttcttcggcctcggtccttttccttttccccaaccaccg

SEQ ID NO: 576 - DNA, 102 bp, synthetic construct
  misc_feature 1..102: note = Epichloe festucae
  misc_feature 51: note = Variation - S is G strain AR37 or A strain RGT18
  source 1..102: mol_type = other DNA
gcgaaggtcgcaaaaggatgaatcgtgtttgacacgggcagcatctcaacstcaaggatggacacgagcccggggtccttgactgtgcgtgtgcccgaggag

SEQ ID NO: 577 - DNA, 102 bp, synthetic construct
  misc_feature 1..102: note = Epichloe festucae
  misc_feature 51: note = Variation - S is C strain AR37 or T strain RGT18
  source 1..102: mol_type = other DNA
ccttcggttagtgtgcgtcggtcgagggagtcccggtggcgcaacgtctcsatttggccacagattggcagattggggcgagaacgggggcctggaaaagct

SEQ ID NO: 578 - DNA, 102 bp, synthetic construct
  misc_feature 1..102: note = Epichloe festucae
  misc_feature 51: note = Variation - S is T strain AR37 or C strain RGT18
  source 1..102: mol_type = other DNA
cacgtgcgtctgcgttgacgatttatacctctcaacaacataaacgttacscgcagcaatctgcctaggtatgtttcacgacaccgatgcccttcatcctac

SEQ ID NO: 579 - DNA, 102 bp, synthetic construct
  misc_feature 1..102: note = Epichloe festucae
  misc_feature 51: note = Variation - S is A strain AR37 or G strain RGT18
  source 1..102: mol_type = other DNA
cagaagacatcatcttattttccgccttcaacgacttgtggaaaaagaacsacatgtcaacgttcgatgctgaccagttttggggcattaacggtgcggttt

SEQ ID NO: 580 - DNA, 102 bp, synthetic construct
  misc_feature 1..102: note = Epichloe festucae
  misc_feature 51: note = Variation - S is C strain AR37 or T strain RGT18
  source 1..102: mol_type = other DNA
gcatctgacatgttatcaaatcgtgtccacggatggcagccgggtatctcsttttttttttttttttttttttcaaaagtcccaaaagctcttttgagcagc

SEQ ID NO: 581 - DNA, 102 bp, synthetic construct
  misc_feature 1..102: note = Epichloe festucae
  misc_feature 51: note = Variation - S is A strain AR37 or T strain RGT18
  source 1..102: mol_type = other DNA
aaaaggccgcctgcctgtttcctgctgcactcctctctcaggctctctggsagaacatgtggacccgccatcaccggccagttttggcggccacgaccacat

SEQ ID NO: 582 - DNA, 102 bp, synthetic construct
  misc_feature 1..102: note = Epichloe festucae
  misc_feature 51: note = Variation - S is C strain AR37 or T strain RGT18
  source 1..102: mol_type = other DNA
atcttcatcatcgaggggatcccgagcgtggtgctgggcgtggtgacgtastttgcgctgcccaacgatgccgggacggcgtactttctggacgacgcggag

SEQ ID NO: 583 - DNA, 102 bp, synthetic construct
  misc_feature 1..102: note = Epichloe festucae
  misc_feature 51: note = Variation - S is G strain AR37 or A strain RGT18
  source 1..102: mol_type = other DNA
taaataggtaaaggctatgctagttaggaatgtaataatactagtaattasgaagttccttttctccttaattagtagatttaggcttttctgctttatagt

SEQ ID NO: 584 - DNA, 102 bp, synthetic construct
  misc_feature 1..102: note = Epichloe festucae
  misc_feature 51: note = Variation - S is A strain AR37 or T strain RGT18
  source 1..102: mol_type = other DNA
tcacggaaatgagacatgaacccgcggcccaatagttggggcgttgcacasgcccttgtgcgagcgagggcttaattccccgaagctggaccacgtgccttg

SEQ ID NO: 585 - DNA, 102 bp, synthetic construct
  misc_feature 1..102: note = Epichloe festucae
  misc_feature 51: note = Variation - S is T strain AR37 or C strain RGT18
  source 1..102: mol_type = other DNA
tttaataaaattatttaacctttattaaataataaaattatattatactcsatcttaatacttttaattaaatagttaattaaattaactttatataaaact

SEQ ID NO: 586 - DNA, 102 bp, synthetic construct
  misc_feature 1..102: note = Epichloe festucae
  misc_feature 51: note = Variation - S is T strain AR37 or C strain RGT18
  source 1..102: mol_type = other DNA
ggcaatctttgcattgccttgtgtttttttttttttttttttttttttttsggtcagcaaaggttgagaacatgggcagtcactggaaagggcgcggggcag

SEQ ID NO: 587 - DNA, 102 bp, synthetic construct
  misc_feature 1..102: note = Epichloe festucae
  misc_feature 51: note = Variation - S is A strain AR37 or G strain RGT18
  source 1..102: mol_type = other DNA
tcttctcccatcgcgcctcgccttcagcaaccttgttgagatatgacgtcscaatgccccggctctgccgcacctcacagcaagacagtcgagccgcgcatc

SEQ ID NO: 588 - DNA, 102 bp, synthetic construct
  misc_feature 1..102: note = Epichloe festucae
  misc_feature 51: note = Variation - S is A strain AR37 or T strain RGT18
  source 1..102: mol_type = other DNA
tgctggcatgccgtcgatacatcgttaacgagggcaaaaaaaaaaaaaaastttttccatctcacactcggtgaaatgtaaatatgtcccctcacttgtaat

SEQ ID NO: 589 - DNA, 102 bp, synthetic construct
  misc_feature 1..102: note = Epichloe festucae
  misc_feature 51: note = Variation - S is G strain AR37 or C strain RGT18
  source 1..102: mol_type = other DNA
accgagcccgctcttcccgaagaagccctcaagctgatcgactgcggtgasgcggacaaattcggcctggccaagcagttccagaatgtcgtttctacacag

SEQ ID NO: 590 - DNA, 102 bp, synthetic construct
  misc_feature 1..102: note = Epichloe festucae
  misc_feature 51: note = Variation - S is T strain AR37 or G strain RGT18
  source 1..102: mol_type = other DNA
catcagtattttcatgactgtcagagggccaccgggggggggggggggggsgtctttacttacatccagttggaaatgcaaaaggcaataaaaatgccaagg

SEQ ID NO: 591 - DNA, 102 bp, synthetic construct
  misc_feature 1..102: note = Epichloe festucae
  misc_feature 51: note = Variation - S is C strain AR37 or T strain RGT18
  source 1..102: mol_type = other DNA
tttacgaatatcggggtcggcatcggcaaattgtcccacagaaagacaaasggtcgtgagtgggccggccgtggcaaaggtcaactgaaagttgagcttcag

SEQ ID NO: 592 - DNA, 102 bp, synthetic construct
  misc_feature 1..102: note = Epichloe festucae
  misc_feature 51: note = Variation - S is G strain AR37 or A strain RGT18
  source 1..102: mol_type = other DNA
tgtctcatcagcaaaaaaagaaaaagaaaaaaaaaaaaaaaaaaaaaaaasaaaaaaaaaaaaaaaaaaaaaaaggaaaagggcctcgtttcgtaattctag

SEQ ID NO: 593 - DNA, 102 bp, synthetic construct
  misc_feature 1..102: note = Epichloe festucae
  misc_feature 51: note = Variation - S is A strain AR37 or G strain RGT18
  source 1..102: mol_type = other DNA
agcgtccctgaaatatcaaggggactgacagtgaaatcaagacgacaagasaaaaaaaaaaaaaaaaaaaagaaaagaccaagggaaaatgaaccaaatcaa

SEQ ID NO: 594 - DNA, 102 bp, synthetic construct
  misc_feature 1..102: note = Epichloe festucae
  misc_feature 51: note = Variation - S is C strain AR37 or T strain RGT18
  source 1..102: mol_type = other DNA
tgtactccgtacacacggattaaagagcaccagatctgtggctggtggtcsgccacatccggcattgggacttgtaggcttattagcgctcgcatcccatct

SEQ ID NO: 595 - DNA, 102 bp, synthetic construct
  misc_feature 1..102: note = Epichloe festucae
  misc_feature 51: note = Variation - S is G strain AR37 or T strain RGT18
  source 1..102: mol_type = other DNA
cgaagaattggggcatgtagatttataaaataattcggggggggggggggsgggttgtacaaagtgtctctccatcgtgatatcaatatcccaacgcccaaa

SEQ ID NO: 596 - DNA, 102 bp, synthetic construct
  misc_feature 1..102: note = Epichloe festucae
  misc_feature 51: note = Variation - S is T strain AR37 or C strain RGT18
  source 1..102: mol_type = other DNA
tttgagaagaagatgacgctgaacacaccctggctggacggatcggcgtasctgaagaggccgggacggggcggtcggctggcggccaaggcggtgccggtg

SEQ ID NO: 597 - DNA, 102 bp, synthetic construct
  misc_feature 1..102: note = Epichloe festucae
  misc_feature 51: note = Variation - S is A strain AR37 or T strain RGT18
  source 1..102: mol_type = other DNA
gagggtgctgttgtacaacgtcggccaagtagagagagatgtgggatgtasaaattactttcgtctggcagaggctggacgacggatgcgtcggtacaacat

SEQ ID NO: 598 - DNA, 102 bp, synthetic construct
  misc_feature 1..102: note = Epichloe festucae
  misc_feature 51: note = Variation - S is C strain AR37 or A strain RGT18
  source 1..102: mol_type = other DNA
cctcgctgttcaaagggcacttgttcgcacagttgaacgttcaatgccccsccaggagctacgacccaaacatcacagctcagaaggacgaagtgttgtttg

SEQ ID NO: 599 - DNA, 102 bp, synthetic construct
  misc_feature 1..102: note = Epichloe festucae
  misc_feature 51: note = Variation - S is T strain AR37 or C strain RGT18
  source 1..102: mol_type = other DNA
ctgcgatgagttttgcgctaggggcataatgaaagactgagggagcgtacsgtgtggccgagcgacaggaggagccatcccaccgcggtgactctgagggat

SEQ ID NO: 600 - DNA, 102 bp, synthetic construct
  misc_feature 1..102: note = Epichloe festucae
  misc_feature 51: note = Variation - S is G strain AR37 or C strain RGT18
  source 1..102: mol_type = other DNA
gccaggtataatatattagccagcatctcttgtgtagaaagaaccaacccsaaaaaaaaaaaaaaaaaaaaaaaaacactccgaaaatcaatcatgatgatt

SEQ ID NO: 601 - DNA, 102 bp, synthetic construct
  misc_feature 1..102: note = Epichloe festucae
  misc_feature 51: note = Variation - S is G strain AR37 or C strain RGT18
  source 1..102: mol_type = other DNA
gccagcaccgttgggtccaatcacagcaatacgagatcccaaagagcactsgaaagtgatgtcggaaacctggggcttggaggtaccgggatactggaagga

SEQ ID NO: 602 - DNA, 102 bp, synthetic construct
  misc_feature 1..102: note = Epichloe festucae
  misc_feature 51: note = Variation - S is C strain AR37 or A strain RGT18
  source 1..102: mol_type = other DNA
tcgccgcagttgaagaaggcgaacaacaggccgtcatcgtcatcctccccstcggcgttgccacgcgcccgcgcccgcgtccgcgcccgctcgtacgcctcg

SEQ ID NO: 603 - DNA, 102 bp, synthetic construct
  misc_feature 1..102: note = Epichloe festucae
  misc_feature 51: note = Variation - S is G strain AR37 or T strain RGT18
  source 1..102: mol_type = other DNA
ggcaaccatgacaccataaacgcggtatttttttttttttttttttttttstttttttttttttttttttttttttgcttttttgaatcccccaacatgccg

SEQ ID NO: 604 - DNA, 102 bp, synthetic construct
  misc_feature 1..102: note = Epichloe festucae
  misc_feature 51: note = Variation - S is G strain AR37 or A strain RGT18
  source 1..102: mol_type = other DNA
attcttcttgagcaagcgtttgatgggctgggtgctcggtctcctttcaasgcgcgaatgcctcacagtcgtgcattttagattcaggatttcttgggtcga

SEQ ID NO: 605 - DNA, 102 bp, synthetic construct
  misc_feature 1..102: note = Epichloe festucae
  misc_feature 51: note = Variation - S is G strain AR37 or T strain RGT18
  source 1..102: mol_type = other DNA
tttcggctgagacattgggaaaaaaggaaaaaaggaaaaaaaaaaaaaagstatggctttggttctggttcctgacgaaagctgccacccccggcacggttc

SEQ ID NO: 606 - DNA, 102 bp, synthetic construct
  misc_feature 1..102: note = Epichloe festucae
  misc_feature 51: note = Variation - S is A strain AR37 or C strain RGT18
  source 1..102: mol_type = other DNA
aaagagacgttgatgtggataacccacggatacggattcgcacttcccgtsatggttcgtgaagttttcgtcgcggatgaagggtgctttgcagttgaatgg

SEQ ID NO: 607 - DNA, 102 bp, synthetic construct
  misc_feature 1..102: note = Epichloe festucae
  misc_feature 51: note = Variation - S is C strain AR37 or T strain RGT18
  source 1..102: mol_type = other DNA
tctcgcagtggagatcgcccgcgcaagtatgtgcgcgtctgaaatatgtasaggatgctgaggcttgtttcctgggcgaagaagacgaagagctggacacga

SEQ ID NO: 608 - DNA, 102 bp, synthetic construct
  misc_feature 1..102: note = Epichloe festucae
  misc_feature 51: note = Variation - S is A strain AR37 or G strain RGT18
  source 1..102: mol_type = other DNA
ttcaggtggacacgcagcgcaatattgtctttgcaaggctgggggctaagsactgtgagtcgtcgcgcccgacgtacgcaatgcccaacacatggacgcaca

SEQ ID NO: 609 - DNA, 102 bp, synthetic construct
  misc_feature 1..102: note = Epichloe festucae
  misc_feature 51: note = Variation - S is C strain AR37 or T strain RGT18
  source 1..102: mol_type = other DNA
agcagcggcaggctcagctgcgagagggtgaaggcgcggtgcaggttcagsgtgaggagcttcgtccacgccgcgtcggggtgctcgtcgaagggggcgccc

SEQ ID NO: 610 - DNA, 102 bp, synthetic construct
  misc_feature 1..102: note = Epichloe festucae
  misc_feature 51: note = Variation - S is T strain AR37 or G strain RGT18
  source 1..102: mol_type = other DNA
ctgccaaacgacacggttgtctgtgtaggttctgctttttttttttggggsttttttttccctacgaatgagcaaggattcgggaagcatgcctggtgctaa

SEQ ID NO: 611 - DNA, 102 bp, synthetic construct
  misc_feature 1..102: note = Epichloe festucae
  misc_feature 51: note = Variation - S is A strain AR37 or G strain RGT18
  source 1..102: mol_type = other DNA
tcgtgggtgccgaatgaaaaaaaaaaaatagaaatttgaaagcgttaaatsgtgccagctcaattgagaggtaccgccgaccagctcccatgtgccatgagg

SEQ ID NO: 612 - DNA, 102 bp, synthetic construct
  misc_feature 1..102: note = Epichloe festucae
  misc_feature 51: note = Variation - S is T strain AR37 or G strain RGT18
  source 1..102: mol_type = other DNA
cgacggattggatgcatatttgtgtgcttggggaggggcgggggggggggstgaatgcgcccccgggaagcattaatatcaggtttctagacaatttttgtt

SEQ ID NO: 613 - DNA, 102 bp, synthetic construct
  misc_feature 1..102: note = Epichloe festucae
  misc_feature 51: note = Variation - S is G strain AR37 or A strain RGT18
  source 1..102: mol_type = other DNA
cctgcatctgtcccgggcagtccgtgagggctacgaaaaaaaaaaaaaaasaaaaaaaaaagtcgccaccaccaccaccaccactcaacatatcgttttatt

SEQ ID NO: 614 - DNA, 102 bp, synthetic construct
  misc_feature 1..102: note = Epichloe festucae
  misc_feature 51: note = Variation - S is C strain AR37 or T strain RGT18
  source 1..102: mol_type = other DNA
ctctcgcccgttagcccggccgccagtgccatttttgccgtttgctgcaasagctgcgagaagaacatccccgatgctcattatcactgctctacctgcgac

SEQ ID NO: 615 - DNA, 102 bp, synthetic construct
  misc_feature 1..102: note = Epichloe festucae
  misc_feature 51: note = Variation - S is T strain AR37 or A strain RGT18
  source 1..102: mol_type = other DNA
tcctatattcgtcgctggttcgacgaccgtgacttcgtctcagtgcaaacscctatgcttaatccaattgctggtggtgccactgccaagcccttcgttact

SEQ ID NO: 616 - DNA, 102 bp, synthetic construct
  misc_feature 1..102: note = Epichloe festucae
  misc_feature 51: note = Variation - S is A strain AR37 or G strain RGT18
  source 1..102: mol_type = other DNA
gcgttggcagtcggtcccctcatgcatctgaacggggaacagcacgatccsggaccagcgagcccaactgcgccaacggccggacgccaatgaagtcatcct

SEQ ID NO: 617 - DNA, 102 bp, synthetic construct
  misc_feature 1..102: note = Epichloe festucae
  misc_feature 51: note = Variation - S is T strain AR37 or C strain RGT18
  source 1..102: mol_type = other DNA
ccgaactatgttatgaaaaagaagaggccgagaactcgagaacttcttcasagctaccaagagattgtttgggctacatgtgtttttttcccttccgacctt

SEQ ID NO: 618 - DNA, 102 bp, synthetic construct
  misc_feature 1..102: note = Epichloe festucae
  misc_feature 51: note = Variation - S is C strain AR37 or T strain RGT18
  source 1..102: mol_type = other DNA
cgtttccagtttccctactctgtattatttatctgctgcgtcgactctttsccccccccctatccatgttctttcatggaaccaaggagctcttttcctttt

SEQ ID NO: 619 - DNA, 102 bp, synthetic construct
  misc_feature 1..102: note = Epichloe festucae
  misc_feature 51: note = Variation - S is A strain AR37 or G strain RGT18
  source 1..102: mol_type = other DNA
cgtccaattaggatagccttgggctcatccaggctactggaaggagcaccsccgtctttgctctgattttccatgatggatgcaatcgtagcactcaagtcg

SEQ ID NO: 620 - DNA, 102 bp, synthetic construct
  misc_feature 1..102: note = Epichloe festucae
  misc_feature 51: note = Variation - S is T strain AR37 or G strain RGT18
  source 1..102: mol_type = other DNA
attctaaataattagctaaaagagcaggttattaagtaacaagatgctatsaatctattattacttataaaagctagaggctctaactacagctattaataa

SEQ ID NO: 621 - DNA, 102 bp, synthetic construct
  misc_feature 1..102: note = Epichloe festucae
  misc_feature 51: note = Variation - S is G strain AR37 or C strain RGT18
  source 1..102: mol_type = other DNA
ctgttgggagacggtcatgctgcctggggaagaggtggcgcgacgcgggasttgggcggcgttgaggtcgacttggttctttggtgcgacttgttggaccgg

SEQ ID NO: 622 - DNA, 102 bp, synthetic construct
  misc_feature 1..102: note = Epichloe festucae
  misc_feature 51: note = Variation - S is G strain AR37 or A strain RGT18
  source 1..102: mol_type = other DNA
agggagaaatcgtgtccctccgctgtttgtcggagaggaattgaaatgcascctccattagttctgcgacgaaagcctcgtcatctcggagaagttgtcgaa

SEQ ID NO: 623 - DNA, 102 bp, synthetic construct
  misc_feature 1..102: note = Epichloe festucae
  misc_feature 51: note = Variation - S is T strain AR37 or C strain RGT18
  source 1..102: mol_type = other DNA
ggacgactcgacttcctctagtgtgtattcgcactacgtgtcctccgtctsacaatcggcggggctcgacacgaatcgcgtgcacgtactccgcatgcagcg

SEQ ID NO: 624 - DNA, 102 bp, synthetic construct
  misc_feature 1..102: note = Epichloe festucae
  misc_feature 51: note = Variation - S is C strain AR37 or T strain RGT18
  source 1..102: mol_type = other DNA
tatagttataataattcccttacttccttattatatatatattatatatastatattataagtgtatttatactaatatattatagggactagtatatatag

SEQ ID NO: 625 - DNA, 102 bp, synthetic construct
  misc_feature 1..102: note = Epichloe festucae
  misc_feature 51: note = Variation - S is C strain AR37 or T strain RGT18
  source 1..102: mol_type = other DNA
gactgaccgacttgtcttgagaatgcggcaccatcccatcaatgccccccsccccccccccctcttgagaatgcggcaccatcccatcaatgcccccctccc

SEQ ID NO: 626 - DNA, 102 bp, synthetic construct
  misc_feature 1..102: note = Epichloe festucae
  misc_feature 51: note = Variation - S is G strain AR37 or C strain RGT18
  source 1..102: mol_type = other DNA
gccctccctcacgggaccggcctggcacaatttgggggggggggggggggsgcttgttcgttgactcttcagatgttttcgatgtctttttaactctcgcgc

SEQ ID NO: 627 - DNA, 102 bp, synthetic construct
  misc_feature 1..102: note = Epichloe festucae
  misc_feature 51: note = Variation - S is A strain AR37 or G strain RGT18
  source 1..102: mol_type = other DNA
aagactatcgcagtcgctactagatagatactagctaggggcaggtgcgtsaaggttttaatctctaaccttacactaataatatgcgtagtctttaataaa

SEQ ID NO: 628 - DNA, 102 bp, synthetic construct
  misc_feature 1..102: note = Epichloe festucae
  misc_feature 51: note = Variation - S is T strain AR37 or A strain RGT18
  source 1..102: mol_type = other DNA
ctggggggatgatgagagggacatactcgtcttggtgtcaccagattgcasgatacaacttgtgcacaggctcgcgacgcgagccacgtcgaagctccgatt

SEQ ID NO: 629 - DNA, 102 bp, synthetic construct
  misc_feature 1..102: note = Epichloe festucae
  misc_feature 51: note = Variation - S is A strain AR37 or G strain RGT18
  source 1..102: mol_type = other DNA
gctccagcagcaggcgcctatgcaatttgacaaaaaaaaaaaaaaaaaaasagtccagcgttagtataatcattgatcattcagtttgttccgtatccttgg

SEQ ID NO: 630 - DNA, 102 bp, synthetic construct
  misc_feature 1..102: note = Epichloe festucae
  misc_feature 51: note = Variation - S is T strain AR37 or C strain RGT18
  source 1..102: mol_type = other DNA
acttgcaacagcacttcctttcgctgtttgcataccagtcctttcccttcscgcttctttgaaagaccgcgtgaacaactctccttgacggccgtgccgatt

SEQ ID NO: 631 - DNA, 102 bp, synthetic construct
  misc_feature 1..102: note = Epichloe festucae
  misc_feature 51: note = Variation - S is C strain AR37 or T strain RGT18
  source 1..102: mol_type = other DNA
actcgttatccaagtcgatgggtttgcgtcctttttttttttttttttttstttttttcccctcttctaatatatttcttttttttttttttttttttcttt

SEQ ID NO: 632 - DNA, 102 bp, synthetic construct
  misc_feature 1..102: note = Epichloe festucae
  misc_feature 51: note = Variation - S is T strain AR37 or G strain RGT18
  source 1..102: mol_type = other DNA
ctatcagagacccataaaagacccacttttttatatttactctataaaatsaaaatagtatacctatagctttaaaattatataaatctagctaatttatag

SEQ ID NO: 633 - DNA, 102 bp, synthetic construct
  misc_feature 1..102: note = Epichloe festucae
  misc_feature 51: note = Variation - S is A strain AR37 or C strain RGT18
  source 1..102: mol_type = other DNA
ccgcatcgctggcctggacgctgtaagaggtcgtgtgaaaagggggtctcstgtattgttgttgttccatgccgcagaagttggagatgcacacaatttgcc

SEQ ID NO: 634 - DNA, 102 bp, synthetic construct
  misc_feature 1..102: note = Epichloe festucae
  misc_feature 51: note = Variation - S is A strain AR37 or C strain RGT18
  source 1..102: mol_type = other DNA
aaagaagaagaagaagaagaagcaaaaaaaaaaaaccaaaaaaaaaaaaasaagttctgtacaggtgcagtaagaagagagggtaagctgcatatgtgtcta

SEQ ID NO: 635 - DNA, 102 bp, synthetic construct
  misc_feature 1..102: note = Epichloe festucae
  misc_feature 51: note = Variation - S is G strain AR37 or A strain RGT18
  source 1..102: mol_type = other DNA
ggactgcctgcgagccgaagagttgttgcgcgctgcgaacagggcccagtstaggtcgaatcgaggcgggatcggtggtcttggagggagacgctgatgccg

SEQ ID NO: 636 - DNA, 102 bp, synthetic construct
  misc_feature 1..102: note = Epichloe festucae
  misc_feature 51: note = Variation - S is C strain AR37 or T strain RGT18
  source 1..102: mol_type = other DNA
gaaatgtgtctgacgacgcaacatgtgcgtcatcgtcaaaaaccagatttsaggatagctagtagagtcgaattctaagcaacattgcaaagaagttctagt

SEQ ID NO: 637 - DNA, 102 bp, synthetic construct
  misc_feature 1..102: note = Epichloe festucae
  misc_feature 51: note = Variation - S is A strain AR37 or G strain RGT18
  source 1..102: mol_type = other DNA
attgctgctgaactccgtccattgatcgtggtggaattagagtgctcccascgttgcgagaaacggccagtcgagcctctcgagggcgatgatgccggtgtg

SEQ ID NO: 638 - DNA, 102 bp, synthetic construct
  misc_feature 1..102: note = Epichloe festucae
  misc_feature 51: note = Variation - S is A strain AR37 or G strain RGT18
  source 1..102: mol_type = other DNA
ctactaatccgtacggagcatagtaatgactcctgcaggagctgaggcagstgcggctataggcatattactggatggattggacttgccataatatgtcaa

SEQ ID NO: 639 - DNA, 102 bp, synthetic construct
  misc_feature 1..102: note = Epichloe festucae
  misc_feature 51: note = Variation - S is T strain AR37 or C strain RGT18
  source 1..102: mol_type = other DNA
cttgcttatctgctgccttcttggctgcctttgcggctttgctcccacctscatcgtcgtcgtcttcttcgccgtctacctccacgacatcatcgtcaatgt

SEQ ID NO: 640 - DNA, 102 bp, synthetic construct
  misc_feature 1..102: note = Epichloe festucae
  misc_feature 51: note = Variation - S is T strain AR37 or A strain RGT18
  source 1..102: mol_type = other DNA
aatatataaaaatacacatgtcccccggctcaactcgtcgacttctctcastcaatcgaccaaaccaaccaaccaaccaaccaaccaaccgtaacacacagc

SEQ ID NO: 641 - DNA, 102 bp, synthetic construct
  misc_feature 1..102: note = Epichloe festucae
  misc_feature 51: note = Variation - S is A strain AR37 or G strain RGT18
  source 1..102: mol_type = other DNA
gacgagctttttgacgccgtgtccaccacgagcccatctacgttctgtaasgcattcttcctgcttgcggccctgggtgttctgtcgctgaatgtcctccct

SEQ ID NO: 642 - DNA, 102 bp, synthetic construct
  misc_feature 1..102: note = Epichloe festucae
  misc_feature 51: note = Variation - S is T strain AR37 or A strain RGT18
  source 1..102: mol_type = other DNA
gctctgcttcgtccttctcccactcgtcgttgactggaagctgaggtcttscgcgctctttccccttgccgctgcgctgctgacccccgactcctctctctt

SEQ ID NO: 643 - DNA, 102 bp, synthetic construct
  misc_feature 1..102: note = Epichloe festucae
  misc_feature 51: note = Variation - S is T strain AR37 or A strain RGT18
  source 1..102: mol_type = other DNA
agatgatctcagaagtggtgtccctataggaacggaagggtttgtgatcgscagcgtagtagagggtgtcgctccttttgggtgtgtaccttggaggaggag

SEQ ID NO: 644 - DNA, 102 bp, synthetic construct
  misc_feature 1..102: note = Epichloe festucae
  misc_feature 51: note = Variation - S is G strain AR37 or A strain RGT18
  source 1..102: mol_type = other DNA
ttgttgagggtggctttgtcgccggcggcaaaggcctcgagcatctcgcgstacatggcttttgcggtgggcgcaatcttggccctgcgggccttccatttc

SEQ ID NO: 645 - DNA, 102 bp, synthetic construct
  misc_feature 1..102: note = Epichloe festucae
  misc_feature 51: note = Variation - S is A strain AR37 or C strain RGT18
  source 1..102: mol_type = other DNA
tgtgtactcgccatttggagaaccaacaaaaaaaaaaaaaaaaaaaaaaastatgtatagacacaacagcgcctcgacggagaatacatctactgaaccgtc

SEQ ID NO: 646 - DNA, 102 bp, synthetic construct
  misc_feature 1..102: note = Epichloe festucae
  misc_feature 51: note = Variation - S is A strain AR37 or C strain RGT18
  source 1..102: mol_type = other DNA
gatgccaaggccacacgagagcgtccaccgcccaaaaaaaaaaaaaaaaasgtcatgaggcgaagcatcccgccgagtaagataatcgggcatggaatggga

SEQ ID NO: 647 - DNA, 102 bp, synthetic construct
  misc_feature 1..102: note = Epichloe festucae
  misc_feature 51: note = Variation - S is A strain AR37 or C strain RGT18
  source 1..102: mol_type = other DNA
ttcgtgaacgtggtgttggtactccaaaaaaaaaaaaaaaaaaaaaaaaasactatgatgctaattgaaacatgaagaagttgtagcgaccaaatgtcgccc

SEQ ID NO: 648 - DNA, 102 bp, synthetic construct
  misc_feature 1..102: note = Epichloe festucae
  misc_feature 51: note = Variation - S is C strain AR37 or A strain RGT18
  source 1..102: mol_type = other DNA
cgctccgtaaacggagaagcgacggctaccccttcacactccgtcggtatsgtgagctccataatattaatcatcaagtttttgaccgacttctaataagtc

SEQ ID NO: 649 - DNA, 102 bp, synthetic construct
  misc_feature 1..102: note = Epichloe festucae
  misc_feature 51: note = Variation - S is T strain AR37 or A strain RGT18
  source 1..102: mol_type = other DNA
gagtaaacgcaagcacgaggatgacgattttgagggcactcccgtttgggsgctctatgtagcctcaatggcactcgttctacttggtggtgcttttgctgg

SEQ ID NO: 650 - DNA, 102 bp, synthetic construct
  misc_feature 1..102: note = Epichloe festucae
  misc_feature 51: note = Variation - S is C strain AR37 or T strain RGT18
  source 1..102: mol_type = other DNA
gggttgcagacccccgttgttggatcatttgttcttttttctttttttttsttttttttttttttttgccgtttttttttttctttttttttttttttgccg

SEQ ID NO: 651 - DNA, 102 bp, synthetic construct
  misc_feature 1..102: note = Epichloe festucae
  misc_feature 51: note = Variation - S is A strain AR37 or G strain RGT18
  source 1..102: mol_type = other DNA
gtcgaggtggcggtcgatggcgtcgagtgcacagagattgtcctgtccaascctcacaagtactactctctgattttggtaagtttctcaacggtccccaac

SEQ ID NO: 652 - DNA, 102 bp, synthetic construct
  misc_feature 1..102: note = Epichloe festucae
  misc_feature 51: note = Variation - S is A strain AR37 or G strain RGT18
  source 1..102: mol_type = other DNA
tgtctgtcccgaccgtcctgtacggagtaaactacggtccgtatcaagtcscctcctctagtccgtaggctctggggctctcatctacagcgctctcggaga

SEQ ID NO: 653 - DNA, 102 bp, synthetic construct
  misc_feature 1..102: note = Epichloe festucae
  misc_feature 51: note = Variation - S is T strain AR37 or C strain RGT18
  source 1..102: mol_type = other DNA
tagaccgtcctttgcatccagcagcagcaggacgaagggtggcggcaaagstcatggtaagatgaccatcaacaagggcaagggcaagggcaagggcaaggg

SEQ ID NO: 654 - DNA, 102 bp, synthetic construct
  misc_feature 1..102: note = Epichloe festucae
  misc_feature 51: note = Variation - S is T strain AR37 or A strain RGT18
  source 1..102: mol_type = other DNA
tcttgagaaaaggacggtctggtctcctttttggggcgtatcaggtctcgstcgatcctgtcgcggtcgtcgcgaggttcgcgccgaatgtctgcttctggt

SEQ ID NO: 655 - DNA, 102 bp, synthetic construct
  misc_feature 1..102: note = Epichloe festucae
  misc_feature 51: note = Variation - S is G strain AR37 or A strain RGT18
  source 1..102: mol_type = other DNA
cgttgcgaagctcttggagacgagtttagacaggactgtgcggcatgagtscttgcaagaacttgcattcagctatcgacgccacaggctgaagctgaacca

SEQ ID NO: 656 - DNA, 102 bp, synthetic construct
  misc_feature 1..102: note = Epichloe festucae
  misc_feature 51: note = Variation - S is A strain AR37 or G strain RGT18
  source 1..102: mol_type = other DNA
gaactggttgcctggtttcatgatgtgccagccaatgagtgggtatggagsaacattggctaatatacgcttgcaggttaaatacaaaattagtatcaaggg

SEQ ID NO: 657 - DNA, 102 bp, synthetic construct
  misc_feature 1..102: note = Epichloe festucae
  misc_feature 51: note = Variation - S is C strain AR37 or A strain RGT18
  source 1..102: mol_type = other DNA
tcaaggttgggtcatgtcgatgcgacgagcgaaacatgaaaaattgatacsccccccccaaaaccgactggtgcccgccaagtcgatgtggaatacgcttgt

SEQ ID NO: 658 - DNA, 102 bp, synthetic construct
  misc_feature 1..102: note = Epichloe festucae
  misc_feature 51: note = Variation - S is A strain AR37 or G strain RGT18
  source 1..102: mol_type = other DNA
gttgctacatcagctatacgtccacgtagagcggacacggatcaagatttstcgcgctggaagagatgcattcctatctttatgaatccatcgccagtatcc

SEQ ID NO: 659 - DNA, 102 bp, synthetic construct
  misc_feature 1..102: note = Epichloe festucae
  misc_feature 51: note = Variation - S is C strain AR37 or T strain RGT18
  source 1..102: mol_type = other DNA
ggagggggggggcaagcccagaccccctcaagcgcgcccgacttctagaasaagtctgcagctgattgtgtgtgggcttcatcatattagtttcagttacta

SEQ ID NO: 660 - DNA, 102 bp, synthetic construct
  misc_feature 1..102: note = Epichloe festucae
  misc_feature 51: note = Variation - S is A strain AR37 or G strain RGT18
  source 1..102: mol_type = other DNA
gtctagcggccttttgcgcccctcgtgggcgaaatggggcgaatgggcgastggggcgagtggggcgagtggggcgagtggggcgagtggatccccctgatc

SEQ ID NO: 661 - DNA, 102 bp, synthetic construct
  misc_feature 1..102: note = Epichloe festucae
  misc_feature 51: note = Variation - S is G strain AR37 or A strain RGT18
  source 1..102: mol_type = other DNA
gtgattttaatagataatttttctttaatttacttagctaggtaaagaatsaatctagttatagtctaactatttctatctaggatagttatcttttaaggc

SEQ ID NO: 662 - DNA, 102 bp, synthetic construct
  misc_feature 1..102: note = Epichloe festucae
  misc_feature 51: note = Variation - S is T strain AR37 or A strain RGT18
  source 1..102: mol_type = other DNA
tctgcatcttttttgcgtcctcgtgcagggaaccttgtgggtatttttttstttttggtttctgccagatgcggttggaaatttgaaggctcaggttggggt

SEQ ID NO: 663 - DNA, 102 bp, synthetic construct
  misc_feature 1..102: note = Epichloe festucae
  misc_feature 51: note = Variation - S is A strain AR37 or T strain RGT18
  source 1..102: mol_type = other DNA
tccaagaggggctgagagcagacttggtcctggtggagggtgacccgttgsatgacattcgggacactctaaacctgagaggcgtgtggaagaagggcattc

SEQ ID NO: 664 - DNA, 102 bp, synthetic construct
  misc_feature 1..102: note = Epichloe festucae
  misc_feature 51: note = Variation - S is G strain AR37 or A strain RGT18
  source 1..102: mol_type = other DNA
gaccattgagcattagtaacaggagtagatgtggttgtcttttgtcacaasctgctctgagtgagacgtggcaccgactgctatcagccgatggtgaagtcg

SEQ ID NO: 665 - DNA, 102 bp, synthetic construct
  misc_feature 1..102: note = Epichloe festucae
  misc_feature 51: note = Variation - S is C strain AR37 or G strain RGT18
  source 1..102: mol_type = other DNA
gcccgaaacgtcgagaaggctggccttatcgtaagaccattgaaaaaacascagtctatacaagttttttggtactggtcgacaaatgtttgctgacaagag

SEQ ID NO: 666 - DNA, 102 bp, synthetic construct
  misc_feature 1..102: note = Epichloe festucae
  misc_feature 51: note = Variation - S is C strain AR37 or T strain RGT18
  source 1..102: mol_type = other DNA
cgcaggtctcgagctgcctctcgacgaagactcgttgttgtgtcggtgtgscgcgcgtggctgtggggagatttctgtgggcgtgtcggaatcggggtcgac

SEQ ID NO: 667 - DNA, 102 bp, synthetic construct
  misc_feature 1..102: note = Epichloe festucae
  misc_feature 51: note = Variation - S is G strain AR37 or C strain RGT18
  source 1..102: mol_type = other DNA
gaacaactgtggaaacaaaacatgcatcttctagctttgaaagcaaaggcsaatctgtacacgtcgtggggggaaatcgctattcgatttcaaacatctcgt

SEQ ID NO: 668 - DNA, 102 bp, synthetic construct
  misc_feature 1..102: note = Epichloe festucae
  misc_feature 51: note = Variation - S is C strain AR37 or T strain RGT18
  source 1..102: mol_type = other DNA
tttgtctttatcacgatcccctcctccccttacggagtacacccccccccsgcgattccccaaccgcaatactgccccctcgctcactcgtgcggaaaggaa

SEQ ID NO: 669 - DNA, 102 bp, synthetic construct
  misc_feature 1..102: note = Epichloe festucae
  misc_feature 51: note = Variation - S is C strain AR37 or A strain RGT18
  source 1..102: mol_type = other DNA
tttgtggaatggaaaaaaagaataaaaaagaacgctttatattcaatcgcsaaggactcacaatttggagtgaagacgctattaacagaactgacttccaaa

SEQ ID NO: 670 - DNA, 102 bp, synthetic construct
  misc_feature 1..102: note = Epichloe festucae
  misc_feature 51: note = Variation - S is T strain AR37 or C strain RGT18
  source 1..102: mol_type = other DNA
cgacctgcgcagggacgagcggcccgagctgggctatcaggtcggcgtgasgctcgaggggaccgagaggcccaggtgcgccgtcgacgagccctgcctgga

SEQ ID NO: 671 - DNA, 102 bp, synthetic construct
  misc_feature 1..102: note = Epichloe festucae
  misc_feature 51: note = Variation - S is G strain AR37 or A strain RGT18
  source 1..102: mol_type = other DNA
gagagaaagcatagaagtaaactctaggagtagctttagtataagggatasgctagtttatcttactaatcccttttactaatctaggatagcttactatct

SEQ ID NO: 672 - DNA, 102 bp, synthetic construct
  misc_feature 1..102: note = Epichloe festucae
  misc_feature 51: note = Variation - S is C strain AR37 or A strain RGT18
  source 1..102: mol_type = other DNA
ggtcctggtgcgcatggccccttgtatcttcagcacaaacgggtcccgtastactacgcaccacaacaccgaccgcttcgtgaagaatagcaacgcaatggg

SEQ ID NO: 673 - DNA, 102 bp, synthetic construct
  misc_feature 1..102: note = Epichloe festucae
  misc_feature 51: note = Variation - S is T strain AR37 or C strain RGT18
  source 1..102: mol_type = other DNA
cgaggccccagccggatgaggaagcaacaactctctctggactttttttcsttcgatggtggtcgtgagatgtaccgagtaccgagtaatgtatagtgtgtt

SEQ ID NO: 674 - DNA, 102 bp, synthetic construct
  misc_feature 1..102: note = Epichloe festucae
  misc_feature 51: note = Variation - S is A strain AR37 or G strain RGT18
  source 1..102: mol_type = other DNA
aaaggcgccgagagtcattgcgccgaacgtgacagtttcatgttctcaacstccgagacgagtctgccagaaatcagaatagacgagagtagctgtcctggc

SEQ ID NO: 675 - DNA, 102 bp, synthetic construct
  misc_feature 1..102: note = Epichloe festucae
  misc_feature 51: note = Variation - S is G strain AR37 or A strain RGT18
  source 1..102: mol_type = other DNA
atcaaattggctcgcgagtctcaggttcctgttccccggatagagacgctstatgccattctccataatctcaacattgtcaaccgttccaggcctaagcct

SEQ ID NO: 676 - DNA, 102 bp, synthetic construct
  misc_feature 1..102: note = Epichloe festucae
  misc_feature 51: note = Variation - S is T strain AR37 or C strain RGT18
  source 1..102: mol_type = other DNA
aggttgaatcttttggtttaatagcttacccttatacctttaggttctaasattaatgctagctcttataggtcttctagtgtactagtcctaggtttaatt

SEQ ID NO: 677 - DNA, 102 bp, synthetic construct
  misc_feature 1..102: note = Epichloe festucae
  misc_feature 51: note = Variation - S is C strain AR37 or A strain RGT18
  source 1..102: mol_type = other DNA
tgctcacatggacaacccaaccttctctagtccaacgacgatgtcttcaasaccaaccaccccctcttccactggatgttccgcgcttcccgcaactggggc

SEQ ID NO: 678 - DNA, 102 bp, synthetic construct
  misc_feature 1..102: note = Epichloe festucae
  misc_feature 51: note = Variation - S is T strain AR37 or G strain RGT18
  source 1..102: mol_type = other DNA
ctctgttcttttctgatgcctcctggtcgtccgacgtctcactggaagctsactcgttagtgacagccatcacatgctcttcgggccgccacccatcaccac

SEQ ID NO: 679 - DNA, 102 bp, synthetic construct
  misc_feature 1..102: note = Epichloe festucae
  misc_feature 51: note = Variation - S is G strain AR37 or A strain RGT18
  source 1..102: mol_type = other DNA
ccgccgcggggcagagctctacggagtattacagcctgtcactcagtggtscttgacgctccgtatactgacattgaacgaggcgcaggggcgggcgccttc

SEQ ID NO: 680 - DNA, 102 bp, synthetic construct
  misc_feature 1..102: note = Epichloe festucae
  misc_feature 51: note = Variation - S is A strain AR37 or G strain RGT18
  source 1..102: mol_type = other DNA
ttagggtcatgaaagcatggagatgtatggagcaaaggcttgtgcagcacsaacaaatgtgtcgtgtaattctctgccaacccaggagctgatgttttggcg

SEQ ID NO: 681 - DNA, 102 bp, synthetic construct
  misc_feature 1..102: note = Epichloe festucae
  misc_feature 51: note = Variation - S is T strain AR37 or C strain RGT18
  source 1..102: mol_type = other DNA
ctcgcagtttgcatgcgtaccggcaagattcaaccccatagttgtccgcascatggccgagtgtgaaattgctgaaatcaccttgcaagtcatagcagcgga

SEQ ID NO: 682 - DNA, 102 bp, synthetic construct
  misc_feature 1..102: note = Epichloe festucae
  misc_feature 51: note = Variation - S is A strain AR37 or G strain RGT18
  source 1..102: mol_type = other DNA
aacatccagctgtcgactgccatggcgagcgacatatctgatgagtcttcscgaggctctaccatggccataatcggagcatgcttctccattgcctttacc

SEQ ID NO: 683 - DNA, 102 bp, synthetic construct
  misc_feature 1..102: note = Epichloe festucae
  misc_feature 51: note = Variation - S is T strain AR37 or C strain RGT18
  source 1..102: mol_type = other DNA
tagtaaaatagcaaaaaactaaatagttttataatagggagcgctagtaasactagttttacctagcctaaataaaacactacctatattattagataaatt

SEQ ID NO: 684 - DNA, 102 bp, synthetic construct
  misc_feature 1..102: note = Epichloe festucae
  misc_feature 51: note = Variation - S is C strain AR37 or T strain RGT18
  source 1..102: mol_type = other DNA
acccagctgaagagcgcgcgagccgaggcgcgagcctcatttggccaaggsggcgaggttatgctggtggaaaagtatattgtacggccacgtcacgtcgaa

SEQ ID NO: 685 - DNA, 102 bp, synthetic construct
  misc_feature 1..102: note = Epichloe festucae
  misc_feature 51: note = Variation - S is T strain AR37 or C strain RGT18
  source 1..102: mol_type = other DNA
tctacacgaccacaatgtactctgaaatgccatgtccaacacacctttttstcgacatcatccgaatcaatcgtctcagaacccaagcgacggctggcgtgt

SEQ ID NO: 686 - DNA, 102 bp, synthetic construct
  misc_feature 1..102: note = Epichloe festucae
  misc_feature 51: note = Variation - S is G strain AR37 or A strain RGT18
  source 1..102: mol_type = other DNA
tattactatagtaaataataaaaggtaggatttatataattacttatatastaaaggatagtctatagttaaaaaaggtaaaaggaagctaaaagtttactt

SEQ ID NO: 687 - DNA, 102 bp, synthetic construct
  misc_feature 1..102: note = Epichloe festucae
  misc_feature 51: note = Variation - S is C strain AR37 or T strain RGT18
  source 1..102: mol_type = other DNA
tacaatagcaaagcttgattttcaactcggggggcggtttttttcttcttstttttttttttggggggggggggcatcgcatagcttgtgtagagggcatgg

SEQ ID NO: 688 - DNA, 102 bp, synthetic construct
  misc_feature 1..102: note = Epichloe festucae
  misc_feature 51: note = Variation - S is G strain AR37 or T strain RGT18
  source 1..102: mol_type = other DNA
agcaggaggagcaggaggagcaggctggttgtcaggaggaggagcaggctsgttgtcaggaggaggagcaggctggttgtcaggagtaggagcaggcttgtt

SEQ ID NO: 689 - DNA, 102 bp, synthetic construct
  misc_feature 1..102: note = Epichloe festucae
  misc_feature 51: note = Variation - S is A strain AR37 or G strain RGT18
  source 1..102: mol_type = other DNA
gaaggcgctagacggggcgttgaatcaagcacgacagccgcgggacatggsacttgggactggaggcgcacgccccccccccggccttggatatgtggtcca

SEQ ID NO: 690 - DNA, 102 bp, synthetic construct
  misc_feature 1..102: note = Epichloe festucae
  misc_feature 51: note = Variation - S is G strain AR37 or A strain RGT18
  source 1..102: mol_type = other DNA
tgtttcaaggttttgtcatgagagccgtcaaagagaagggccaatatgacsaaaaaaaaaaaaaaaaaagggatgaatctgcatatattggtcaaggagtcg

SEQ ID NO: 691 - DNA, 102 bp, synthetic construct
  misc_feature 1..102: note = Epichloe festucae
  misc_feature 51: note = Variation - S is G strain AR37 or T strain RGT18
  source 1..102: mol_type = other DNA
cactagtctgtttttggctgtggcttccgagagagcggttggggggggggstccattctcttcgcttgcacaccggtgacacacgtgacaagcagccctaaa

SEQ ID NO: 692 - DNA, 102 bp, synthetic construct
  misc_feature 1..102: note = Epichloe festucae
  misc_feature 51: note = Variation - S is G strain AR37 or C strain RGT18
  source 1..102: mol_type = other DNA
agggccgtccttgggcttcctggatgcaggctcgctggctagaccgagggsctctctcattttcttgcgagcaagctcctttttggacaattttggtgcacc

SEQ ID NO: 693 - DNA, 102 bp, synthetic construct
  misc_feature 1..102: note = Epichloe festucae
  misc_feature 51: note = Variation - S is C strain AR37 or T strain RGT18
  source 1..102: mol_type = other DNA
tctaattaaatagttaataattagtaaataagtaagtaagaaaaatctaastaaaaagtaataatccttaaggaagaagaaattaaactcttaccttagaga

SEQ ID NO: 694 - DNA, 102 bp, synthetic construct
  misc_feature 1..102: note = Epichloe festucae
  misc_feature 51: note = Variation - S is C strain AR37 or T strain RGT18
  source 1..102: mol_type = other DNA
tccgaggccttttgtgatttggccgaatacgagaagtcccgaagagctggstccatgcccaaagccatgcccaacaagccatgccaaacgccaattttggca

SEQ ID NO: 695 - DNA, 102 bp, synthetic construct
  misc_feature 1..102: note = Epichloe festucae
  misc_feature 51: note = Variation - S is G strain AR37 or A strain RGT18
  source 1..102: mol_type = other DNA
gcgtctcttgacatgtcgacaagacgaagctggttgcgatgagaacatgtstacaatgtccaatcatctgagcaaaatgatcaaaaacgccatcccagtgtg

SEQ ID NO: 696 - DNA, 102 bp, synthetic construct
  misc_feature 1..102: note = Epichloe festucae
  misc_feature 51: note = Variation - S is G strain AR37 or C strain RGT18
  source 1..102: mol_type = other DNA
tgctatgataccgtcttttgcagccaatactgtcacgacattgcccaggascgctaccacccatccgtgtgcgagaaggacgtggatgctattgccaaggac

SEQ ID NO: 697 - DNA, 102 bp, synthetic construct
  misc_feature 1..102: note = Epichloe festucae
  misc_feature 51: note = Variation - S is T strain AR37 or C strain RGT18
  source 1..102: mol_type = other DNA
ttttttttccccctttcctcaacgacagccacttttttttttttttttttscccctttcctcaacgacagccacaaagcgccaacagccgagggctcgctaa

SEQ ID NO: 698 - DNA, 102 bp, synthetic construct
  misc_feature 1..102: note = Epichloe festucae
  misc_feature 51: note = Variation - S is T strain AR37 or C strain RGT18
  source 1..102: mol_type = other DNA
tacatgtttgcatgccaagctagttagtctcatttgcatgtgtctcagccsttttttttttttttttttttttaacttgtgttgattctgcgaagccgaatt

SEQ ID NO: 699 - DNA, 102 bp, synthetic construct
  misc_feature 1..102: note = Epichloe festucae
  misc_feature 51: note = Variation - S is T strain AR37 or C strain RGT18
  source 1..102: mol_type = other DNA
taatttacgagcgcgagtcaccggagataatggtgcccaaagtccaaagtsggcaactgattgcgccggttgatcaatctccacgtgaacattctgccattg

SEQ ID NO: 700 - DNA, 102 bp, synthetic construct
  misc_feature 1..102: note = Epichloe festucae
  misc_feature 51: note = Variation - S is C strain AR37 or T strain RGT18
  source 1..102: mol_type = other DNA
ttcttccgacattgtctgatgaataacggccgtctccaacatgtcccatgsctcagactgcgaatccaagatcgccagagactgtgaatataaggtttcctg

SEQ ID NO: 701 - DNA, 102 bp, synthetic construct
  misc_feature 1..102: note = Epichloe festucae
  misc_feature 51: note = Variation - S is C strain AR37 or G strain RGT18
  source 1..102: mol_type = other DNA
tttggacagtgccatgacgatggactcaccctctctgaaggcaatcaaggsgaagaagcgaaaacgcgagagtcttaacattcggcccgagagggagcagat

SEQ ID NO: 702 - DNA, 102 bp, synthetic construct
  misc_feature 1..102: note = Epichloe festucae
  misc_feature 51: note = Variation - S is A strain AR37 or T strain RGT18
  source 1..102: mol_type = other DNA
ccctagatttattaaattattttaagtacttaatactataggtaaataagsatataaacttatattacctaaaaaatatagttaactatataatatatttta

SEQ ID NO: 703 - DNA, 102 bp, synthetic construct
  misc_feature 1..102: note = Epichloe festucae
  misc_feature 51: note = Variation - S is T strain AR37 or C strain RGT18
  source 1..102: mol_type = other DNA
aaggcctggagctggagccatgattgggcagtgcacgcgtggcctgaattstttacccttgtgccccaactgcccctccttcagagcaggaatgaaggggcc

SEQ ID NO: 704 - DNA, 102 bp, synthetic construct
  misc_feature 1..102: note = Epichloe festucae
  misc_feature 51: note = Variation - S is G strain AR37 or C strain RGT18
  source 1..102: mol_type = other DNA
cttgaccttcaaagacgtcattagccgacttggccgcgggggggggggggsggcgcaggcacaagacaagaaaacaagcgaggacttacaggctccaaaggc

SEQ ID NO: 705 - DNA, 102 bp, synthetic construct
  misc_feature 1..102: note = Epichloe festucae
  misc_feature 51: note = Variation - S is C strain AR37 or G strain RGT18
  source 1..102: mol_type = other DNA
aagtcaatagaggagtttgacagcgagggcgtcggtttgatcggaaagcgscccctttcacagcagccagtcatggtcaaggcaaagatgtggcagagataa

SEQ ID NO: 706 - DNA, 102 bp, synthetic construct
  misc_feature 1..102: note = Epichloe festucae
  misc_feature 51: note = Variation - S is G strain AR37 or T strain RGT18
  source 1..102: mol_type = other DNA
tctccccccggagtacacgatgcgtcccatccggatggaggttcacgatasaatggacctccgaggcgagatccctgagagaatatgtctgttggcaagtga

SEQ ID NO: 707 - DNA, 102 bp, synthetic construct
  misc_feature 1..102: note = Epichloe festucae
  misc_feature 51: note = Variation - S is G strain AR37 or C strain RGT18
  source 1..102: mol_type = other DNA
agagaaagcaggacgaggaagaggaagagctcgtttctcttcccgaggaasatgatggcgaggaggaagaagagtgagtgaccagcgccaacgaacccaagc

SEQ ID NO: 708 - DNA, 102 bp, synthetic construct
  misc_feature 1..102: note = Epichloe festucae
  misc_feature 51: note = Variation - S is T strain AR37 or C strain RGT18
  source 1..102: mol_type = other DNA
aattgactactggaaagaccatgcacaaataattcactcatatggcccgtstgaatgcactcccatatctatcagtcatatcctggatcccgatcgatctcg

SEQ ID NO: 709 - DNA, 102 bp, synthetic construct
  misc_feature 1..102: note = Epichloe festucae
  misc_feature 51: note = Variation - S is A strain AR37 or T strain RGT18
  source 1..102: mol_type = other DNA
gatggcctaaccagaaggggcatcagcaaaaaaaaaaaaaaaaaaaaaaasagttcaataatgtaggagactttttttgcggctcccaattcatacgacgta

SEQ ID NO: 710 - DNA, 102 bp, synthetic construct
  misc_feature 1..102: note = Epichloe festucae
  misc_feature 51: note = Variation - S is C strain AR37 or T strain RGT18
  source 1..102: mol_type = other DNA
acacttagaagtgggcaggggttattatattggataataaggcagtgaggsaggtgcctattaaacgctttataaatagctattagtaaggatagtttttat

SEQ ID NO: 711 - DNA, 102 bp, synthetic construct
  misc_feature 1..102: note = Epichloe festucae
  misc_feature 51: note = Variation - S is T strain AR37 or C strain RGT18
  source 1..102: mol_type = other DNA
acgaactcacgagagatagccttacaatcctttcagagatggtgtaccaastatgaccagcactatttcagagtcaagcgcagtaatatgccctgcgcgatc

SEQ ID NO: 712 - DNA, 102 bp, synthetic construct
  misc_feature 1..102: note = Epichloe festucae
  misc_feature 51: note = Variation - S is T strain AR37 or A strain RGT18
  source 1..102: mol_type = other DNA
atgacgcgtggagatgtgtcgagattttcaacccaagaccaaaagtccttstgtgcacgttttgcattggtaaaatccgtgctgtttgccaaagggcataca

SEQ ID NO: 713 - DNA, 102 bp, synthetic construct
  misc_feature 1..102: note = Epichloe festucae
  misc_feature 51: note = Variation - S is T strain AR37 or C strain RGT18
  source 1..102: mol_type = other DNA
tccaaggccttgatagtctagaaacaacagacagctcgtgcgaagcggtasgattccatcgttgaccacgttggagtatgttgtgcggtttctgaatttctt

SEQ ID NO: 714 - DNA, 102 bp, synthetic construct
  misc_feature 1..102: note = Epichloe festucae
  misc_feature 51: note = Variation - S is C strain AR37 or T strain RGT18
  source 1..102: mol_type = other DNA
catcgcgggcatcaccggcccacacttgattgtcgttcccaagtcaacatsggacaattggaagcgagagttcgccaggtggacgccagaggtcaacgtttt

SEQ ID NO: 715 - DNA, 102 bp, synthetic construct
  misc_feature 1..102: note = Epichloe festucae
  misc_feature 51: note = Variation - S is A strain AR37 or G strain RGT18
  source 1..102: mol_type = other DNA
aaatctcggatgaggacccgagaaatcttgagcaagagctggtctcttctsctgggcaagctgtaaatgaacaaaagttggtcgtgttgacttccaagaaat

SEQ ID NO: 716 - DNA, 102 bp, synthetic construct
  misc_feature 1..102: note = Epichloe festucae
  misc_feature 51: note = Variation - S is A strain AR37 or G strain RGT18
  source 1..102: mol_type = other DNA
ggcccgtttgcctgaatcaggggcatggactttctgtaaacctgccaatasgacggctgtggttggttgtaattgtattacataataataaacgaaagcaag

SEQ ID NO: 717 - DNA, 102 bp, synthetic construct
  misc_feature 1..102: note = Epichloe festucae
  misc_feature 51: note = Variation - S is G strain AR37 or A strain RGT18
  source 1..102: mol_type = other DNA
gcggttacagctgcgagaggatggggcgaaccagggacggcaacggcgttstgaaagctggttggctggcaggggaccaagttaagcgcccgggcgagcagg

SEQ ID NO: 718 - DNA, 102 bp, synthetic construct
  misc_feature 1..102: note = Epichloe festucae
  misc_feature 51: note = Variation - S is T strain AR37 or G strain RGT18
  source 1..102: mol_type = other DNA
atttttgagttgcaaatattcgtcacttggtccagcctcttgtctttttascacgtaggagagcagtagcgatagctaggtgggacgaggactggagaagag

SEQ ID NO: 719 - DNA, 102 bp, synthetic construct
  misc_feature 1..102: note = Epichloe festucae
  misc_feature 51: note = Variation - S is A strain AR37 or G strain RGT18
  source 1..102: mol_type = other DNA
ggcatgtgccgatcaataacactccacaaaggccatgagcgttgcggaagsacgcagagctatttatctatgtgccaaactggctcttcacccggctcgctt

SEQ ID NO: 720 - DNA, 102 bp, synthetic construct
  misc_feature 1..102: note = Epichloe festucae
  misc_feature 51: note = Variation - S is T strain AR37 or G strain RGT18
  source 1..102: mol_type = other DNA
cgccaattgtttccctgttggtctgcggagattcagtcctccgagcggtgstttttcctcttcatggcattccgcagcgaggggatgttacgagagcagcga

SEQ ID NO: 721 - DNA, 102 bp, synthetic construct
  misc_feature 1..102: note = Epichloe festucae
  misc_feature 51: note = Variation - S is T strain AR37 or A strain RGT18
  source 1..102: mol_type = other DNA
ttaatagttttattactataagtaaagtaatataacccttaaaaatattastacttaaaaccctaaaaaaagtaagcttaaataccttaagattttattaac

SEQ ID NO: 722 - DNA, 102 bp, synthetic construct
  misc_feature 1..102: note = Epichloe festucae
  misc_feature 51: note = Variation - S is A strain AR37 or T strain RGT18
  source 1..102: mol_type = other DNA
tgtacgtcttgtacggaccaacgataatcgtatgataattattatataatsaactttcaaagaacacaaaacacttcctatgtagcaagcttccggagattc

SEQ ID NO: 723 - DNA, 102 bp, synthetic construct
  misc_feature 1..102: note = Epichloe festucae
  misc_feature 51: note = Variation - S is A strain AR37 or G strain RGT18
  source 1..102: mol_type = other DNA
gccccctatcaaagctgatgccgccccgcacatgctccgtgccgccggggsaataggaaaataagccggctcttcgtgcctttttactccgtaccttgtccc

SEQ ID NO: 724 - DNA, 102 bp, synthetic construct
  misc_feature 1..102: note = Epichloe festucae
  misc_feature 51: note = Variation - S is T strain AR37 or A strain RGT18
  source 1..102: mol_type = other DNA
ttcgactcgtccgtgagggcgacgggagagaagacggcgaggttgccagasgtgagtttgactgaaagaggggggggggggggggggttgcagttggtcagt

SEQ ID NO: 725 - DNA, 102 bp, synthetic construct
  misc_feature 1..102: note = Epichloe festucae
  misc_feature 51: note = Variation - S is G strain AR37 or A strain RGT18
  source 1..102: mol_type = other DNA
ctaggttccccgtcgtcggcgtccgcgacggcctcgtctccagcgtcgacscaacactctcgggcagggcggcgtaaaacgcattcaggcaattgattgtcc

SEQ ID NO: 726 - DNA, 102 bp, synthetic construct
  misc_feature 1..102: note = Epichloe festucae
  misc_feature 51: note = Variation - S is C strain AR37 or T strain RGT18
  source 1..102: mol_type = other DNA
gtaccgtgggcacagtggttcctgaggtttgaagtgaagaggtcgaggggstgaccaaggttgagcctacagtagagatgctgcttgtactgtcactgctgc

SEQ ID NO: 727 - DNA, 102 bp, synthetic construct
  misc_feature 1..102: note = Epichloe festucae
  misc_feature 51: note = Variation - S is C strain AR37 or T strain RGT18
  source 1..102: mol_type = other DNA
taacctcaccatccgagtcgcctcgtttgaattccgagacgtggtcaactsgtgatctcttgacacgatccaggtcggcatagaacctcttcgcaccggcac

SEQ ID NO: 728 - DNA, 102 bp, synthetic construct
  misc_feature 1..102: note = Epichloe festucae
  misc_feature 51: note = Variation - S is T strain AR37 or C strain RGT18
  source 1..102: mol_type = other DNA
gtcggcaactgccagctcctcgatggacagaatgaagccacagtgttgacsgatacaggaagagctgccagagactttgtggacttctttgctgctagctta

SEQ ID NO: 729 - DNA, 102 bp, synthetic construct
  misc_feature 1..102: note = Epichloe festucae
  misc_feature 51: note = Variation - S is A strain AR37 or T strain RGT18
  source 1..102: mol_type = other DNA
cctatctttaatctttatactcctaatataatacctcccttatatataatsaaccttaattataaaataagctacttacttagggtatagttactatattaa

SEQ ID NO: 730 - DNA, 102 bp, synthetic construct
  misc_feature 1..102: note = Epichloe festucae
  misc_feature 51: note = Variation - S is A strain AR37 or T strain RGT18
  source 1..102: mol_type = other DNA
agtcgtaccaagatggcgaggtgttagaggcttttttgtattatgtgtctsctagaacggcgacgtcggcatgaagcgcgaataggagcacacggcacgact

SEQ ID NO: 731 - DNA, 102 bp, synthetic construct
  misc_feature 1..102: note = Epichloe festucae
  misc_feature 51: note = Variation - S is G strain AR37 or A strain RGT18
  source 1..102: mol_type = other DNA
ggaaagaaaaagaaaaaaaaaaaaaaataagttgtgtggggaaagaaaaasaaaaaaaaaaaaaaagcacagcctaagcacaaaatgtccacatgcttcctt

SEQ ID NO: 732 - DNA, 102 bp, synthetic construct
  misc_feature 1..102: note = Epichloe festucae
  misc_feature 51: note = Variation - S is T strain AR37 or C strain RGT18
  source 1..102: mol_type = other DNA
gcaccattgggcaggataactctgctggcgtacaacgtgtcgacactgtasgcttacagtttgagtcagaaggtagatgatgatgacgatgacgaaggcgga

SEQ ID NO: 733 - DNA, 102 bp, synthetic construct
  misc_feature 1..102: note = Epichloe festucae
  misc_feature 51: note = Variation - S is T strain AR37 or G strain RGT18
  source 1..102: mol_type = other DNA
cacccctctcctcttccaatcgccattcgccaaatcgccaagaattgaaastaaaaaaaaaaaaaaaaaaaaggttgaagctttactaaccgctgtgtgcct

SEQ ID NO: 734 - DNA, 102 bp, synthetic construct
  misc_feature 1..102: note = Epichloe festucae
  misc_feature 51: note = Variation - S is A strain AR37 or T strain RGT18
  source 1..102: mol_type = other DNA
ctttacgagctcctcggtcccccgactctccgtggccacttttgcgcatcsacaccacgacgagatcatggcgactccagacgccaaggcgtctcgcgcccc

SEQ ID NO: 735 - DNA, 102 bp, synthetic construct
  misc_feature 1..102: note = Epichloe festucae
  misc_feature 51: note = Variation - S is A strain AR37 or T strain RGT18
  source 1..102: mol_type = other DNA
tggccctcctcgtccgggatcattggtggcccgaatgaggtttgaggcgasaagacggtgttataatgacgccttgtgcattcgacggcatcttgttcagaa

SEQ ID NO: 736 - DNA, 102 bp, synthetic construct
  misc_feature 1..102: note = Epichloe festucae
  misc_feature 51: note = Variation - S is A strain AR37 or C strain RGT18
  source 1..102: mol_type = other DNA
ctgtacaacgcggcgaggacaagaatttttgtggcatgtcttgcgataaasagacattcaagagatttatatcccgacatgggtatatttgccatgtgatgt

SEQ ID NO: 737 - DNA, 102 bp, synthetic construct
  misc_feature 1..102: note = Epichloe festucae
  misc_feature 51: note = Variation - S is T strain AR37 or A strain RGT18
  source 1..102: mol_type = other DNA
agcttggcctcacttatccaattgtttcttcgcatttggcaacatactgtscgcgagtttgagtgggtaacttctggtattgtccttgctacttatggattt

SEQ ID NO: 738 - DNA, 102 bp, synthetic construct
  misc_feature 1..102: note = Epichloe festucae
  misc_feature 51: note = Variation - S is G strain AR37 or A strain RGT18
  source 1..102: mol_type = other DNA
ctcaaatgtacggatccgtagaacgtctgcttgttggccgttgtacgcctsccgttcctcttttttcttttcttcttttccctcaacttttccgtgtgtggg

SEQ ID NO: 739 - DNA, 102 bp, synthetic construct
  misc_feature 1..102: note = Epichloe festucae
  misc_feature 51: note = Variation - S is T strain AR37 or A strain RGT18
  source 1..102: mol_type = other DNA
agacctggtacacttgcattagtgctgtacgcagactgcacggtccatatsgaaaaaaaaaaaaaaaaaaaaaaaaaaaaggccgtactcacgtttctgaag

SEQ ID NO: 740 - DNA, 102 bp, synthetic construct
  misc_feature 1..102: note = Epichloe festucae
  misc_feature 51: note = Variation - S is T strain AR37 or A strain RGT18
  source 1..102: mol_type = other DNA
gcaaaaatggacaagaatccggattctcttttttttttttttttttttttsagagggtccgggtccccctttggaatcgcctcgaaacaccaaaacaccaac

SEQ ID NO: 741 - DNA, 102 bp, synthetic construct
  misc_feature 1..102: note = Epichloe festucae
  misc_feature 51: note = Variation - S is T strain AR37 or C strain RGT18
  source 1..102: mol_type = other DNA
ctttccccttctttttcttcttgcctcgcggcgcgttccgggtccacacastcccggggaagctgggaagctgggaagctgggatctaggaagctaggaagg

SEQ ID NO: 742 - DNA, 102 bp, synthetic construct
  misc_feature 1..102: note = Epichloe festucae
  misc_feature 51: note = Variation - S is G strain AR37 or T strain RGT18
  source 1..102: mol_type = other DNA
agacaccaacatgcgattcttcagcaactcagtggcttctgctactctttsggccgctactctatctcaagcgcaaatcctcatcaatgagcaaagctttgg

SEQ ID NO: 743 - DNA, 102 bp, synthetic construct
  misc_feature 1..102: note = Epichloe festucae
  misc_feature 51: note = Variation - S is C strain AR37 or T strain RGT18
  source 1..102: mol_type = other DNA
atcagccagcgtgttgcccgcgtgttaacggtcgctcaatcggcccccccscccccccaaattggttgaagacatgcactgatgacgaggcgctgcggggag

SEQ ID NO: 744 - DNA, 102 bp, synthetic construct
  misc_feature 1..102: note = Epichloe festucae
  misc_feature 51: note = Variation - S is A strain AR37 or G strain RGT18
  source 1..102: mol_type = other DNA
gtcacatggctctgctgcgaaggacgtgttccatgctgatgatcgattagstgaaacttgttgcggtcttgacagctgcaagggtcccgtggagatgccacg

SEQ ID NO: 745 - DNA, 102 bp, synthetic construct
  misc_feature 1..102: note = Epichloe festucae
  misc_feature 51: note = Variation - S is C strain AR37 or A strain RGT18
  source 1..102: mol_type = other DNA
tcattgactgcctgtgagacgaagaccgatgtcggaaaagccatcgagtcstgcacggacgacatgctgtcgattcccgagaatcccgcgtttcgcaaaagt

SEQ ID NO: 746 - DNA, 102 bp, synthetic construct
  misc_feature 1..102: note = Epichloe festucae
  misc_feature 51: note = Variation - S is G strain AR37 or C strain RGT18
  source 1..102: mol_type = other DNA
cgtgcagctggcatgcctaatctggtatttgatcagctattttcccatggsgtccacgggtcttcgcctggcagcttcatttggcgccaggcaagcagcttc

SEQ ID NO: 747 - DNA, 102 bp, synthetic construct
  misc_feature 1..102: note = Epichloe festucae
  misc_feature 51: note = Variation - S is A strain AR37 or G strain RGT18
  source 1..102: mol_type = other DNA
ggaacgcaaccgtatacttggcatgttggcgttctggaaaaaaaaaagaasaaaagaagaaaagaaaaaaaaacccccatccgtggcaaacggttggatggt

SEQ ID NO: 748 - DNA, 102 bp, synthetic construct
  misc_feature 1..102: note = Epichloe festucae
  misc_feature 51: note = Variation - S is A strain AR37 or T strain RGT18
  source 1..102: mol_type = other DNA
ctttgaaggcaatgccctcattcgccgtctcgtccgcgttggtgtcctcgscgagtcccgcatgaagctcgattacgtgcttgccctgaagatcgaggattt

SEQ ID NO: 749 - DNA, 102 bp, synthetic construct
  misc_feature 1..102: note = Epichloe festucae
  misc_feature 51: note = Variation - S is T strain AR37 or C strain RGT18
  source 1..102: mol_type = other DNA
tgtggactatccttggctgatgggtatttcgaagttggaggctacgcatastgtgagcgggatgcatggagaagggtccaggcccagtcatatgcagagcaa

SEQ ID NO: 750 - DNA, 102 bp, synthetic construct
  misc_feature 1..102: note = Epichloe festucae
  misc_feature 51: note = Variation - S is G strain AR37 or T strain RGT18
  source 1..102: mol_type = other DNA
agcatcaggtttccgagagacgggtcgggcccccggggggggggggggggsgggtccctaatggatagatagaccaagacttacggagggagtggttcacgc

SEQ ID NO: 751 - DNA, 102 bp, synthetic construct
  misc_feature 1..102: note = Epichloe festucae
  misc_feature 51: note = Variation - S is T strain AR37 or A strain RGT18
  source 1..102: mol_type = other DNA
ggaccgcaccgtccgcctctggaatcgtgacaggggccactcccgcgacasataccacaccaagcgcatgcagcgcgtcatggcagccaaatggacccccga

SEQ ID NO: 752 - DNA, 102 bp, synthetic construct
  misc_feature 1..102: note = Epichloe festucae
  misc_feature 51: note = Variation - S is A strain AR37 or C strain RGT18
  source 1..102: mol_type = other DNA
cttcgctgcttcgcagaggttgggaatctcgtttatgaaactattcagccsctatcgcggaccaagtatgatcaatgagttcctcgatcctcacggcgaagg

SEQ ID NO: 753 - DNA, 102 bp, synthetic construct
  misc_feature 1..102: note = Epichloe festucae
  misc_feature 51: note = Variation - S is G strain AR37 or C strain RGT18
  source 1..102: mol_type = other DNA
aagtccaccgatgagtactcggagatcgtctacgagagaaaagcattctgsaaccacccccacacccgtacgcaacaaaggtagccgaactcctacgccaat

SEQ ID NO: 754 - DNA, 102 bp, synthetic construct
  misc_feature 1..102: note = Epichloe festucae
  misc_feature 51: note = Variation - S is G strain AR37 or A strain RGT18
  source 1..102: mol_type = other DNA
atattgccattccagagcgagaattcgttcttagacctttatcgcagtaascccaatcttgcccaaactaaaggacttgttgctattgaccacagtctcatt

SEQ ID NO: 755 - DNA, 102 bp, synthetic construct
  misc_feature 1..102: note = Epichloe festucae
  misc_feature 51: note = Variation - S is T strain AR37 or A strain RGT18
  source 1..102: mol_type = other DNA
atagcgacgttggcgcctctgcagttgcgcctggtcgtcatggacgcgacscgacttggacacggggccggtttttggtgggtactgggttgtccggcgcta

SEQ ID NO: 756 - DNA, 102 bp, synthetic construct
  misc_feature 1..102: note = Epichloe festucae
  misc_feature 51: note = Variation - S is C strain AR37 or T strain RGT18
  source 1..102: mol_type = other DNA
aaatttggcatctggagagtcttgacacccgtttttttttttttttttttstttctttttctttttttttttttttttttttctttctttttcttttggcca

SEQ ID NO: 757 - DNA, 102 bp, synthetic construct
  misc_feature 1..102: note = Epichloe festucae
  misc_feature 51: note = Variation - S is C strain AR37 or T strain RGT18
  source 1..102: mol_type = other DNA
atcgccgtaatatcggtaaatcaaatccatcgttgcgtgtttccccgatgsggatatgaaggcagagcgcaaagctaaagcacatcgtccttttaaccaatg

SEQ ID NO: 758 - DNA, 102 bp, synthetic construct
  misc_feature 1..102: note = Epichloe festucae
  misc_feature 51: note = Variation - S is G strain AR37 or A strain RGT18
  source 1..102: mol_type = other DNA
ggataatcttgttgcctagctgagagtaagaacggctttggggacatcatscttcatattggtcatggagcatgcccctctttatacctggttgtgcggatg

SEQ ID NO: 759 - DNA, 102 bp, synthetic construct
  misc_feature 1..102: note = Epichloe festucae
  misc_feature 51: note = Variation - S is C strain AR37 or G strain RGT18
  source 1..102: mol_type = other DNA
cggtggagcaacattcatcgacggcggggaaagagaaacaaagtctgtctsactctctctagcaagctccgagtccgagctgaccagatgctgccgacttga

SEQ ID NO: 760 - DNA, 102 bp, synthetic construct
  misc_feature 1..102: note = Epichloe festucae
  misc_feature 51: note = Variation - S is C strain AR37 or T strain RGT18
  source 1..102: mol_type = other DNA
ttattatcttatagagagttttatagctctcttataagattattagtagcsctcctaaatatatctttagtttaacctttaaaatcttctctaaagttcttc

SEQ ID NO: 761 - DNA, 102 bp, synthetic construct
  misc_feature 1..102: note = Epichloe festucae
  misc_feature 51: note = Variation - S is G strain AR37 or A strain RGT18
  source 1..102: mol_type = other DNA
attaaaaaagaggtaaataaagacactataaggatagatttaataaagctsaactaactagttctaggataagtaattaaggctattataagactataagaa

SEQ ID NO: 762 - DNA, 102 bp, synthetic construct
  misc_feature 1..102: note = Epichloe festucae
  misc_feature 51: note = Variation - S is G strain AR37 or C strain RGT18
  source 1..102: mol_type = other DNA
ttatttaatagatatctataaattcctaagaaaagcctataagacactaastaaagactagcttaactagtttaaactaattactataagtaagattattat

SEQ ID NO: 763 - DNA, 102 bp, synthetic construct
  misc_feature 1..102: note = Epichloe festucae
  misc_feature 51: note = Variation - S is A strain AR37 or G strain RGT18
  source 1..102: mol_type = other DNA
gttataagggtatttatgctagataagttactaagctaaggctattaaatsttaagatttattttatctaagggaaatagaatactactgctaataggttat

SEQ ID NO: 764 - DNA, 102 bp, synthetic construct
  misc_feature 1..102: note = Epichloe festucae
  misc_feature 51: note = Variation - S is T strain AR37 or A strain RGT18
  source 1..102: mol_type = other DNA
gtgtcatcatcttgcagttgttgtccctcgcacctggcactgcactgcacsgcacagcacagcacagcacagcacagcacagcactgcactgcactgacttg

SEQ ID NO: 765 - DNA, 102 bp, synthetic construct
  misc_feature 1..102: note = Epichloe festucae
  misc_feature 51: note = Variation - S is C strain AR37 or T strain RGT18
  source 1..102: mol_type = other DNA
cactagtccctttataatttctattagtcttttttaaagataactattctstaagtaaaacttctttaccttattatatagttttctatagtcctttatact

SEQ ID NO: 766 - DNA, 102 bp, synthetic construct
  misc_feature 1..102: note = Epichloe festucae
  misc_feature 51: note = Variation - S is T strain AR37 or G strain RGT18
  source 1..102: mol_type = other DNA
taatactattattataaggactataattctctatagccttactacctttastagtaattttactagtctttatagtagtctttatatatttagttattactt

SEQ ID NO: 767 - DNA, 102 bp, synthetic construct
  misc_feature 1..102: note = Epichloe festucae
  misc_feature 51: note = Variation - S is A strain AR37 or G strain RGT18
  source 1..102: mol_type = other DNA
aaatatgccgtaaaaaaggcctaaccttattagttactataaaaactattscctaaaggcctaggttatattactaaataataaaggaaaacatgcttagag

SEQ ID NO: 768 - DNA, 102 bp, synthetic construct
  misc_feature 1..102: note = Epichloe festucae
  misc_feature 51: note = Variation - S is A strain AR37 or G strain RGT18
  source 1..102: mol_type = other DNA
ttactttaaagctaaaataaaaggtttttaaagtaatttataactttaggsatataaatagtaagactattaaattaggttatttatattataatatagaag

SEQ ID NO: 769 - DNA, 102 bp, synthetic construct
  misc_feature 1..102: note = Epichloe festucae
  misc_feature 51: note = Variation - S is A strain AR37 or G strain RGT18
  source 1..102: mol_type = other DNA
cttattttccttataaagctttaatatagtaactacaccctaagtaagtascttattttataattaaggttaattatatataagggaggtattatattagga

SEQ ID NO: 770 - DNA, 102 bp, synthetic construct
  misc_feature 1..102: note = Epichloe festucae
  misc_feature 51: note = Variation - S is G strain AR37 or A strain RGT18
  source 1..102: mol_type = other DNA
tattaaagataataaataagagtttaaagttaactataatagaaggtattstaaatatctagttaaataaaaaggctataatactttagagaattcttaggt

SEQ ID NO: 771 - DNA, 102 bp, synthetic construct
  misc_feature 1..102: note = Epichloe festucae
  misc_feature 51: note = Variation - S is T strain AR37 or A strain RGT18
  source 1..102: mol_type = other DNA
tagaagaaaaaaaatagataacctatattaatttttataattagttaaaasaaataaggtacttaatactatagttctaaatagtctaactaaagggcttgt

SEQ ID NO: 772 - DNA, 102 bp, synthetic construct
  misc_feature 1..102: note = Epichloe festucae
  misc_feature 51: note = Variation - S is C strain AR37 or A strain RGT18
  source 1..102: mol_type = other DNA
tattagtaataagtaagaaaagtctttttattaataaggtattctagaatsttataagtactattttttaggagaatattttatattattacttactaataa

SEQ ID NO: 773 - DNA, 102 bp, synthetic construct
  misc_feature 1..102: note = Epichloe festucae
  misc_feature 51: note = Variation - S is T strain AR37 or C strain RGT18
  source 1..102: mol_type = other DNA
tctatctcttattctctttttcctttacttagtaactataaggcttacctstatctcttattctctttttcctttacttagtaaagctatatatttacctct

SEQ ID NO: 774 - DNA, 102 bp, synthetic construct
  misc_feature 1..102: note = Epichloe festucae
  misc_feature 51: note = Variation - S is G strain AR37 or C strain RGT18
  source 1..102: mol_type = other DNA
taaataggattaataaaataaagactttaaaacactattatataaaaacasgtgtataaatactatactagataaagaaaataaacttatataaggaagtaa

SEQ ID NO: 775 - DNA, 102 bp, synthetic construct
  misc_feature 1..102: note = Epichloe festucae
  misc_feature 51: note = Variation - S is T strain AR37 or G strain RGT18
  source 1..102: mol_type = other DNA
ttgtagaatcttgatgtgttctttgctgctgcgcgcggggggggggggggsgagattgcctctcgctggttggaaaaccgtgatattgccaagatgattgat

SEQ ID NO: 776 - DNA, 102 bp, synthetic construct
  misc_feature 1..102: note = Epichloe festucae
  misc_feature 51: note = Variation - S is T strain AR37 or A strain RGT18
  source 1..102: mol_type = other DNA
ttacttaaaggaaataattattctctaagtctttatttaaattaataaaasagcttatataagtatatattacctttatttaaagttagtgctttactaata

SEQ ID NO: 777 - DNA, 102 bp, synthetic construct
  misc_feature 1..102: note = Epichloe festucae
  misc_feature 51: note = Variation - S is G strain AR37 or A strain RGT18
  source 1..102: mol_type = other DNA
agattatacaaaagtcttatatttaacagcgattttctctttaactagagsttatacaaaagtcttatatatagcaaattaaagctagaagatagggctttc

SEQ ID NO: 778 - DNA, 102 bp, synthetic construct
  misc_feature 1..102: note = Epichloe festucae
  misc_feature 51: note = Variation - S is A strain AR37 or C strain RGT18
  source 1..102: mol_type = other DNA
aggctagtaaacactatttatatagtgtatctagataatatccttattttsttaaaaatataaaagaagcatactatatatattaaggaagttttagaatat

SEQ ID NO: 779 - DNA, 102 bp, synthetic construct
  misc_feature 1..102: note = Epichloe festucae
  misc_feature 51: note = Variation - S is G strain AR37 or A strain RGT18
  source 1..102: mol_type = other DNA
gggctgtatggatcatggtaagcaacatctgctactcttccctgtcttctstgcttcatctccttgaattattgcgtgtgcatttgcgtttcttgagttttt

SEQ ID NO: 780 - DNA, 102 bp, synthetic construct
  misc_feature 1..102: note = Epichloe festucae
  misc_feature 51: note = Variation - S is C strain AR37 or T strain RGT18
  source 1..102: mol_type = other DNA
acgtgttgttgcctctgtcctaagcgtccgcagttgaagcgcattgctgascgcagcctcagcttcttggattagtgctcgccgttacactgtcttcgtatt

SEQ ID NO: 781 - DNA, 102 bp, synthetic construct
  misc_feature 1..102: note = Epichloe festucae
  misc_feature 51: note = Variation - S is T strain AR37 or A strain RGT18
  source 1..102: mol_type = other DNA
tactattttaactaccttttattagtatatataagggtactataatcctasagtattagtaaataaacctttagtaaaagttataaaatcctaggaaagact

SEQ ID NO: 782 - DNA, 102 bp, synthetic construct
  misc_feature 1..102: note = Epichloe festucae
  misc_feature 51: note = Variation - S is T strain AR37 or C strain RGT18
  source 1..102: mol_type = other DNA
tcctagtattatttttaaaaataagttaaacttattttttatagcttaatsaagctatataaggtaattaaaataatactattaattatttattaaaagatt

SEQ ID NO: 783 - DNA, 102 bp, synthetic construct
  misc_feature 1..102: note = Epichloe festucae
  misc_feature 51: note = Variation - S is A strain AR37 or G strain RGT18
  source 1..102: mol_type = other DNA
tataagctataggcagacagggactttattagaactaataaggataagtasatatttatttactagaacctatcctctaaagtctagtcctaggtggctact

SEQ ID NO: 784 - DNA, 102 bp, synthetic construct
  misc_feature 1..102: note = Epichloe festucae
  misc_feature 51: note = Variation - S is A strain AR37 or G strain RGT18
  source 1..102: mol_type = other DNA
ataagctaattctagttagacttatactacctattatgcgttagacttatsctacctattatatataaagcaaaggctttttatagtatttcacccttaaac

SEQ ID NO: 785 - DNA, 102 bp, synthetic construct
  misc_feature 1..102: note = Epichloe festucae
  misc_feature 51: note = Variation - S is G strain AR37 or A strain RGT18
  source 1..102: mol_type = other DNA
tttatgcctagtgctactttagtaatgttattattatcttaagagttatasgaagtatctaatagtaatatactaataagtagctagcctagtaaccttcta

SEQ ID NO: 786 - DNA, 102 bp, synthetic construct
  misc_feature 1..102: note = Epichloe festucae
  misc_feature 51: note = Variation - S is T strain AR37 or G strain RGT18
  source 1..102: mol_type = other DNA
gggactatttaatctataaagagattacctatagctagattcttttaaggstctttatgcatgcctaactttagatttttaacttaaatgcctagcgctact

SEQ ID NO: 787 - DNA, 102 bp, synthetic construct
  misc_feature 1..102: note = Epichloe festucae
  misc_feature 51: note = Variation - S is T strain AR37 or A strain RGT18
  source 1..102: mol_type = other DNA
acccttaggattattatcccctaggtctttctttttactagctttacctcsagtctttttacccttagtaattttttctttaaatatattacccttagtatt

SEQ ID NO: 788 - DNA, 102 bp, synthetic construct
  misc_feature 1..102: note = Epichloe festucae
  misc_feature 51: note = Variation - S is T strain AR37 or C strain RGT18
  source 1..102: mol_type = other DNA
ctatagtttgcgttaggactagtacctatagtaagggccttaatattaacsataatcttataatactacataatagctatataccacacgctttagctaata

SEQ ID NO: 789 - DNA, 102 bp, synthetic construct
  misc_feature 1..102: note = Epichloe festucae
  misc_feature 51: note = Variation - S is A strain AR37 or G strain RGT18
  source 1..102: mol_type = other DNA
ttactacctaggacttaattatataatatatttaatattactagtcttaasccttttaaaggggacctaactaatataaaagatatatccttactataagat

SEQ ID NO: 790 - DNA, 102 bp, synthetic construct
  misc_feature 1..102: note = Epichloe festucae
  misc_feature 51: note = Variation - S is T strain AR37 or C strain RGT18
  source 1..102: mol_type = other DNA
aagaggaatccatagtgaagtgagtctaggtctttttttccgattttttcsgattttttctgattttttccgatttctttctgatttttctaattttctgat

SEQ ID NO: 791 - DNA, 102 bp, synthetic construct
  misc_feature 1..102: note = Epichloe festucae
  misc_feature 51: note = Variation - S is T strain AR37 or C strain RGT18
  source 1..102: mol_type = other DNA
aagaaaaaagatattaagataaaaagacttttaaaaagtataaaaaaaatsattctataaactaaactaagaattactttattaaggtatataatataaact

SEQ ID NO: 792 - DNA, 102 bp, synthetic construct
  misc_feature 1..102: note = Epichloe festucae
  misc_feature 51: note = Variation - S is A strain AR37 or G strain RGT18
  source 1..102: mol_type = other DNA
aggatagatttaataaagctaaactaactagtcctaggataagtaattaasgctattataagactataagaagttaaatataataggaagtaagtaaatata

SEQ ID NO: 793 - DNA, 102 bp, synthetic construct
  misc_feature 1..102: note = Epichloe festucae
  misc_feature 51: note = Variation - S is T strain AR37 or C strain RGT18
  source 1..102: mol_type = other DNA
cataactaagtgctagtaacctagtactaatattataagtatagccctaastatatatctagatatatctatcttcactctaagatatataagtaagttaaa

SEQ ID NO: 794 - DNA, 102 bp, synthetic construct
  misc_feature 1..102: note = Epichloe festucae
  misc_feature 51: note = Variation - S is T strain AR37 or C strain RGT18
  source 1..102: mol_type = other DNA
atgctatataataaatagttaatttacttatttctagttaactaaaagacsagatataagtaagttatcttattactaaataaggaaggcctaactatttat

SEQ ID NO: 795 - DNA, 102 bp, synthetic construct
  misc_feature 1..102: note = Epichloe festucae
  misc_feature 51: note = Variation - S is T strain AR37 or C strain RGT18
  source 1..102: mol_type = other DNA
ctaataactctatagatttattataaccttagctaattcttaatatctatstagaataacttattagttactacttactattattaaagagtttagtttata

SEQ ID NO: 796 - DNA, 102 bp, synthetic construct
  misc_feature 1..102: note = Epichloe festucae
  misc_feature 51: note = Variation - S is C strain AR37 or T strain RGT18
  source 1..102: mol_type = other DNA
ctagtgtaaattaaaggggatatagtaaaggaagtaagatataacctatasattagctccttatataatatccttagggagggaaatggatttatagttaaa

SEQ ID NO: 797 - DNA, 102 bp, synthetic construct
  misc_feature 1..102: note = Epichloe festucae
  misc_feature 51: note = Variation - S is A strain AR37 or G strain RGT18
  source 1..102: mol_type = other DNA
tatctatagtattacccttatttaattaggtataactcttatttattaggsttaggttattatctaatattactcttatttattagggttaggttattatct

SEQ ID NO: 798 - DNA, 102 bp, synthetic construct
  misc_feature 1..102: note = Epichloe festucae
  misc_feature 51: note = Variation - S is C strain AR37 or T strain RGT18
  source 1..102: mol_type = other DNA
gcccaacaagctgattctcccatcgcccattttttccgactcgcccccccsccccccaccgaaatttagccaaccgctaaaaagtgcgggctcttgtctcaa

SEQ ID NO: 799 - DNA, 102 bp, synthetic construct
  misc_feature 1..102: note = Epichloe festucae
  misc_feature 51: note = Variation - S is T strain AR37 or C strain RGT18
  source 1..102: mol_type = other DNA
actttttttcttagccttatagttagctttaagttattaaaatctcttaastaattatttactttcttatagtattatttaagctatttaaaaagattataa

SEQ ID NO: 800 - DNA, 102 bp, synthetic construct
  misc_feature 1..102: note = Epichloe festucae
  misc_feature 51: note = Variation - S is A strain AR37 or G strain RGT18
  source 1..102: mol_type = other DNA
gcgaatacaggtagaatacctttacatttagatcctagctttaatataatsgaattaactattaggttagcttatagttactaatttagcatagtaataatc

SEQ ID NO: 801 - DNA, 102 bp, synthetic construct
  misc_feature 1..102: note = Epichloe festucae
  misc_feature 51: note = Variation - S is C strain AR37 or T strain RGT18
  source 1..102: mol_type = other DNA
actagtcccttattattaggggtggctataggtttataatagagttagtcsctaagactactagtcccttattattaggggtggctataggaactatagagg

SEQ ID NO: 802 - DNA, 102 bp, synthetic construct
  misc_feature 1..102: note = Epichloe festucae
  misc_feature 51: note = Variation - S is T strain AR37 or A strain RGT18
  source 1..102: mol_type = other DNA
ttctctaatttttactttaagcttactcttagcttactttttcttacctcstaattaattactaacctataccttttatcttttcctttctctttctcttac

SEQ ID NO: 803 - DNA, 102 bp, synthetic construct
  misc_feature 1..102: note = Epichloe festucae
  misc_feature 51: note = Variation - S is T strain AR37 or C strain RGT18
  source 1..102: mol_type = other DNA
gccttaaatactttcctatcttcttaaaaactttattataataaagtttasaagctcttttaacaaaaaccctaacttcactatctaatcttagttaagaga

SEQ ID NO: 804 - DNA, 102 bp, synthetic construct
  misc_feature 1..102: note = Epichloe festucae
  misc_feature 51: note = Variation - S is T strain AR37 or C strain RGT18
  source 1..102: mol_type = other DNA
ctataattctttagtaactctataagtgttaggagcgcagaggtcagagasaggatgtttattaaagcaagtcttcagagaacctttaggctatacgaataa

SEQ ID NO: 805 - DNA, 102 bp, synthetic construct
  misc_feature 1..102: note = Epichloe festucae
  misc_feature 51: note = Variation - S is T strain AR37 or C strain RGT18
  source 1..102: mol_type = other DNA
agagatcctaaactagtgctaagaagcttattacttcttaaagattaatastaagaatacttactattaaatctatattaaagagagtaataagtaaaagac

SEQ ID NO: 806 - DNA, 102 bp, synthetic construct
  misc_feature 1..102: note = Epichloe festucae
  misc_feature 51: note = Variation - S is G strain AR37 or A strain RGT18
  source 1..102: mol_type = other DNA
attagtaattataagttaatttccttaatattctaactttagcctttttasgttagagttagtaagttattagtattttaggttaggatatagctattaaag

SEQ ID NO: 807 - DNA, 102 bp, synthetic construct
  misc_feature 1..102: note = Epichloe festucae
  misc_feature 51: note = Variation - S is T strain AR37 or C strain RGT18
  source 1..102: mol_type = other DNA
actaaaaaagccatgtttaatttttatattctagggatagcttatagaacsaaaatcactagatatttcatagtaatagcagacgtaatgctaaatctagga

SEQ ID NO: 808 - DNA, 102 bp, synthetic construct
  misc_feature 1..102: note = Epichloe festucae
  misc_feature 51: note = Variation - S is A strain AR37 or T strain RGT18
  source 1..102: mol_type = other DNA
atttctatgaattattttatatttctataaattattattattacttatttsaaaaaaactataaaaagaactactagtaaacttaatataagtagcttatta

SEQ ID NO: 809 - DNA, 102 bp, synthetic construct
  misc_feature 1..102: note = Epichloe festucae
  misc_feature 51: note = Variation - S is T strain AR37 or C strain RGT18
  source 1..102: mol_type = other DNA
aattataggtctagtttaaggtctagctaatcctagatttaccttaagctstctaatttatacctttatttataagaccttttattttctttaaaggtaata

SEQ ID NO: 810 - DNA, 102 bp, synthetic construct
  misc_feature 1..102: note = Epichloe festucae
  misc_feature 51: note = Variation - S is A strain AR37 or T strain RGT18
  source 1..102: mol_type = other DNA
tattctagattaactaaaagactataactaggtccttaaggaagccctttsggtataacctataatctctagtgcttagctttacttatagtataaatctta

SEQ ID NO: 811 - DNA, 102 bp, synthetic construct
  misc_feature 1..102: note = Epichloe festucae
  misc_feature 51: note = Variation - S is T strain AR37 or G strain RGT18
  source 1..102: mol_type = other DNA
tcgaattcatattacataaatcactacgcttgtttatgggaagtaacagcstccgagatcgttggtcactgggcttgggactatcttgaaaagtcgcacaac

SEQ ID NO: 812 - DNA, 102 bp, synthetic construct
  misc_feature 1..102: note = Epichloe festucae
  misc_feature 51: note = Variation - S is T strain AR37 or C strain RGT18
  source 1..102: mol_type = other DNA
ttataactaattattaaggtaattctctataagaataagtattttcttagsatttagcttatattaattataaagaagcttaagtatcctttaggtataata

SEQ ID NO: 813 - DNA, 102 bp, synthetic construct
  misc_feature 1..102: note = Epichloe festucae
  misc_feature 51: note = Variation - S is T strain AR37 or A strain RGT18
  source 1..102: mol_type = other DNA
tgttattactaatctagtactaaagtaaataacttctaggttatagggttsaattattaataatggcattaatcttagtaaggctctagcctatgctagact

SEQ ID NO: 814 - DNA, 102 bp, synthetic construct
  misc_feature 1..102: note = Epichloe festucae
  misc_feature 51: note = Variation - S is T strain AR37 or C strain RGT18
  source 1..102: mol_type = other DNA
agctatattccataggaaactaagctaggtagcactctatagctatattcsataggaaactaagctaggtagcactactaaagtatatataaataatattag

SEQ ID NO: 815 - DNA, 102 bp, synthetic construct
  misc_feature 1..102: note = Epichloe festucae
  misc_feature 51: note = Variation - S is C strain AR37 or T strain RGT18
  source 1..102: mol_type = other DNA
gaacctatcttctataagctactagagggtataaatatataaggttatctstagaaaataactagagtattatataggctataggaagctccttaataatag

SEQ ID NO: 816 - DNA, 102 bp, synthetic construct
  misc_feature 1..102: note = Epichloe festucae
  misc_feature 51: note = Variation - S is T strain AR37 or C strain RGT18
  source 1..102: mol_type = other DNA
tttataagattaattaaaagcactttttactaagcctatatctaaccttasactatcttactcctaatagctaagtaaagcaagacctagcaagcacctaag

SEQ ID NO: 817 - DNA, 102 bp, synthetic construct
  misc_feature 1..102: note = Epichloe festucae
  misc_feature 51: note = Variation - S is T strain AR37 or C strain RGT18
  source 1..102: mol_type = other DNA
gggtttatagcttcttagagctttaggcatgcctaattttctagataatcsggatatttctagggcgctaggggacgctaactaagctattatcctaatgtt